European Patent Specification EP 3 550 023 B1, published June 25, 2025. Title: OLIGOMERS AND OLIGOMER CONJUGATES TARGETING HBV. Applicant: F. Hoffmann la Roche AG. The sequence listing filed with the application follows.

SEQUENCE LISTING (862 sequences)

SEQ ID NO: 1 - DNA, 746 bp, Hepatitis B virus
aacccccactggctggggcttggtcatgggccatcagcgcgtgcgtggaaccttttcggctcctctgccgatccatactgcggaactcctagccgcttgttttgctcgcagcaggtctggagcaaacattatcgggactgataactctgttgtcctctcccgcaaatatacatcgtatccatggctgctaggctgtgctgccaactggatcctgcgcgggacgtcctttgtttacgtcccgtcggcgctgaatcctgcggacgacccttctcggggtcgcttgggactctctcgtccccttctccgtctgccgttccgaccgaccacggggcgcacctctctttacgcggactccccgtctgtgccttctcatctgccggaccgtgtgcacttcgcttcacctctgcacgtcgcatggagaccaccgtgaacgcccaccgaatgttgcccaaggtcttacataagaggactcttggactctctgcaatgtcaacgaccgaccttgaggcatacttcaaagactgtttgtttaaagactgggaggagttgggggaggagattagattaaaggtctttgtactaggaggctgtaggcataaattggtctgcgcaccagcaccatgcaactttttcacctctgcctaatcatctcttgttcatgtcctactgttcaagcctccaagctgtgccttgggtggctttggggcatggacatcgacccttataaagaatttggagctactgtg

SEQ ID NO: 2 - DNA, 1969 bp, Hepatitis B virus
cactcatcctcaggccatgcagtggaattccacaacctttcaccaaactctgcaagatcccagagtgagaggcctgtatttccctgctggtggctccagttcaggagcagtaaaccctgttccgactactgcctctcccttatcgtcaatcttctcgaggattggggaccctgcgctgaacatggagaacatcacatcaggattcctaggaccccttctcgtgttacaggcggggtttttcttgttgacaagaatcctcacaataccgcagagtctagactcgtggtggacttctctcaattttctagggggaactaccgtgtgtcttggccaaaattcgcagtccccaacctccaatcactcaccaacctcctgtcctccaacttgtcctggttatcgctggatgtgtctgcggcgttttatcatcttcctcttcatcctgctgctatgcctcatcttcttgttggttcttctggactatcaaggtatgttgcccgtttgtcctctaattccaggatcctcaaccaccagcacgggaccatgccgaacctgcatgactactgctcaaggaacctctatgtatccctcctgttgctgtaccaaaccttcggacggaaattgcacctgtattcccatcccatcatcctgggctttcggaaaattcctatgggagtgggcctcagcccgtttctcctggctcagtttactagtgccatttgttcagtggttcgtagggctttcccccactgtttggctttcagttatatggatgatgtggtattgggggccaagtctgtacagcatcttgagtccctttttaccgctgttaccaattttcttttgtctttgggtatacatttaaaccctaacaaaacaaagagatggggttactctctgaattttatgggttatgtcattggaagttatgggtccttgccacaagaacacatcatacaaaaaatcaaagaatgttttagaaaacttcctattaacaggcctattgattggaaagtatgtcaacgaattgtgggtcttttgggttttgctgccccatttacacaatgtggttatcctgcgttaatgcccttgtatgcatgtattcaatctaagcaggctttcactttctcgccaacttacaaggcctttctgtgtaaacaatacctgaacctttaccccgttgcccggcaacggccaggtctgtgccaagtgtttgctgacgcaacccccactggctggggcttggtcatgggccatcagcgcgtgcgtggaaccttttcggctcctctgccgatccatactgcggaactcctagccgcttgttttgctcgcagcaggtctggagcaaacattatcgggactgataactctgttgtcctctcccgcaaatatacatcgtatccatggctgctaggctgtgctgccaactggatcctgcgcgggacgtcctttgtttacgtcccgtcggcgctgaatcctgcggacgacccttctcggggtcgcttgggactctctcgtccccttctccgtctgccgttccgaccgaccacggggcgcacctctctttacgcggactccccgtctgtgccttctcatctgccggaccgtgtgcacttcgcttcacctctgcacgtcgcatggagaccaccgtgaacgcccaccgaatgttgcccaaggtcttacataagaggactcttggactctctgcaatgtcaacgaccgaccttgaggcatacttcaaagactgtttgtttaaagactgggaggagttgggggaggagattagattaaaggtctttgtactaggaggctgtaggcataaattggtctgcgcaccagcaccatgcaactttttcacctctgcctaatcatctcttgttcatgtcctactgttcaagcctccaagctgtgccttgggtggctttggggcatggacatcgacccttataaagaatttggagctactgtggag

SEQ ID NO: 3 - DNA, 3182 bp, Hepatitis B virus
aattccacaacctttcaccaaactctgcaagatcccagagtgagaggcctgtatttccctgctggtggctccagttcaggagcagtaaaccctgttccgactactgcctctcccttatcgtcaatcttctcgaggattggggaccctgcgctgaacatggagaacatcacatcaggattcctaggaccccttctcgtgttacaggcggggtttttcttgttgacaagaatcctcacaataccgcagagtctagactcgtggtggacttctctcaattttctagggggaactaccgtgtgtcttggccaaaattcgcagtccccaacctccaatcactcaccaacctcctgtcctccaacttgtcctggttatcgctggatgtgtctgcggcgttttatcatcttcctcttcatcctgctgctatgcctcatcttcttgttggttcttctggactatcaaggtatgttgcccgtttgtcctctaattccaggatcctcaaccaccagcacgggaccatgccgaacctgcatgactactgctcaaggaacctctatgtatccctcctgttgctgtaccaaaccttcggacggaaattgcacctgtattcccatcccatcatcctgggctttcggaaaattcctatgggagtgggcctcagcccgtttctcctggctcagtttactagtgccatttgttcagtggttcgtagggctttcccccactgtttggctttcagttatatggatgatgtggtattgggggccaagtctgtacagcatcttgagtccctttttaccgctgttaccaattttcttttgtctttgggtatacatttaaaccctaacaaaacaaagagatggggttactctctgaattttatgggttatgtcattggaagttatgggtccttgccacaagaacacatcatacaaaaaatcaaagaatgttttagaaaacttcctattaacaggcctattgattggaaagtatgtcaacgaattgtgggtcttttgggttttgctgccccatttacacaatgtggttatcctgcgttaatgcccttgtatgcatgtattcaatctaagcaggctttcactttctcgccaacttacaaggcctttctgtgtaaacaatacctgaacctttaccccgttgcccggcaacggccaggtctgtgccaagtgtttgctgacgcaacccccactggctggggcttggtcatgggccatcagcgcgtgcgtggaaccttttcggctcctctgccgatccatactgcggaactcctagccgcttgttttgctcgcagcaggtctggagcaaacattatcgggactgataactctgttgtcctctcccgcaaatatacatcgtatccatggctgctaggctgtgctgccaactggatcctgcgcgggacgtcctttgtttacgtcccgtcggcgctgaatcctgcggacgacccttctcggggtcgcttgggactctctcgtccccttctccgtctgccgttccgaccgaccacggggcgcacctctctttacgcggactccccgtctgtgccttctcatctgccggaccgtgtgcacttcgcttcacctctgcacgtcgcatggagaccaccgtgaacgcccaccgaatgttgcccaaggtcttacataagaggactcttggactctctgcaatgtcaacgaccgaccttgaggcatacttcaaagactgtttgtttaaagactgggaggagttgggggaggagattagattaaaggtctttgtactaggaggctgtaggcataaattggtctgcgcaccagcaccatgcaactttttcacctctgcctaatcatctcttgttcatgtcctactgttcaagcctccaagctgtgccttgggtggctttggggcatggacatcgacccttataaagaatttggagctactgtggagttactctcgtttttgccttctgacttctttccttcagtacgagatcttctagataccgcctcagctctgtatcgggaagccttagagtctcctgagcattgttcacctcaccatactgcactcaggcaagcaattctttgctggggggaactaatgactctagctacctgggtgggtgttaatttggaagatccagcatctagagacctagtagtcagttatgtcaacactaatatgggcctaaagttcaggcaactcttgtggtttcacatttcttgtctcacttttggaagagaaaccgttatagagtatttggtgtctttcggagtgtggattcgcactcctccagcttatagaccaccaaatgcccctatcctatcaacacttccggaaactactgttgttagacgacgaggcaggtcccctagaagaagaactccctcgcctcgcagacgaaggtctcaatcgccgcgtcgcagaagatctcaatctcgggaacctcaatgttagtattccttggactcataaggtggggaactttactggtctttattcttctactgtacctgtctttaatcctcattggaaaacaccatcttttcctaatatacatttacaccaagacattatcaaaaaatgtgaacagtttgtaggcccacttacagttaatgagaaaagaagattgcaattgattatgcctgctaggttttatccaaaggttaccaaatatttaccattggataagggtattaaaccttattatccagaacatctagttaatcattacttccaaactagacactatttacacactctatggaaggcgggtatattatataagagagaaacaacacatagcgcctcattttgtgggtcaccatattcttgggaacaagatctacagcatggggcagaatctttccaccagcaatcctctgggattctttcccgaccaccagttggatccagccttcagagcaaacacagcaaatccagattgggacttcaatcccaacaaggacacctggccagacgccaacaaggtaggagctggagcattcgggctgggtttcaccccaccgcacggaggccttttggggtggagccctcaggctcagggcatactacaaactttgccagcaaatccgcctcctgcctccaccaatcgccagacaggaaggcagcctaccccgctgtctccacctttgagaaacactcatcctcaggccatgcagtgg

SEQ ID NO: 4 - DNA, 15 bp, Artificial Sequence
  oligonucleotide sequence motif
gaaccactgaacaaa

SEQ ID NO: 5 - DNA, 16 bp, Artificial Sequence
  oligonucleotide sequence motif
cgaaccactgaacaaa

SEQ ID NO: 6 - DNA, 15 bp, Artificial Sequence
  oligonucleotide sequence motif
cgaaccactgaacaa

SEQ ID NO: 7 - DNA, 14 bp, Artificial Sequence
  oligonucleotide sequence motif
cgaaccactgaaca

SEQ ID NO: 8 - DNA, 13 bp, Artificial Sequence
  oligonucleotide sequence motif
cgaaccactgaac

SEQ ID NO: 9 - DNA, 15 bp, Artificial Sequence
  oligonucleotide sequence motif
ccgcagtatggatcg

SEQ ID NO: 10 - DNA, 13 bp, Artificial Sequence
  oligonucleotide sequence motif
cgcagtatggatc

SEQ ID NO: 11 - DNA, 14 bp, Artificial Sequence
  oligonucleotide sequence motif
gcgtaaagagaggt

SEQ ID NO: 12 - DNA, 15 bp, Artificial Sequence
  oligonucleotide sequence motif
cgcgtaaagagaggt

SEQ ID NO: 13 - DNA, 13 bp, Artificial Sequence
  oligonucleotide sequence motif
gcgtaaagagagg

SEQ ID NO: 14 - DNA, 15 bp, Artificial Sequence
  oligonucleotide sequence motif
agaaggcacagacgg

SEQ ID NO: 15 - DNA, 16 bp, Artificial Sequence
  oligonucleotide sequence motif
gagaaggcacagacgg

SEQ ID NO: 16 - DNA, 13 bp, Artificial Sequence
  oligonucleotide sequence motif
gaagtgcacacgg

SEQ ID NO: 17 - DNA, 15 bp, Artificial Sequence
  oligonucleotide sequence motif
gcgaagtgcacacgg

SEQ ID NO: 18 - DNA, 16 bp, Artificial Sequence
  oligonucleotide sequence motif
agcgaagtgcacacgg

SEQ ID NO: 19 - DNA, 13 bp, Artificial Sequence
  oligonucleotide sequence motif
cgaagtgcacacg

SEQ ID NO: 20 - DNA, 15 bp, Artificial Sequence
  oligonucleotide sequence motif
agcgaagtgcacacg

SEQ ID NO: 21 - DNA, 16 bp, Artificial Sequence
  oligonucleotide sequence motif
aagcgaagtgcacacg

SEQ ID NO: 22 - DNA, 15 bp, Artificial Sequence
  oligonucleotide sequence motif
gaagcgaagtgcaca

SEQ ID NO: 23 - DNA, 16 bp, Artificial Sequence
  oligonucleotide sequence motif
ggtgaagcgaagtgca

SEQ ID NO: 24 - DNA, 15 bp, Artificial Sequence
  oligonucleotide sequence motif
ggtgaagcgaagtgc

SEQ ID NO: 25 - DNA, 16 bp, Artificial Sequence
  oligonucleotide sequence motif
aggtgaagcgaagtgc

SEQ ID NO: 26 - DNA, 15 bp, Artificial Sequence
  oligonucleotide sequence motif
aggtgaagcgaagtg

SEQ ID NO: 27 - DNA, 14 bp, Artificial Sequence
  oligonucleotide sequence motif
aggtgaagcgaagt

SEQ ID NO: 28 - DNA, 14 bp, Artificial Sequence
  oligonucleotide sequence motif
cagaggtgaagcga

SEQ ID NO: 29 - DNA, 14 bp, Artificial Sequence
  oligonucleotide sequence motif
aaaaccccgcctgt

SEQ ID NO: 30 - DNA, 13 bp, Artificial Sequence
  oligonucleotide sequence motif
aaaaccccgcctg

SEQ ID NO: 31 - DNA, 15 bp, Artificial Sequence
  oligonucleotide sequence motif
acgagtctagactct

SEQ ID NO: 32 - DNA, 16 bp, Artificial Sequence
  oligonucleotide sequence motif
cacgagtctagactct

SEQ ID NO: 33 - DNA, 14 bp, Artificial Sequence
  oligonucleotide sequence motif
acgagtctagactc

SEQ ID NO: 34 - DNA, 15 bp, Artificial Sequence
  oligonucleotide sequence motif
cacgagtctagactc

SEQ ID NO: 35 - DNA, 16 bp, Artificial Sequence
  oligonucleotide sequence motif
ccacgagtctagactc

SEQ ID NO: 36 - DNA, 13 bp, Artificial Sequence
  oligonucleotide sequence motif
acgagtctagact

SEQ ID NO: 37 - DNA, 14 bp, Artificial Sequence
  oligonucleotide sequence motif
cacgagtctagact

SEQ ID NO: 38 - DNA, 15 bp, Artificial Sequence
  oligonucleotide sequence motif
ccacgagtctagact

SEQ ID NO: 39 - DNA, 16 bp, Artificial Sequence
  oligonucleotide sequence motif
accacgagtctagact

SEQ ID NO: 40 - DNA, 12 bp, Artificial Sequence
  oligonucleotide sequence motif
acgagtctagac

SEQ ID NO: 41 - DNA, 13 bp, Artificial Sequence
  oligonucleotide sequence motif
cacgagtctagac

SEQ ID NO: 42 - DNA, 14 bp, Artificial Sequence
  oligonucleotide sequence motif
ccacgagtctagac

SEQ ID NO: 43 - DNA, 15 bp, Artificial Sequence
  oligonucleotide sequence motif
accacgagtctagac

SEQ ID NO: 44 - DNA, 16 bp, Artificial Sequence
  oligonucleotide sequence motif
caccacgagtctagac

SEQ ID NO: 45 - DNA, 14 bp, Artificial Sequence
  oligonucleotide sequence motif
accacgagtctaga

SEQ ID NO: 46 - DNA, 15 bp, Artificial Sequence
  oligonucleotide sequence motif
caccacgagtctaga

SEQ ID NO: 47 - DNA, 16 bp, Artificial Sequence
  oligonucleotide sequence motif
ccaccacgagtctaga

SEQ ID NO: 48 - DNA, 15 bp, Artificial Sequence
  oligonucleotide sequence motif
ccaccacgagtctag

SEQ ID NO: 49 - DNA, 16 bp, Artificial Sequence
  oligonucleotide sequence motif
tccaccacgagtctag

SEQ ID NO: 50 - DNA, 14 bp, Artificial Sequence
  oligonucleotide sequence motif
ccaccacgagtcta

SEQ ID NO: 51 - DNA, 15 bp, Artificial Sequence
  oligonucleotide sequence motif
tccaccacgagtcta

SEQ ID NO: 52 - DNA, 16 bp, Artificial Sequence
  oligonucleotide sequence motif
gtccaccacgagtcta

SEQ ID NO: 53 - DNA, 14 bp, Artificial Sequence
  oligonucleotide sequence motif
tccaccacgagtct

SEQ ID NO: 54 - DNA, 15 bp, Artificial Sequence
  oligonucleotide sequence motif
gtccaccacgagtct

SEQ ID NO: 55 - DNA, 16 bp, Artificial Sequence
  oligonucleotide sequence motif
agtccaccacgagtct

SEQ ID NO: 56 - DNA, 14 bp, Artificial Sequence
  oligonucleotide sequence motif
gtccaccacgagtc

SEQ ID NO: 57 - DNA, 15 bp, Artificial Sequence
  oligonucleotide sequence motif
agtccaccacgagtc

SEQ ID NO: 58 - DNA, 16 bp, Artificial Sequence
  oligonucleotide sequence motif
aagtccaccacgagtc

SEQ ID NO: 59 - DNA, 14 bp, Artificial Sequence
  oligonucleotide sequence motif
agtccaccacgagt

SEQ ID NO: 60 - DNA, 15 bp, Artificial Sequence
  oligonucleotide sequence motif
aagtccaccacgagt

SEQ ID NO: 61 - DNA, 16 bp, Artificial Sequence
  oligonucleotide sequence motif
gaagtccaccacgagt

SEQ ID NO: 62 - DNA, 14 bp, Artificial Sequence
  oligonucleotide sequence motif
aagtccaccacgag

SEQ ID NO: 63 - DNA, 15 bp, Artificial Sequence
  oligonucleotide sequence motif
gaagtccaccacgag

SEQ ID NO: 64 - DNA, 16 bp, Artificial Sequence
  oligonucleotide sequence motif
agaagtccaccacgag

SEQ ID NO: 65 - DNA, 15 bp, Artificial Sequence
  oligonucleotide sequence motif
agaagtccaccacga

SEQ ID NO: 66 - DNA, 16 bp, Artificial Sequence
  oligonucleotide sequence motif
gagaagtccaccacga

SEQ ID NO: 67 - DNA, 15 bp, Artificial Sequence
  oligonucleotide sequence motif
gagaagtccaccacg

SEQ ID NO: 68 - DNA, 16 bp, Artificial Sequence
  oligonucleotide sequence motif
agagaagtccaccacg

SEQ ID NO: 69 - DNA, 16 bp, Artificial Sequence
  oligonucleotide sequence motif
gagagaagtccaccac

SEQ ID NO: 70 - DNA, 15 bp, Artificial Sequence
  oligonucleotide sequence motif
gagagaagtccacca

SEQ ID NO: 71 - DNA, 16 bp, Artificial Sequence
  oligonucleotide sequence motif
tgagagaagtccacca

SEQ ID NO: 72 - DNA, 14 bp, Artificial Sequence
  oligonucleotide sequence motif
gagagaagtccacc

SEQ ID NO: 73 - DNA, 15 bp, Artificial Sequence
  oligonucleotide sequence motif
tgagagaagtccacc

SEQ ID NO: 74 - DNA, 14 bp, Artificial Sequence
  oligonucleotide sequence motif
tgagagaagtccac

SEQ ID NO: 75 - DNA, 13 bp, Artificial Sequence
  oligonucleotide sequence motif
aaaacgccgcaga

SEQ ID NO: 76 - DNA, 14 bp, Artificial Sequence
  oligonucleotide sequence motif
taaaacgccgcaga

SEQ ID NO: 77 - DNA, 15 bp, Artificial Sequence
  oligonucleotide sequence motif
ataaaacgccgcaga

SEQ ID NO: 78 - DNA, 16 bp, Artificial Sequence
  oligonucleotide sequence motif
gataaaacgccgcaga

SEQ ID NO: 79 - DNA, 14 bp, Artificial Sequence
  oligonucleotide sequence motif
ataaaacgccgcag

SEQ ID NO: 80 - DNA, 15 bp, Artificial Sequence
  oligonucleotide sequence motif
gataaaacgccgcag

SEQ ID NO: 81 - DNA, 16 bp, Artificial Sequence
  oligonucleotide sequence motif
tgataaaacgccgcag

SEQ ID NO: 82 - DNA, 13 bp, Artificial Sequence
  oligonucleotide sequence motif
ataaaacgccgca

SEQ ID NO: 83 - DNA, 14 bp, Artificial Sequence
  oligonucleotide sequence motif
gataaaacgccgca

SEQ ID NO: 84 - DNA, 15 bp, Artificial Sequence
  oligonucleotide sequence motif
tgataaaacgccgca

SEQ ID NO: 85 - DNA, 16 bp, Artificial Sequence
  oligonucleotide sequence motif
atgataaaacgccgca

SEQ ID NO: 86 - DNA, 12 bp, Artificial Sequence
  oligonucleotide sequence motif
ataaaacgccgc

SEQ ID NO: 87 - DNA, 13 bp, Artificial Sequence
  oligonucleotide sequence motif
gataaaacgccgc

SEQ ID NO: 88 - DNA, 14 bp, Artificial Sequence
  oligonucleotide sequence motif
tgataaaacgccgc

SEQ ID NO: 89 - DNA, 15 bp, Artificial Sequence
  oligonucleotide sequence motif
atgataaaacgccgc

SEQ ID NO: 90 - DNA, 12 bp, Artificial Sequence
  oligonucleotide sequence motif
gataaaacgccg

SEQ ID NO: 91 - DNA, 13 bp, Artificial Sequence
  oligonucleotide sequence motif
tgataaaacgccg

SEQ ID NO: 92 - DNA, 14 bp, Artificial Sequence
  oligonucleotide sequence motif
atgataaaacgccg

SEQ ID NO: 93 - DNA, 12 bp, Artificial Sequence
  oligonucleotide sequence motif
tgataaaacgcc

SEQ ID NO: 94 - DNA, 13 bp, Artificial Sequence
  oligonucleotide sequence motif
atgataaaacgcc

SEQ ID NO: 95 - DNA, 12 bp, Artificial Sequence
  oligonucleotide sequence motif
atgataaaacgc

SEQ ID NO: 96 - DNA, 13 bp, Artificial Sequence
  oligonucleotide sequence motif
tagcagcaggatg

SEQ ID NO: 97 - DNA, 14 bp, Artificial Sequence
  oligonucleotide sequence motif
atagcagcaggatg

SEQ ID NO: 98 - DNA, 15 bp, Artificial Sequence
  oligonucleotide sequence motif
catagcagcaggatg

SEQ ID NO: 99 - DNA, 16 bp, Artificial Sequence
  oligonucleotide sequence motif
gcatagcagcaggatg

SEQ ID NO: 100 - DNA, 15 bp, Artificial Sequence
  oligonucleotide sequence motif
gcatagcagcaggat

SEQ ID NO: 101 - DNA, 16 bp, Artificial Sequence
  oligonucleotide sequence motif
ggcatagcagcaggat

SEQ ID NO: 102 - DNA, 16 bp, Artificial Sequence
  oligonucleotide sequence motif
gaggcatagcagcagg

SEQ ID NO: 103 - DNA, 16 bp, Artificial Sequence
  oligonucleotide sequence motif
tgaggcatagcagcag

SEQ ID NO: 104 - DNA, 15 bp, Artificial Sequence
  oligonucleotide sequence motif
tgaggcatagcagca

SEQ ID NO: 105 - DNA, 16 bp, Artificial Sequence
  oligonucleotide sequence motif
atgaggcatagcagca

SEQ ID NO: 106 - DNA, 14 bp, Artificial Sequence
  oligonucleotide sequence motif
tgaggcatagcagc

SEQ ID NO: 107 - DNA, 15 bp, Artificial Sequence
  oligonucleotide sequence motif
atgaggcatagcagc

SEQ ID NO: 108 - DNA, 16 bp, Artificial Sequence
  oligonucleotide sequence motif
gatgaggcatagcagc

SEQ ID NO: 109 - DNA, 15 bp, Artificial Sequence
  oligonucleotide sequence motif
gatgaggcatagcag

SEQ ID NO: 110 - DNA, 16 bp, Artificial Sequence
  oligonucleotide sequence motif
agatgaggcatagcag

SEQ ID NO: 111 - DNA, 14 bp, Artificial Sequence
  oligonucleotide sequence motif
gatgaggcatagca

SEQ ID NO: 112 - DNA, 15 bp, Artificial Sequence
  oligonucleotide sequence motif
agatgaggcatagca

SEQ ID NO: 113 - DNA, 16 bp, Artificial Sequence
  oligonucleotide sequence motif
aagatgaggcatagca

SEQ ID NO: 114 - DNA, 16 bp, Artificial Sequence
  oligonucleotide sequence motif
aagaagatgaggcata

SEQ ID NO: 115 - DNA, 15 bp, Artificial Sequence
  oligonucleotide sequence motif
aagaagatgaggcat

SEQ ID NO: 116 - DNA, 15 bp, Artificial Sequence
  oligonucleotide sequence motif
tgggatgggaataca

SEQ ID NO: 117 - DNA, 16 bp, Artificial Sequence
  oligonucleotide sequence motif
atgggatgggaataca

SEQ ID NO: 118 - DNA, 14 bp, Artificial Sequence
  oligonucleotide sequence motif
tgggatgggaatac

SEQ ID NO: 119 - DNA, 15 bp, Artificial Sequence
  oligonucleotide sequence motif
atgggatgggaatac

SEQ ID NO: 120 - DNA, 16 bp, Artificial Sequence
  oligonucleotide sequence motif
gatgggatgggaatac

SEQ ID NO: 121 - DNA, 14 bp, Artificial Sequence
  oligonucleotide sequence motif
atgggatgggaata

SEQ ID NO: 122 - DNA, 15 bp, Artificial Sequence
  oligonucleotide sequence motif
gatgggatgggaata

SEQ ID NO: 123 - DNA, 14 bp, Artificial Sequence
  oligonucleotide sequence motif
gatgggatgggaat

SEQ ID NO: 124 - DNA, 14 bp, Artificial Sequence
  oligonucleotide sequence motif
aaccactgaacaaa

SEQ ID NO: 125 - DNA, 12 bp, Artificial Sequence
  oligonucleotide sequence motif
cgaaccactgaa

SEQ ID NO: 126 - DNA, 13 bp, Artificial Sequence
  oligonucleotide sequence motif
gggggaaagccct

SEQ ID NO: 127 - DNA, 14 bp, Artificial Sequence
  oligonucleotide sequence motif
tgggggaaagccct

SEQ ID NO: 128 - DNA, 15 bp, Artificial Sequence
  oligonucleotide sequence motif
gcaacggggtaaagg

SEQ ID NO: 129 - DNA, 14 bp, Artificial Sequence
  oligonucleotide sequence motif
gcaacggggtaaag

SEQ ID NO: 130 - DNA, 13 bp, Artificial Sequence
  oligonucleotide sequence motif
gcaacggggtaaa

SEQ ID NO: 131 - DNA, 15 bp, Artificial Sequence
  oligonucleotide sequence motif
agcaaacacttggca

SEQ ID NO: 132 - DNA, 16 bp, Artificial Sequence
  oligonucleotide sequence motif
cagcaaacacttggca

SEQ ID NO: 133 - DNA, 15 bp, Artificial Sequence
  oligonucleotide sequence motif
cagcaaacacttggc

SEQ ID NO: 134 - DNA, 16 bp, Artificial Sequence
  oligonucleotide sequence motif
tcagcaaacacttggc

SEQ ID NO: 135 - DNA, 15 bp, Artificial Sequence
  oligonucleotide sequence motif
tcagcaaacacttgg

SEQ ID NO: 136 - DNA, 13 bp, Artificial Sequence
  oligonucleotide sequence motif
gcagtatggatcg

SEQ ID NO: 137 - DNA, 14 bp, Artificial Sequence
  oligonucleotide sequence motif
cgcagtatggatcg

SEQ ID NO: 138 - DNA, 16 bp, Artificial Sequence
  oligonucleotide sequence motif
tccgcagtatggatcg

SEQ ID NO: 139 - DNA, 14 bp, Artificial Sequence
  oligonucleotide sequence motif
ccgcagtatggatc

SEQ ID NO: 140 - DNA, 15 bp, Artificial Sequence
  oligonucleotide sequence motif
tccgcagtatggatc

SEQ ID NO: 141 - DNA, 12 bp, Artificial Sequence
  oligonucleotide sequence motif
cgcagtatggat

SEQ ID NO: 142 - DNA, 13 bp, Artificial Sequence
  oligonucleotide sequence motif
ccgcagtatggat

SEQ ID NO: 143 - DNA, 14 bp, Artificial Sequence
  oligonucleotide sequence motif
tccgcagtatggat

SEQ ID NO: 144 - DNA, 13 bp, Artificial Sequence
  oligonucleotide sequence motif
tccgcagtatgga

SEQ ID NO: 145 - DNA, 12 bp, Artificial Sequence
  oligonucleotide sequence motif
ttccgcagtatg

SEQ ID NO: 146 - DNA, 13 bp, Artificial Sequence
  oligonucleotide sequence motif
cgtaaagagaggt

SEQ ID NO: 147 - DNA, 16 bp, Artificial Sequence
  oligonucleotide sequence motif
ccgcgtaaagagaggt

SEQ ID NO: 148 - DNA, 12 bp, Artificial Sequence
  oligonucleotide sequence motif
cgtaaagagagg

SEQ ID NO: 149 - DNA, 14 bp, Artificial Sequence
  oligonucleotide sequence motif
cgcgtaaagagagg

SEQ ID NO: 150 - DNA, 15 bp, Artificial Sequence
  oligonucleotide sequence motif
ccgcgtaaagagagg

SEQ ID NO: 151 - DNA, 13 bp, Artificial Sequence
  oligonucleotide sequence motif
cgcgtaaagagag

SEQ ID NO: 152 - DNA, 14 bp, Artificial Sequence
  oligonucleotide sequence motif
ccgcgtaaagagag

SEQ ID NO: 153 - DNA, 12 bp, Artificial Sequence
  oligonucleotide sequence motif
cgcgtaaagaga

SEQ ID NO: 154 - DNA, 13 bp, Artificial Sequence
  oligonucleotide sequence motif
ccgcgtaaagaga

SEQ ID NO: 155 - DNA, 12 bp, Artificial Sequence
  oligonucleotide sequence motif
ccgcgtaaagag

SEQ ID NO: 156 - DNA, 15 bp, Artificial Sequence
  oligonucleotide sequence motif
ggcacagacggggag

SEQ ID NO: 157 - DNA, 16 bp, Artificial Sequence
  oligonucleotide sequence motif
aggcacagacggggag

SEQ ID NO: 158 - DNA, 14 bp, Artificial Sequence
  oligonucleotide sequence motif
ggcacagacgggga

SEQ ID NO: 159 - DNA, 15 bp, Artificial Sequence
  oligonucleotide sequence motif
aggcacagacgggga

SEQ ID NO: 160 - DNA, 16 bp, Artificial Sequence
  oligonucleotide sequence motif
aaggcacagacgggga

SEQ ID NO: 161 - DNA, 14 bp, Artificial Sequence
  oligonucleotide sequence motif
aggcacagacgggg

SEQ ID NO: 162 - DNA, 15 bp, Artificial Sequence
  oligonucleotide sequence motif
aaggcacagacgggg

SEQ ID NO: 163 - DNA, 16 bp, Artificial Sequence
  oligonucleotide sequence motif
gaaggcacagacgggg

SEQ ID NO: 164 - DNA, 16 bp, Artificial Sequence
  oligonucleotide sequence motif
agaaggcacagacggg

SEQ ID NO: 165 - DNA, 15 bp, Artificial Sequence
  oligonucleotide sequence motif
gagaaggcacagacg

SEQ ID NO: 166 - DNA, 14 bp, Artificial Sequence
  oligonucleotide sequence motif
cgaagtgcacacgg

SEQ ID NO: 167 - DNA, 14 bp, Artificial Sequence
  oligonucleotide sequence motif
gcgaagtgcacacg

SEQ ID NO: 168 - DNA, 13 bp, Artificial Sequence
  oligonucleotide sequence motif
gcgaagtgcacac

SEQ ID NO: 169 - DNA, 14 bp, Artificial Sequence
  oligonucleotide sequence motif
agcgaagtgcacac

SEQ ID NO: 170 - DNA, 15 bp, Artificial Sequence
  oligonucleotide sequence motif
aagcgaagtgcacac

SEQ ID NO: 171 - DNA, 16 bp, Artificial Sequence
  oligonucleotide sequence motif
gaagcgaagtgcacac

SEQ ID NO: 172 - DNA, 13 bp, Artificial Sequence
  oligonucleotide sequence motif
agcgaagtgcaca

SEQ ID NO: 173 - DNA, 14 bp, Artificial Sequence
  oligonucleotide sequence motif
aagcgaagtgcaca

SEQ ID NO: 174 - DNA, 16 bp, Artificial Sequence
  oligonucleotide sequence motif
tgaagcgaagtgcaca

SEQ ID NO: 175 - DNA, 13 bp, Artificial Sequence
  oligonucleotide sequence motif
aagcgaagtgcac

SEQ ID NO: 176 - DNA, 14 bp, Artificial Sequence
  oligonucleotide sequence motif
gaagcgaagtgcac

SEQ ID NO: 177 - DNA, 15 bp, Artificial Sequence
  oligonucleotide sequence motif
tgaagcgaagtgcac

SEQ ID NO: 178 - DNA, 16 bp, Artificial Sequence
  oligonucleotide sequence motif
gtgaagcgaagtgcac

SEQ ID NO: 179 - DNA, 12 bp, Artificial Sequence
  oligonucleotide sequence motif
aagcgaagtgca

SEQ ID NO: 180 - DNA, 13 bp, Artificial Sequence
  oligonucleotide sequence motif
gaagcgaagtgca

SEQ ID NO: 181 - DNA, 14 bp, Artificial Sequence
  oligonucleotide sequence motif
tgaagcgaagtgca

SEQ ID NO: 182 - DNA, 15 bp, Artificial Sequence
  oligonucleotide sequence motif
gtgaagcgaagtgca

SEQ ID NO: 183 - DNA, 13 bp, Artificial Sequence
  oligonucleotide sequence motif
tgaagcgaagtgc

SEQ ID NO: 184 - DNA, 14 bp, Artificial Sequence
  oligonucleotide sequence motif
gtgaagcgaagtgc

SEQ ID NO: 185 - DNA, 13 bp, Artificial Sequence
  oligonucleotide sequence motif
gtgaagcgaagtg

SEQ ID NO: 186 - DNA, 14 bp, Artificial Sequence
  oligonucleotide sequence motif
ggtgaagcgaagtg

SEQ ID NO: 187 - DNA, 16 bp, Artificial Sequence
  oligonucleotide sequence motif
gaggtgaagcgaagtg

SEQ ID NO: 188 - DNA, 12 bp, Artificial Sequence
  oligonucleotide sequence motif
gtgaagcgaagt

SEQ ID NO: 189 - DNA, 13 bp, Artificial Sequence
  oligonucleotide sequence motif
ggtgaagcgaagt

SEQ ID NO: 190 - DNA, 15 bp, Artificial Sequence
  oligonucleotide sequence motif
gaggtgaagcgaagt

SEQ ID NO: 191 - DNA, 16 bp, Artificial Sequence
  oligonucleotide sequence motif
agaggtgaagcgaagt

SEQ ID NO: 192 - DNA, 15 bp, Artificial Sequence
  oligonucleotide sequence motif
agaggtgaagcgaag

SEQ ID NO: 193 - DNA, 16 bp, Artificial Sequence
  oligonucleotide sequence motif
cagaggtgaagcgaag

SEQ ID NO: 194 - DNA, 14 bp, Artificial Sequence
  oligonucleotide sequence motif
agaggtgaagcgaa

SEQ ID NO: 195 - DNA, 15 bp, Artificial Sequence
  oligonucleotide sequence motif
cagaggtgaagcgaa

SEQ ID NO: 196 - DNA, 16 bp, Artificial Sequence
  oligonucleotide sequence motif
gcagaggtgaagcgaa

SEQ ID NO: 197 - DNA, 15 bp, Artificial Sequence
  oligonucleotide sequence motif
gcagaggtgaagcga

SEQ ID NO: 198 - DNA, 16 bp, Artificial Sequence
  oligonucleotide sequence motif
tgcagaggtgaagcga

SEQ ID NO: 199 - DNA, 15 bp, Artificial Sequence
  oligonucleotide sequence motif
tgcagaggtgaagcg

SEQ ID NO: 200 - DNA, 16 bp, Artificial Sequence
  oligonucleotide sequence motif
gtgcagaggtgaagcg

SEQ ID NO: 201 - DNA, 16 bp, Artificial Sequence
  oligonucleotide sequence motif
cgtgcagaggtgaagc

SEQ ID NO: 202 - DNA, 15 bp, Artificial Sequence
  oligonucleotide sequence motif
cgtgcagaggtgaag

SEQ ID NO: 203 - DNA, 16 bp, Artificial Sequence
  oligonucleotide sequence motif
acgtgcagaggtgaag

SEQ ID NO: 204 - DNA, 14 bp, Artificial Sequence
  oligonucleotide sequence motif
cgtgcagaggtgaa

SEQ ID NO: 205 - DNA, 15 bp, Artificial Sequence
  oligonucleotide sequence motif
acgtgcagaggtgaa

SEQ ID NO: 206 - DNA, 13 bp, Artificial Sequence
  oligonucleotide sequence motif
cgtgcagaggtga

SEQ ID NO: 207 - DNA, 14 bp, Artificial Sequence
  oligonucleotide sequence motif
acgtgcagaggtga

SEQ ID NO: 208 - DNA, 13 bp, Artificial Sequence
  oligonucleotide sequence motif
cgttcacggtggt

SEQ ID NO: 209 - DNA, 13 bp, Artificial Sequence
  oligonucleotide sequence motif
ctcaaggtcggtc

SEQ ID NO: 210 - DNA, 13 bp, Artificial Sequence
  oligonucleotide sequence motif
cctcaaggtcggt

SEQ ID NO: 211 - DNA, 14 bp, Artificial Sequence
  oligonucleotide sequence motif
gcctcaaggtcggt

SEQ ID NO: 212 - DNA, 15 bp, Artificial Sequence
  oligonucleotide sequence motif
acagtctttgaagta

SEQ ID NO: 213 - DNA, 13 bp, Artificial Sequence
  oligonucleotide sequence motif
tttatgcctacag

SEQ ID NO: 214 - DNA, 14 bp, Artificial Sequence
  oligonucleotide sequence motif
aatttatgcctaca

SEQ ID NO: 215 - DNA, 13 bp, Artificial Sequence
  oligonucleotide sequence motif
aatttatgcctac

SEQ ID NO: 216 - DNA, 13 bp, Artificial Sequence
  oligonucleotide sequence motif
ccaatttatgcct

SEQ ID NO: 217 - DNA, 15 bp, Artificial Sequence
  oligonucleotide sequence motif
gcttggaggcttgaa

SEQ ID NO: 218 - DNA, 16 bp, Artificial Sequence
  oligonucleotide sequence motif
agcttggaggcttgaa

SEQ ID NO: 219 - DNA, 14 bp, Artificial Sequence
  oligonucleotide sequence motif
gcttggaggcttga

SEQ ID NO: 220 - DNA, 15 bp, Artificial Sequence
  oligonucleotide sequence motif
agcttggaggcttga

SEQ ID NO: 221 - DNA, 16 bp, Artificial Sequence
  oligonucleotide sequence motif
cagcttggaggcttga

SEQ ID NO: 222 - DNA, 13 bp, Artificial Sequence
  oligonucleotide sequence motif
gcttggaggcttg

SEQ ID NO: 223 - DNA, 14 bp, Artificial Sequence
  oligonucleotide sequence motif
agcttggaggcttg

SEQ ID NO: 224 - DNA, 15 bp, Artificial Sequence
  oligonucleotide sequence motif
cagcttggaggcttg

SEQ ID NO: 225 - DNA, 16 bp, Artificial Sequence
  oligonucleotide sequence motif
acagcttggaggcttg

SEQ ID NO: 226 - DNA, 16 bp, Artificial Sequence
  oligonucleotide sequence motif
cacagcttggaggctt

SEQ ID NO: 227 - DNA, 15 bp, Artificial Sequence
  oligonucleotide sequence motif
cacagcttggaggct

SEQ ID NO: 228 - DNA, 16 bp, Artificial Sequence
  oligonucleotide sequence motif
gcacagcttggaggct

SEQ ID NO: 229 - DNA, 15 bp, Artificial Sequence
  oligonucleotide sequence motif
gcacagcttggaggc

SEQ ID NO: 230 - DNA, 16 bp, Artificial Sequence
  oligonucleotide sequence motif
ggcacagcttggaggc

SEQ ID NO: 231 - DNA, 16 bp, Artificial Sequence
  oligonucleotide sequence motif
aggcacagcttggagg

SEQ ID NO: 232 - DNA, 15 bp, Artificial Sequence
  oligonucleotide sequence motif
aggcacagcttggag

SEQ ID NO: 233 - DNA, 16 bp, Artificial Sequence
  oligonucleotide sequence motif
aaggcacagcttggag

SEQ ID NO: 234 - DNA, 15 bp, Artificial Sequence
  oligonucleotide sequence motif
aaggcacagcttgga

SEQ ID NO: 235 - DNA, 16 bp, Artificial Sequence
  oligonucleotide sequence motif
caaggcacagcttgga

SEQ ID NO: 236 - DNA, 14 bp, Artificial Sequence
  oligonucleotide sequence motif
aaggcacagcttgg

SEQ ID NO: 237 - DNA, 15 bp, Artificial Sequence
  oligonucleotide sequence motif
caaggcacagcttgg

SEQ ID NO: 238 - DNA, 16 bp, Artificial Sequence
  oligonucleotide sequence motif
ccaaggcacagcttgg

SEQ ID NO: 239 - DNA, 14 bp, Artificial Sequence
  oligonucleotide sequence motif
caaggcacagcttg

SEQ ID NO: 240 - DNA, 15 bp, Artificial Sequence
  oligonucleotide sequence motif
ccaaggcacagcttg

SEQ ID NO: 241 - DNA, 14 bp, Artificial Sequence
  oligonucleotide sequence motif
ccaaggcacagctt

SEQ ID NO: 242 - DNA, 13 bp, Artificial Sequence
  oligonucleotide sequence motif
tgcgaatccacac

SEQ ID NO: 243 - DNA, 14 bp, Artificial Sequence
  oligonucleotide sequence motif
gtgcgaatccacac

SEQ ID NO: 244 - DNA, 15 bp, Artificial Sequence
  oligonucleotide sequence motif
ggagttcttcttcta

SEQ ID NO: 245 - DNA, 16 bp, Artificial Sequence
  oligonucleotide sequence motif
gggagttcttcttcta

SEQ ID NO: 246 - DNA, 15 bp, Artificial Sequence
  oligonucleotide sequence motif
gggagttcttcttct

SEQ ID NO: 247 - DNA, 16 bp, Artificial Sequence
  oligonucleotide sequence motif
agggagttcttcttct

SEQ ID NO: 248 - DNA, 15 bp, Artificial Sequence
  oligonucleotide sequence motif
agggagttcttcttc

SEQ ID NO: 249 - DNA, 16 bp, Artificial Sequence
  oligonucleotide sequence motif
gagggagttcttcttc

SEQ ID NO: 250 - DNA, 14 bp, Artificial Sequence
  oligonucleotide sequence motif
agggagttcttctt

SEQ ID NO: 251 - DNA, 15 bp, Artificial Sequence
  oligonucleotide sequence motif
gagggagttcttctt

SEQ ID NO: 252 - DNA, 16 bp, Artificial Sequence
  oligonucleotide sequence motif
cgagggagttcttctt

SEQ ID NO: 253 - DNA, 15 bp, Artificial Sequence
  oligonucleotide sequence motif
cgagggagttcttct

SEQ ID NO: 254 - DNA, 16 bp, Artificial Sequence
  oligonucleotide sequence motif
gcgagggagttcttct

SEQ ID NO: 255 - DNA, 15 bp, Artificial Sequence
  oligonucleotide sequence motif
gcgagggagttcttc

SEQ ID NO: 256 - DNA, 16 bp, Artificial Sequence
  oligonucleotide sequence motif
ggcgagggagttcttc

SEQ ID NO: 257 - DNA, 14 bp, Artificial Sequence
  oligonucleotide sequence motif
gcgagggagttctt

SEQ ID NO: 258 - DNA, 15 bp, Artificial Sequence
  oligonucleotide sequence motif
ggcgagggagttctt

SEQ ID NO: 259 - DNA, 16 bp, Artificial Sequence
  oligonucleotide sequence motif
aggcgagggagttctt

SEQ ID NO: 260 - DNA, 13 bp, Artificial Sequence
  oligonucleotide sequence motif
gcgagggagttct

SEQ ID NO: 261 - DNA, 14 bp, Artificial Sequence
  oligonucleotide sequence motif
ggcgagggagttct

SEQ ID NO: 262 - DNA, 15 bp, Artificial Sequence
  oligonucleotide sequence motif
aggcgagggagttct

SEQ ID NO: 263 - DNA, 16 bp, Artificial Sequence
  oligonucleotide sequence motif
gaggcgagggagttct

SEQ ID NO: 264 - DNA, 13 bp, Artificial Sequence
  oligonucleotide sequence motif
ggcgagggagttc

SEQ ID NO: 265 - DNA, 14 bp, Artificial Sequence
  oligonucleotide sequence motif
aggcgagggagttc

SEQ ID NO: 266 - DNA, 15 bp, Artificial Sequence
  oligonucleotide sequence motif
gaggcgagggagttc

SEQ ID NO: 267 - DNA, 16 bp, Artificial Sequence
  oligonucleotide sequence motif
cgaggcgagggagttc

SEQ ID NO: 268 - DNA, 13 bp, Artificial Sequence
  oligonucleotide sequence motif
aggcgagggagtt

SEQ ID NO: 269 - DNA, 14 bp, Artificial Sequence
  oligonucleotide sequence motif
gaggcgagggagtt

SEQ ID NO: 270 - DNA, 15 bp, Artificial Sequence
  oligonucleotide sequence motif
cgaggcgagggagtt

SEQ ID NO: 271 - DNA, 16 bp, Artificial Sequence
  oligonucleotide sequence motif
gcgaggcgagggagtt

SEQ ID NO: 272 - DNA, 13 bp, Artificial Sequence
  oligonucleotide sequence motif
gaggcgagggagt

SEQ ID NO: 273 - DNA, 14 bp, Artificial Sequence
  oligonucleotide sequence motif
cgaggcgagggagt

SEQ ID NO: 274 - DNA, 15 bp, Artificial Sequence
  oligonucleotide sequence motif
gcgaggcgagggagt

SEQ ID NO: 275 - DNA, 16 bp, Artificial Sequence
  oligonucleotide sequence motif
tgcgaggcgagggagt

SEQ ID NO: 276 - DNA, 13 bp, Artificial Sequence
  oligonucleotide sequence motif
cgaggcgagggag

SEQ ID NO: 277 - DNA, 14 bp, Artificial Sequence
  oligonucleotide sequence motif
gcgaggcgagggag

SEQ ID NO: 278 - DNA, 15 bp, Artificial Sequence
  oligonucleotide sequence motif
tgcgaggcgagggag

SEQ ID NO: 279 - DNA, 16 bp, Artificial Sequence
  oligonucleotide sequence motif
ctgcgaggcgagggag

SEQ ID NO: 280 - DNA, 12 bp, Artificial Sequence
  oligonucleotide sequence motif
cgaggcgaggga

SEQ ID NO: 281 - DNA, 13 bp, Artificial Sequence
  oligonucleotide sequence motif
gcgaggcgaggga

SEQ ID NO: 282 - DNA, 14 bp, Artificial Sequence
  oligonucleotide sequence motif
tgcgaggcgaggga

SEQ ID NO: 283 - DNA, 15 bp, Artificial Sequence
  oligonucleotide sequence motif
ctgcgaggcgaggga

SEQ ID NO: 284 - DNA, 16 bp, Artificial Sequence
  oligonucleotide sequence motif
tctgcgaggcgaggga

SEQ ID NO: 285 - DNA, 15 bp, Artificial Sequence
  oligonucleotide sequence motif
tctgcgaggcgaggg

SEQ ID NO: 286 - DNA, 16 bp, Artificial Sequence
  oligonucleotide sequence motif
gtctgcgaggcgaggg

SEQ ID NO: 287 - DNA, 14 bp, Artificial Sequence
  oligonucleotide sequence motif
gttcccaagaatat

SEQ ID NO: 288 - DNA, 15 bp, Artificial Sequence
  oligonucleotide sequence motif
tgttcccaagaatat

SEQ ID NO: 289 - DNA, 13 bp, Artificial Sequence
  oligonucleotide sequence motif
gttcccaagaata

SEQ ID NO: 290 - DNA, 14 bp, Artificial Sequence
  oligonucleotide sequence motif
tgttcccaagaata

SEQ ID NO: 291 - DNA, 15 bp, Artificial Sequence
  oligonucleotide sequence motif
ttgttcccaagaata

SEQ ID NO: 292 - DNA, 13 bp, Artificial Sequence
  oligonucleotide sequence motif
tgttcccaagaat

SEQ ID NO: 293 - DNA, 14 bp, Artificial Sequence
  oligonucleotide sequence motif
ttgttcccaagaat

SEQ ID NO: 294 - DNA, 15 bp, Artificial Sequence
  LNA antisense gapmer oligonucleotide
  phosphorothiate Internucleoside linkages (1)..(15)
  LNA nucleosides (1)..(3)
  LNA nucleosides (13)..(15)
gaaccactgaacaaa

SEQ ID NO: 295 - DNA, 16 bp, Artificial Sequence
  LNA antisense gapmer oligonucleotide
  phosphorothiate Internucleoside linkages (1)..(16)
  LNA nucleosides (1)..(3)
  LNA nucleosides (14)..(16)
cgaaccactgaacaaa

SEQ ID NO: 296 - DNA, 15 bp, Artificial Sequence
  LNA antisense gapmer oligonucleotide
  phosphorothiate Internucleoside linkages (1)..(15)
  LNA nucleosides (1)..(3)
  LNA nucleosides (13)..(15)
cgaaccactgaacaa

SEQ ID NO: 297 - DNA, 14 bp, Artificial Sequence
  LNA antisense gapmer oligonucleotide
  phosphorothiate Internucleoside linkages (1)..(14)
  LNA nucleosides (1)..(3)
  LNA nucleosides (12)..(14)
cgaaccactgaaca

SEQ ID NO: 298 - DNA, 13 bp, Artificial Sequence
  LNA antisense gapmer oligonucleotide
  phosphorothiate Internucleoside linkages (1)..(13)
  LNA nucleosides (1)..(3)
  LNA nucleosides (12)..(13)
cgaaccactgaac

SEQ ID NO: 299 - DNA, 15 bp, Artificial Sequence
  LNA antisense gapmer oligonucleotide
  phosphorothiate Internucleoside linkages (1)..(15)
  LNA nucleosides (1)..(3)
  LNA nucleosides (13)..(15)
ccgcagtatggatcg

SEQ ID NO: 300 - DNA, 13 bp, Artificial Sequence
  LNA antisense gapmer oligonucleotide
  phosphorothiate Internucleoside linkages (1)..(13)
  LNA nucleosides (1)..(3)
  LNA nucleosides (12)..(13)
cgcagtatggatc

SEQ ID NO: 301 - DNA, 14 bp, Artificial Sequence
  LNA antisense gapmer oligonucleotide
  phosphorothiate Internucleoside linkages (1)..(14)
  LNA nucleosides (1)..(3)
  LNA nucleosides (12)..(14)
gcgtaaagagaggt

SEQ ID NO: 302 - DNA, 15 bp, Artificial Sequence
  LNA antisense gapmer oligonucleotide
  phosphorothiate Internucleoside linkages (1)..(15)
  LNA nucleosides (1)..(3)
  LNA nucleosides (13)..(15)
cgcgtaaagagaggt

SEQ ID NO: 303 - DNA, 13 bp, Artificial Sequence
  LNA antisense gapmer oligonucleotide
  phosphorothiate Internucleoside linkages (1)..(13)
  LNA nucleosides (1)..(3)
  LNA nucleosides (12)..(13)
gcgtaaagagagg

SEQ ID NO: 304 - DNA, 15 bp, Artificial Sequence
  LNA antisense gapmer oligonucleotide
  phosphorothiate Internucleoside linkages (1)..(15)
  LNA nucleosides (1)..(3)
  LNA nucleosides (13)..(15)
agaaggcacagacgg

SEQ ID NO: 305 - DNA, 16 bp, Artificial Sequence
  LNA antisense gapmer oligonucleotide
  phosphorothiate Internucleoside linkages (1)..(16)
  LNA nucleosides (1)..(3)
  LNA nucleosides (14)..(16)
gagaaggcacagacgg

SEQ ID NO: 306 - DNA, 13 bp, Artificial Sequence
  LNA antisense gapmer oligonucleotide
  phosphorothiate Internucleoside linkages (1)..(13)
  LNA nucleosides (1)..(3)
  5-methyl c (11)..(11)
  LNA nucleosides (12)..(13)
gaagtgcacacgg

SEQ ID NO: 307 - DNA, 15 bp, Artificial Sequence
  LNA antisense gapmer oligonucleotide
  phosphorothiate Internucleoside linkages (1)..(15)
  LNA nucleosides (1)..(3)
  LNA nucleosides (13)..(15)
gcgaagtgcacacgg

SEQ ID NO: 308 - DNA, 16 bp, Artificial Sequence
  LNA antisense gapmer oligonucleotide
  phosphorothiate Internucleoside linkages (1)..(16)
  LNA nucleosides (1)..(3)
  LNA nucleosides (14)..(16)
agcgaagtgcacacgg

SEQ ID NO: 309 - DNA, 13 bp, Artificial Sequence
  LNA antisense gapmer oligonucleotide
  phosphorothiate Internucleoside linkages (1)..(13)
  LNA nucleosides (1)..(3)
  LNA nucleosides (12)..(13)
cgaagtgcacacg

SEQ ID NO: 310 - DNA, 15 bp, Artificial Sequence
  LNA antisense gapmer oligonucleotide
  phosphorothiate Internucleoside linkages (1)..(15)
  LNA nucleosides (1)..(3)
  LNA nucleosides (13)..(15)
agcgaagtgcacacg

SEQ ID NO: 311 - DNA, 16 bp, Artificial Sequence
  LNA antisense gapmer oligonucleotide
  phosphorothiate Internucleoside linkages (1)..(16)
  LNA nucleosides (1)..(3)
  5-methyl c (4)..(4)
  LNA nucleosides (14)..(16)
aagcgaagtgcacacg

SEQ ID NO: 312 - DNA, 15 bp, Artificial Sequence
  LNA antisense gapmer oligonucleotide
  phosphorothiate Internucleoside linkages (1)..(15)
  LNA nucleosides (1)..(3)
  5-methyl c (5)..(5)
  LNA nucleosides (13)..(15)
gaagcgaagtgcaca

SEQ ID NO: 313 - DNA, 16 bp, Artificial Sequence
  LNA antisense gapmer oligonucleotide
  phosphorothiate Internucleoside linkages (1)..(16)
  LNA nucleosides (1)..(3)
  5-methyl c (8)..(8)
  LNA nucleosides (14)..(16)
ggtgaagcgaagtgca

SEQ ID NO: 314 - DNA, 15 bp, Artificial Sequence
  LNA antisense gapmer oligonucleotide
  phosphorothiate Internucleoside linkages (1)..(15)
  LNA nucleosides (1)..(3)
  5-methyl c (8)..(8)
  LNA nucleosides (13)..(15)
ggtgaagcgaagtgc

SEQ ID NO: 315 - DNA, 16 bp, Artificial Sequence
  LNA antisense gapmer oligonucleotide
  phosphorothiate Internucleoside linkages (1)..(16)
  LNA nucleosides (1)..(3)
  5-methyl c (9)..(9)
  LNA nucleosides (14)..(16)
aggtgaagcgaagtgc

SEQ ID NO: 316 - DNA, 15 bp, Artificial Sequence
  LNA antisense gapmer oligonucleotide
  phosphorothiate Internucleoside linkages (1)..(15)
  LNA nucleosides (1)..(3)
  5-methyl c (9)..(9)
  LNA nucleosides (13)..(15)
aggtgaagcgaagtg

SEQ ID NO: 317 - DNA, 14 bp, Artificial Sequence
  LNA antisense gapmer oligonucleotide
  phosphorothiate Internucleoside linkages (1)..(14)
  LNA nucleosides (1)..(3)
  5-methyl c (9)..(9)
  LNA nucleosides (12)..(14)
aggtgaagcgaagt

SEQ ID NO: 318 - DNA, 14 bp, Artificial Sequence
  LNA antisense gapmer oligonucleotide
  phosphorothiate Internucleoside linkages (1)..(14)
  LNA nucleosides (1)..(3)
  LNA nucleosides (12)..(14)
cagaggtgaagcga

SEQ ID NO: 319 - DNA, 14 bp, Artificial Sequence
  LNA antisense gapmer oligonucleotide
  phosphorothiate Internucleoside linkages (1)..(14)
  LNA nucleosides (1)..(3)
  5-methyl c (8)..(8)
  LNA nucleosides (12)..(14)
aaaaccccgcctgt

SEQ ID NO: 320 - DNA, 13 bp, Artificial Sequence
  LNA antisense gapmer oligonucleotide
  phosphorothiate Internucleoside linkages (1)..(13)
  LNA nucleosides (1)..(3)
  5-methyl c (8)..(8)
  LNA nucleosides (12)..(13)
aaaaccccgcctg

SEQ ID NO: 321 - DNA, 15 bp, Artificial Sequence
  LNA antisense gapmer oligonucleotide
  phosphorothiate Internucleoside linkages (1)..(15)
  LNA nucleosides (1)..(3)
  LNA nucleosides (13)..(15)
acgagtctagactct

SEQ ID NO: 322 - DNA, 16 bp, Artificial Sequence
  LNA antisense gapmer oligonucleotide
  phosphorothiate Internucleoside linkages (1)..(16)
  LNA nucleosides (1)..(3)
  LNA nucleosides (14)..(16)
cacgagtctagactct

SEQ ID NO: 323 - DNA, 14 bp, Artificial Sequence
  LNA antisense gapmer oligonucleotide
  phosphorothiate Internucleoside linkages (1)..(14)
  LNA nucleosides (1)..(3)
  LNA nucleosides (12)..(14)
acgagtctagactc

SEQ ID NO: 324 - DNA, 15 bp, Artificial Sequence
  LNA antisense gapmer oligonucleotide
  phosphorothiate Internucleoside linkages (1)..(15)
  LNA nucleosides (1)..(3)
  LNA nucleosides (13)..(15)
cacgagtctagactc

SEQ ID NO: 325 - DNA, 16 bp, Artificial Sequence
  LNA antisense gapmer oligonucleotide
  phosphorothiate Internucleoside linkages (1)..(16)
  LNA nucleosides (1)..(3)
  5-methyl c (4)..(4)
  LNA nucleosides (14)..(16)
ccacgagtctagactc

SEQ ID NO: 326 - DNA, 13 bp, Artificial Sequence
  LNA antisense gapmer oligonucleotide
  phosphorothiate Internucleoside linkages (1)..(13)
  LNA nucleosides (1)..(3)
  LNA nucleosides (12)..(13)
acgagtctagact

SEQ ID NO: 327 - DNA, 14 bp, Artificial Sequence
  LNA antisense gapmer oligonucleotide
  phosphorothiate Internucleoside linkages (1)..(14)
  LNA nucleosides (1)..(3)
  LNA nucleosides (12)..(14)
cacgagtctagact

SEQ ID NO: 328 - DNA, 15 bp, Artificial Sequence
  LNA antisense gapmer oligonucleotide
  phosphorothiate Internucleoside linkages (1)..(15)
  LNA nucleosides (1)..(3)
  5-methyl c (4)..(4)
  LNA nucleosides (13)..(15)
ccacgagtctagact

SEQ ID NO: 329 - DNA, 16 bp, Artificial Sequence
  LNA antisense gapmer oligonucleotide
  phosphorothiate Internucleoside linkages (1)..(16)
  LNA nucleosides (1)..(3)
  5-methyl c (5)..(5)
  LNA nucleosides (14)..(16)
accacgagtctagact

SEQ ID NO: 330 - DNA, 12 bp, Artificial Sequence
  LNA antisense gapmer oligonucleotide
  phosphorothiate Internucleoside linkages (1)..(12)
  LNA nucleosides (1)..(2)
  LNA nucleosides (11)..(12)
acgagtctagac

SEQ ID NO: 331 - DNA, 13 bp, Artificial Sequence
  LNA antisense gapmer oligonucleotide
  phosphorothiate Internucleoside linkages (1)..(13)
  LNA nucleosides (1)..(3)
  LNA nucleosides (12)..(13)
cacgagtctagac

SEQ ID NO: 332 - DNA, 14 bp, Artificial Sequence
  LNA antisense gapmer oligonucleotide
  phosphorothiate Internucleoside linkages (1)..(14)
  LNA nucleosides (1)..(3)
  5-methyl c (4)..(4)
  LNA nucleosides (12)..(14)
ccacgagtctagac

SEQ ID NO: 333 - DNA, 15 bp, Artificial Sequence
  LNA antisense gapmer oligonucleotide
  phosphorothiate Internucleoside linkages (1)..(15)
  LNA nucleosides (1)..(3)
  5-methyl c (5)..(5)
  LNA nucleosides (13)..(15)
accacgagtctagac

SEQ ID NO: 334 - DNA, 16 bp, Artificial Sequence
  LNA antisense gapmer oligonucleotide
  phosphorothiate Internucleoside linkages (1)..(16)
  LNA nucleosides (1)..(3)
  5-methyl c (6)..(6)
  LNA nucleosides (14)..(16)
caccacgagtctagac

SEQ ID NO: 335 - DNA, 14 bp, Artificial Sequence
  LNA antisense gapmer oligonucleotide
  phosphorothiate Internucleoside linkages (1)..(14)
  LNA nucleosides (1)..(3)
  5-methyl c (5)..(5)
  LNA nucleosides (12)..(14)
accacgagtctaga

SEQ ID NO: 336 - DNA, 15 bp, Artificial Sequence
  LNA antisense gapmer oligonucleotide
  phosphorothiate Internucleoside linkages (1)..(15)
  LNA nucleosides (1)..(3)
  5-methyl c (6)..(6)
  LNA nucleosides (13)..(15)
caccacgagtctaga

SEQ ID NO: 337 - DNA, 16 bp, Artificial Sequence
  LNA antisense gapmer oligonucleotide
  phosphorothiate Internucleoside linkages (1)..(16)
  LNA nucleosides (1)..(3)
  5-methyl c (7)..(7)
  LNA nucleosides (14)..(16)
ccaccacgagtctaga

SEQ ID NO: 338 - DNA, 15 bp, Artificial Sequence
  LNA antisense gapmer oligonucleotide
  phosphorothiate Internucleoside linkages (1)..(15)
  LNA nucleosides (1)..(3)
  5-methyl c (7)..(7)
  LNA nucleosides (13)..(15)
ccaccacgagtctag

SEQ ID NO: 339 - DNA, 16 bp, Artificial Sequence
  LNA antisense gapmer oligonucleotide
  phosphorothiate Internucleoside linkages (1)..(16)
  LNA nucleosides (1)..(3)
  5-methyl c (8)..(8)
  LNA nucleosides (14)..(16)
tccaccacgagtctag

SEQ ID NO: 340 - DNA, 14 bp, Artificial Sequence
  LNA antisense gapmer oligonucleotide
  phosphorothiate Internucleoside linkages (1)..(14)
  LNA nucleosides (1)..(3)
  5-methyl c (7)..(7)
  LNA nucleosides (12)..(14)
ccaccacgagtcta

SEQ ID NO: 341 - DNA, 15 bp, Artificial Sequence
  LNA antisense gapmer oligonucleotide
  phosphorothiate Internucleoside linkages (1)..(15)
  LNA nucleosides (1)..(3)
  5-methyl c (8)..(8)
  LNA nucleosides (13)..(15)
tccaccacgagtcta

SEQ ID NO: 342 - DNA, 16 bp, Artificial Sequence
  LNA antisense gapmer oligonucleotide
  phosphorothiate Internucleoside linkages (1)..(16)
  LNA nucleosides (1)..(3)
  5-methyl c (9)..(9)
  LNA nucleosides (14)..(16)
gtccaccacgagtcta

SEQ ID NO: 343 - DNA, 14 bp, Artificial Sequence
  LNA antisense gapmer oligonucleotide
  phosphorothiate Internucleoside linkages (1)..(14)
  LNA nucleosides (1)..(3)
  5-methyl c (8)..(8)
  LNA nucleosides (12)..(14)
tccaccacgagtct

SEQ ID NO: 344 - DNA, 15 bp, Artificial Sequence
  LNA antisense gapmer oligonucleotide
  phosphorothiate Internucleoside linkages (1)..(15)
  LNA nucleosides (1)..(3)
  5-methyl c (9)..(9)
  LNA nucleosides (13)..(15)
gtccaccacgagtct

SEQ ID NO: 345 - DNA, 16 bp, Artificial Sequence
  LNA antisense gapmer oligonucleotide
  phosphorothiate Internucleoside linkages (1)..(16)
  LNA nucleosides (1)..(3)
  5-methyl c (10)..(10)
  LNA nucleosides (14)..(16)
agtccaccacgagtct

SEQ ID NO: 346 - DNA, 14 bp, Artificial Sequence
  LNA antisense gapmer oligonucleotide
  phosphorothiate Internucleoside linkages (1)..(14)
  LNA nucleosides (1)..(3)
  5-methyl c (9)..(9)
  LNA nucleosides (12)..(14)
gtccaccacgagtc

SEQ ID NO: 347 - DNA, 15 bp, Artificial Sequence
  LNA antisense gapmer oligonucleotide
  phosphorothiate Internucleoside linkages (1)..(15)
  LNA nucleosides (1)..(3)
  5-methyl c (10)..(10)
  LNA nucleosides (13)..(15)
agtccaccacgagtc

SEQ ID NO: 348 - DNA, 16 bp, Artificial Sequence
  LNA antisense gapmer oligonucleotide
  phosphorothiate Internucleoside linkages (1)..(16)
  LNA nucleosides (1)..(3)
  5-methyl c (11)..(11)
  LNA nucleosides (14)..(16)
aagtccaccacgagtc

SEQ ID NO: 349 - DNA, 14 bp, Artificial Sequence
  LNA antisense gapmer oligonucleotide
  phosphorothiate Internucleoside linkages (1)..(14)
  LNA nucleosides (1)..(3)
  5-methyl c (10)..(10)
  LNA nucleosides (12)..(14)
agtccaccacgagt

SEQ ID NO: 350 - DNA, 15 bp, Artificial Sequence
  LNA antisense gapmer oligonucleotide
  phosphorothiate Internucleoside linkages (1)..(15)
  LNA nucleosides (1)..(3)
  5-methyl c (11)..(11)
  LNA nucleosides (13)..(15)
aagtccaccacgagt

SEQ ID NO: 351 - DNA, 16 bp, Artificial Sequence
  LNA antisense gapmer oligonucleotide
  phosphorothiate Internucleoside linkages (1)..(16)
  LNA nucleosides (1)..(3)
  5-methyl c (12)..(12)
  LNA nucleosides (14)..(16)
gaagtccaccacgagt

SEQ ID NO: 352 - DNA, 14 bp, Artificial Sequence
  LNA antisense gapmer oligonucleotide
  phosphorothiate Internucleoside linkages (1)..(14)
  LNA nucleosides (1)..(3)
  5-methyl c (11)..(11)
  LNA nucleosides (13)..(14)
aagtccaccacgag

SEQ ID NO: 353 - DNA, 15 bp, Artificial Sequence
  LNA antisense gapmer oligonucleotide
  phosphorothiate Internucleoside linkages (1)..(15)
  LNA nucleosides (1)..(3)
  5-methyl c (12)..(12)
  LNA nucleosides (14)..(15)
gaagtccaccacgag

SEQ ID NO: 354 - DNA, 16 bp, Artificial Sequence
  LNA antisense gapmer oligonucleotide
  phosphorothiate Internucleoside linkages (1)..(16)
  LNA nucleosides (1)..(3)
  5-methyl c (13)..(13)
  LNA nucleosides (15)..(16)
agaagtccaccacgag

SEQ ID NO: 355 - DNA, 15 bp, Artificial Sequence
  LNA antisense gapmer oligonucleotide
  phosphorothiate Internucleoside linkages (1)..(15)
  LNA nucleosides (1)..(3)
  LNA nucleosides (13)..(15)
agaagtccaccacga

SEQ ID NO: 356 - DNA, 16 bp, Artificial Sequence
  LNA antisense gapmer oligonucleotide
  phosphorothiate Internucleoside linkages (1)..(16)
  LNA nucleosides (1)..(3)
  LNA nucleosides (14)..(16)
gagaagtccaccacga

SEQ ID NO: 357 - DNA, 15 bp, Artificial Sequence
  LNA antisense gapmer oligonucleotide
  phosphorothiate Internucleoside linkages (1)..(15)
  LNA nucleosides (1)..(3)
  LNA nucleosides (13)..(15)
gagaagtccaccacg

SEQ ID NO: 358 - DNA, 16 bp, Artificial Sequence
  LNA antisense gapmer oligonucleotide
  phosphorothiate Internucleoside linkages (1)..(16)
  LNA nucleosides (1)..(3)
  LNA nucleosides (14)..(16)
agagaagtccaccacg

SEQ ID NO: 359 - DNA, 16 bp, Artificial Sequence
  LNA antisense gapmer oligonucleotide
  phosphorothiate Internucleoside linkages (1)..(16)
  LNA nucleosides (1)..(3)
  LNA nucleosides (14)..(16)
gagagaagtccaccac

SEQ ID NO: 360 - DNA, 15 bp, Artificial Sequence
  LNA antisense gapmer oligonucleotide
  phosphorothiate Internucleoside linkages (1)..(15)
  LNA nucleosides (1)..(3)
  LNA nucleosides (13)..(15)
gagagaagtccacca

SEQ ID NO: 361 - DNA, 16 bp, Artificial Sequence
  LNA antisense gapmer oligonucleotide
  phosphorothiate Internucleoside linkages (1)..(16)
  LNA nucleosides (1)..(3)
  LNA nucleosides (14)..(16)
tgagagaagtccacca

SEQ ID NO: 362 - DNA, 14 bp, Artificial Sequence
  LNA antisense gapmer oligonucleotide
  phosphorothiate Internucleoside linkages (1)..(14)
  LNA nucleosides (1)..(3)
  LNA nucleosides (12)..(14)
gagagaagtccacc

SEQ ID NO: 363 - DNA, 15 bp, Artificial Sequence
  LNA antisense gapmer oligonucleotide
  phosphorothiate Internucleoside linkages (1)..(15)
  LNA nucleosides (1)..(3)
  LNA nucleosides (13)..(15)
tgagagaagtccacc

SEQ ID NO: 364 - DNA, 14 bp, Artificial Sequence
  LNA antisense gapmer oligonucleotide
  phosphorothiate Internucleoside linkages (1)..(14)
  LNA nucleosides (1)..(3)
  LNA nucleosides (12)..(14)
tgagagaagtccac

SEQ ID NO: 365 - DNA, 13 bp, Artificial Sequence
  LNA antisense gapmer oligonucleotide
  phosphorothiate Internucleoside linkages (1)..(13)
  LNA nucleosides (1)..(3)
  5-methyl c (5)..(5)
  5-methyl c (8)..(8)
  LNA nucleosides (12)..(13)
aaaacgccgcaga

SEQ ID NO: 366 - DNA, 14 bp, Artificial Sequence
  LNA antisense gapmer oligonucleotide
  phosphorothiate Internucleoside linkages (1)..(14)
  LNA nucleosides (1)..(3)
  5-methyl c (6)..(6)
  5-methyl c (9)..(9)
  LNA nucleosides (12)..(14)
taaaacgccgcaga

SEQ ID NO: 367 - DNA, 15 bp, Artificial Sequence
  LNA antisense gapmer oligonucleotide
  phosphorothiate Internucleoside linkages (1)..(15)
  LNA nucleosides (1)..(3)
  5-methyl c (7)..(7)
  5-methyl c (10)..(10)
  LNA nucleosides (13)..(15)
ataaaacgccgcaga

SEQ ID NO: 368 - DNA, 16 bp, Artificial Sequence
  LNA antisense gapmer oligonucleotide
  phosphorothiate Internucleoside linkages (1)..(16)
  LNA nucleosides (1)..(3)
  5-methyl c (8)..(8)
  5-methyl c (11)..(11)
  LNA nucleosides (14)..(16)
gataaaacgccgcaga

SEQ ID NO: 369 - DNA, 14 bp, Artificial Sequence
  LNA antisense gapmer oligonucleotide
  phosphorothiate Internucleoside linkages (1)..(14)
  LNA nucleosides (1)..(3)
  5-methyl c (7)..(7)
  5-methyl c (10)..(10)
  LNA nucleosides (12)..(14)
ataaaacgccgcag

SEQ ID NO: 370 - DNA, 15 bp, Artificial Sequence
  LNA antisense gapmer oligonucleotide
  phosphorothiate Internucleoside linkages (1)..(15)
  LNA nucleosides (1)..(3)
  5-methyl c (8)..(8)
  5-methyl c (11)..(11)
  LNA nucleosides (13)..(15)
gataaaacgccgcag

SEQ ID NO: 371 - DNA, 16 bp, Artificial Sequence
  LNA antisense gapmer oligonucleotide
  phosphorothiate Internucleoside linkages (1)..(16)
  LNA nucleosides (1)..(3)
  5-methyl c (9)..(9)
  5-methyl c (12)..(12)
  LNA nucleosides (14)..(16)
tgataaaacgccgcag

SEQ ID NO: 372 - DNA, 13 bp, Artificial Sequence
  LNA antisense gapmer oligonucleotide
  phosphorothiate Internucleoside linkages (1)..(13)
  LNA nucleosides (1)..(3)
  5-methyl c (7)..(7)
  5-methyl c (10)..(10)
  LNA nucleosides (12)..(13)
ataaaacgccgca

SEQ ID NO: 373 - DNA, 14 bp, Artificial Sequence
  LNA antisense gapmer oligonucleotide
  phosphorothiate Internucleoside linkages (1)..(14)
  LNA nucleosides (1)..(3)
  5-methyl c (8)..(8)
  5-methyl c (11)..(11)
  LNA nucleosides (12)..(14)
gataaaacgccgca

SEQ ID NO: 374 - DNA, 15 bp, Artificial Sequence
  LNA antisense gapmer oligonucleotide
  phosphorothiate Internucleoside linkages (1)..(15)
  LNA nucleosides (1)..(3)
  5-methyl c (9)..(9)
  5-methyl c (12)..(12)
  LNA nucleosides (13)..(15)
tgataaaacgccgca

SEQ ID NO: 375 - DNA, 16 bp, Artificial Sequence
  LNA antisense gapmer oligonucleotide
  phosphorothiate Internucleoside linkages (1)..(16)
  LNA nucleosides (1)..(3)
  5-methyl c (10)..(10)
  5-methyl c (13)..(13)
  LNA nucleosides (14)..(16)
atgataaaacgccgca

SEQ ID NO: 376 - DNA, 12 bp, Artificial Sequence
  LNA antisense gapmer oligonucleotide
  phosphorothiate Internucleoside linkages (1)..(12)
  LNA nucleosides (1)..(2)
  5-methyl c (7)..(7)
  5-methyl c (10)..(10)
  LNA nucleosides (11)..(12)
ataaaacgccgc

SEQ ID NO: 377 - DNA, 13 bp, Artificial Sequence
  LNA antisense gapmer oligonucleotide
  phosphorothiate Internucleoside linkages (1)..(13)
  LNA nucleosides (1)..(3)
  5-methyl c (8)..(8)
  5-methyl c (11)..(11)
  LNA nucleosides (12)..(13)
gataaaacgccgc

SEQ ID NO: 378 - DNA, 14 bp, Artificial Sequence
  LNA antisense gapmer oligonucleotide
  phosphorothiate Internucleoside linkages (1)..(14)
  LNA nucleosides (1)..(3)
  5-methyl c (9)..(9)
  LNA nucleosides (12)..(14)
tgataaaacgccgc

SEQ ID NO: 379 - DNA, 15 bp, Artificial Sequence
  LNA antisense gapmer oligonucleotide
  phosphorothiate Internucleoside linkages (1)..(15)
  LNA nucleosides (1)..(3)
  5-methyl c (10)..(10)
  LNA nucleosides (13)..(15)
atgataaaacgccgc

SEQ ID NO: 380 - DNA, 12 bp, Artificial Sequence
  LNA antisense gapmer oligonucleotide
  phosphorothiate Internucleoside linkages (1)..(12)
  LNA nucleosides (1)..(2)
  5-methyl c (8)..(8)
  LNA nucleosides (11)..(12)
gataaaacgccg

SEQ ID NO: 381 - DNA, 13 bp, Artificial Sequence
  LNA antisense gapmer oligonucleotide
  phosphorothiate Internucleoside linkages (1)..(13)
  LNA nucleosides (1)..(3)
  5-methyl c (9)..(9)
  LNA nucleosides (12)..(13)
tgataaaacgccg

SEQ ID NO: 382 - DNA, 14 bp, Artificial Sequence
  LNA antisense gapmer oligonucleotide
  phosphorothiate Internucleoside linkages (1)..(14)
  LNA nucleosides (1)..(3)
  5-methyl c (10)..(10)
  LNA nucleosides (12)..(14)
atgataaaacgccg

SEQ ID NO: 383 - DNA, 12 bp, Artificial Sequence
  LNA antisense gapmer oligonucleotide
  phosphorothiate Internucleoside linkages (1)..(12)
  LNA nucleosides (1)..(2)
  5-methyl c (9)..(9)
  LNA nucleosides (11)..(12)
tgataaaacgcc

SEQ ID NO: 384 - DNA, 13 bp, Artificial Sequence
  LNA antisense gapmer oligonucleotide
  phosphorothiate Internucleoside linkages (1)..(13)
  LNA nucleosides (1)..(3)
  5-methyl c (10)..(10)
  LNA nucleosides (12)..(13)
atgataaaacgcc

SEQ ID NO: 385 - DNA, 12 bp, Artificial Sequence
  LNA antisense gapmer oligonucleotide
  phosphorothiate Internucleoside linkages (1)..(12)
  LNA nucleosides (1)..(2)
  5-methyl c (10)..(10)
  LNA nucleosides (11)..(12)
atgataaaacgc

SEQ ID NO: 386 - DNA, 13 bp, Artificial Sequence
  LNA antisense gapmer oligonucleotide
  phosphorothiate Internucleoside linkages (1)..(13)
  LNA nucleosides (1)..(3)
  LNA nucleosides (12)..(13)
tagcagcaggatg

SEQ ID NO: 387 - DNA, 14 bp, Artificial Sequence
  LNA antisense gapmer oligonucleotide
  phosphorothiate Internucleoside linkages (1)..(14)
  LNA nucleosides (1)..(3)
  LNA nucleosides (12)..(14)
atagcagcaggatg

SEQ ID NO: 388 - DNA, 15 bp, Artificial Sequence
  LNA antisense gapmer oligonucleotide
  phosphorothiate Internucleoside linkages (1)..(15)
  LNA nucleosides (1)..(3)
  LNA nucleosides (13)..(15)
catagcagcaggatg

SEQ ID NO: 389 - DNA, 16 bp, Artificial Sequence
  LNA antisense gapmer oligonucleotide
  phosphorothiate Internucleoside linkages (1)..(16)
  LNA nucleosides (1)..(3)
  LNA nucleosides (14)..(16)
gcatagcagcaggatg

SEQ ID NO: 390 - DNA, 15 bp, Artificial Sequence
  LNA antisense gapmer oligonucleotide
  phosphorothiate Internucleoside linkages (1)..(15)
  LNA nucleosides (1)..(3)
  LNA nucleosides (13)..(15)
gcatagcagcaggat

SEQ ID NO: 391 - DNA, 16 bp, Artificial Sequence
  LNA antisense gapmer oligonucleotide
  phosphorothiate Internucleoside linkages (1)..(16)
  LNA nucleosides (1)..(3)
  LNA nucleosides (14)..(16)
ggcatagcagcaggat

SEQ ID NO: 392 - DNA, 16 bp, Artificial Sequence
  LNA antisense gapmer oligonucleotide
  phosphorothiate Internucleoside linkages (1)..(16)
  LNA nucleosides (1)..(3)
  LNA nucleosides (14)..(16)
gaggcatagcagcagg

SEQ ID NO: 393 - DNA, 16 bp, Artificial Sequence
  LNA antisense gapmer oligonucleotide
  phosphorothiate Internucleoside linkages (1)..(16)
  LNA nucleosides (1)..(3)
  LNA nucleosides (14)..(16)
tgaggcatagcagcag

SEQ ID NO: 394 - DNA, 15 bp, Artificial Sequence
  LNA antisense gapmer oligonucleotide
  phosphorothiate Internucleoside linkages (1)..(15)
  LNA nucleosides (1)..(3)
  LNA nucleosides (13)..(15)
tgaggcatagcagca

SEQ ID NO: 395 - DNA, 16 bp, Artificial Sequence
  LNA antisense gapmer oligonucleotide
  phosphorothiate Internucleoside linkages (1)..(16)
  LNA nucleosides (1)..(3)
  LNA nucleosides (14)..(16)
atgaggcatagcagca

SEQ ID NO: 396 - DNA, 14 bp, Artificial Sequence
  LNA antisense gapmer oligonucleotide
  phosphorothiate Internucleoside linkages (1)..(14)
  LNA nucleosides (1)..(3)
  LNA nucleosides (12)..(14)
tgaggcatagcagc

SEQ ID NO: 397 - DNA, 15 bp, Artificial Sequence
  LNA antisense gapmer oligonucleotide
  phosphorothiate Internucleoside linkages (1)..(15)
  LNA nucleosides (1)..(3)
  LNA nucleosides (13)..(15)
atgaggcatagcagc

SEQ ID NO: 398 - DNA, 16 bp, Artificial Sequence
  LNA antisense gapmer oligonucleotide
  phosphorothiate Internucleoside linkages (1)..(16)
  LNA nucleosides (1)..(3)
  LNA nucleosides (14)..(16)
gatgaggcatagcagc

SEQ ID NO: 399 - DNA, 15 bp, Artificial Sequence
  LNA antisense gapmer oligonucleotide
  phosphorothiate Internucleoside linkages (1)..(15)
  LNA nucleosides (1)..(3)
  LNA nucleosides (13)..(15)
gatgaggcatagcag

SEQ ID NO: 400 - DNA, 16 bp, Artificial Sequence
  LNA antisense gapmer oligonucleotide
  phosphorothiate Internucleoside linkages (1)..(16)
  LNA nucleosides (1)..(3)
  LNA nucleosides (14)..(16)
agatgaggcatagcag

SEQ ID NO: 401 - DNA, 14 bp, Artificial Sequence
  LNA antisense gapmer oligonucleotide
  phosphorothiate Internucleoside linkages (1)..(14)
  LNA nucleosides (1)..(3)
  LNA nucleosides (12)..(14)
gatgaggcatagca

SEQ ID NO: 402 - DNA, 15 bp, Artificial Sequence
  LNA antisense gapmer oligonucleotide
  phosphorothiate Internucleoside linkages (1)..(15)
  LNA nucleosides (1)..(3)
  LNA nucleosides (13)..(15)
agatgaggcatagca

SEQ ID NO: 403 - DNA, 16 bp, Artificial Sequence
  LNA antisense gapmer oligonucleotide
  phosphorothiate Internucleoside linkages (1)..(16)
  LNA nucleosides (1)..(3)
  LNA nucleosides (14)..(16)
aagatgaggcatagca

SEQ ID NO: 404 - DNA, 16 bp, Artificial Sequence
  LNA antisense gapmer oligonucleotide
  phosphorothiate Internucleoside linkages (1)..(16)
  LNA nucleosides (1)..(3)
  LNA nucleosides (14)..(16)
aagaagatgaggcata

SEQ ID NO: 405 - DNA, 15 bp, Artificial Sequence
  LNA antisense gapmer oligonucleotide
  phosphorothiate Internucleoside linkages (1)..(15)
  LNA nucleosides (1)..(3)
  LNA nucleosides (13)..(15)
aagaagatgaggcat

SEQ ID NO: 406 - DNA, 15 bp, Artificial Sequence
  LNA antisense gapmer oligonucleotide
  phosphorothiate Internucleoside linkages (1)..(15)
  LNA nucleosides (1)..(3)
  LNA nucleosides (13)..(15)
tgggatgggaataca

SEQ ID NO: 407 - DNA, 16 bp, Artificial Sequence
  LNA antisense gapmer oligonucleotide
  phosphorothiate Internucleoside linkages (1)..(16)
  LNA nucleosides (1)..(3)
  LNA nucleosides (14)..(16)
atgggatgggaataca

SEQ ID NO: 408 - DNA, 14 bp, Artificial Sequence
  LNA antisense gapmer oligonucleotide
  phosphorothiate Internucleoside linkages (1)..(14)
  LNA nucleosides (1)..(3)
  LNA nucleosides (12)..(14)
tgggatgggaatac

SEQ ID NO: 409 - DNA, 15 bp, Artificial Sequence
  LNA antisense gapmer oligonucleotide
  phosphorothiate Internucleoside linkages (1)..(15)
  LNA nucleosides (1)..(3)
  LNA nucleosides (13)..(15)
atgggatgggaatac

SEQ ID NO: 410 - DNA, 16 bp, Artificial Sequence
  LNA antisense gapmer oligonucleotide
  phosphorothiate Internucleoside linkages (1)..(16)
  LNA nucleosides (1)..(3)
  LNA nucleosides (14)..(16)
gatgggatgggaatac

SEQ ID NO: 411 - DNA, 14 bp, Artificial Sequence
  LNA antisense gapmer oligonucleotide
  phosphorothiate Internucleoside linkages (1)..(14)
  LNA nucleosides (1)..(3)
  LNA nucleosides (12)..(14)
atgggatgggaata

SEQ ID NO: 412 - DNA, 15 bp, Artificial Sequence
  LNA antisense gapmer oligonucleotide
  phosphorothiate Internucleoside linkages (1)..(15)
  LNA nucleosides (1)..(3)
  LNA nucleosides (13)..(15)
gatgggatgggaata

SEQ ID NO: 413 - DNA, 14 bp, Artificial Sequence
  LNA antisense gapmer oligonucleotide
  phosphorothiate Internucleoside linkages (1)..(14)
  LNA nucleosides (1)..(3)
  LNA nucleosides (12)..(14)
gatgggatgggaat

SEQ ID NO: 414 - DNA, 14 bp, Artificial Sequence
  LNA antisense gapmer oligonucleotide
  phosphorothiate Internucleoside linkages (1)..(14)
  LNA nucleosides (1)..(3)
  LNA nucleosides (12)..(14)
aaccactgaacaaa

SEQ ID NO: 415 - DNA, 12 bp, Artificial Sequence
  LNA antisense gapmer oligonucleotide
  phosphorothiate Internucleoside linkages (1)..(12)
  LNA nucleosides (1)..(2)
  LNA nucleosides (11)..(12)
cgaaccactgaa

SEQ ID NO: 416 - DNA, 13 bp, Artificial Sequence
  LNA antisense gapmer oligonucleotide
  phosphorothiate Internucleoside linkages (1)..(13)
  LNA nucleosides (1)..(3)
  LNA nucleosides (12)..(13)
gggggaaagccct

SEQ ID NO: 417 - DNA, 14 bp, Artificial Sequence
  LNA antisense gapmer oligonucleotide
  phosphorothiate Internucleoside linkages (1)..(14)
  LNA nucleosides (1)..(3)
  LNA nucleosides (12)..(14)
tgggggaaagccct

SEQ ID NO: 418 - DNA, 15 bp, Artificial Sequence
  LNA antisense gapmer oligonucleotide
  phosphorothiate Internucleoside linkages (1)..(15)
  LNA nucleosides (1)..(3)
  5-methyl c (5)..(5)
  LNA nucleosides (13)..(15)
gcaacggggtaaagg

SEQ ID NO: 419 - DNA, 14 bp, Artificial Sequence
  LNA antisense gapmer oligonucleotide
  phosphorothiate Internucleoside linkages (1)..(14)
  LNA nucleosides (1)..(3)
  5-methyl c (5)..(5)
  LNA nucleosides (12)..(14)
gcaacggggtaaag

SEQ ID NO: 420 - DNA, 13 bp, Artificial Sequence
  LNA antisense gapmer oligonucleotide
  phosphorothiate Internucleoside linkages (1)..(13)
  LNA nucleosides (1)..(3)
  5-methyl c (5)..(5)
  LNA nucleosides (12)..(13)
gcaacggggtaaa

SEQ ID NO: 421 - DNA, 15 bp, Artificial Sequence
  LNA antisense gapmer oligonucleotide
  phosphorothiate Internucleoside linkages (1)..(15)
  LNA nucleosides (1)..(3)
  LNA nucleosides (13)..(15)
agcaaacacttggca

SEQ ID NO: 422 - DNA, 16 bp, Artificial Sequence
  LNA antisense gapmer oligonucleotide
  phosphorothiate Internucleoside linkages (1)..(16)
  LNA nucleosides (1)..(3)
  LNA nucleosides (14)..(16)
cagcaaacacttggca

SEQ ID NO: 423 - DNA, 15 bp, Artificial Sequence
  LNA antisense gapmer oligonucleotide
  phosphorothiate Internucleoside linkages (1)..(15)
  LNA nucleosides (1)..(3)
  LNA nucleosides (13)..(15)
cagcaaacacttggc

SEQ ID NO: 424 - DNA, 16 bp, Artificial Sequence
  LNA antisense gapmer oligonucleotide
  phosphorothiate Internucleoside linkages (1)..(16)
  LNA nucleosides (1)..(3)
  LNA nucleosides (14)..(16)
tcagcaaacacttggc

SEQ ID NO: 425 - DNA, 15 bp, Artificial Sequence
  LNA antisense gapmer oligonucleotide
  phosphorothiate Internucleoside linkages (1)..(15)
  LNA nucleosides (1)..(3)
  LNA nucleosides (13)..(15)
tcagcaaacacttgg

SEQ ID NO: 426 - DNA, 13 bp, Artificial Sequence
  LNA antisense gapmer oligonucleotide
  phosphorothiate Internucleoside linkages (1)..(13)
  LNA nucleosides (1)..(3)
  LNA nucleosides (12)..(13)
gcagtatggatcg

SEQ ID NO: 427 - DNA, 14 bp, Artificial Sequence
  LNA antisense gapmer oligonucleotide
  phosphorothiate Internucleoside linkages (1)..(14)
  LNA nucleosides (1)..(3)
  LNA nucleosides (12)..(14)
cgcagtatggatcg

SEQ ID NO: 428 - DNA, 16 bp, Artificial Sequence
  LNA antisense gapmer oligonucleotide
  phosphorothiate Internucleoside linkages (1)..(16)
  LNA nucleosides (1)..(3)
  LNA nucleosides (14)..(16)
tccgcagtatggatcg

SEQ ID NO: 429 - DNA, 14 bp, Artificial Sequence
  LNA antisense gapmer oligonucleotide
  phosphorothiate Internucleoside linkages (1)..(14)
  LNA nucleosides (1)..(3)
  LNA nucleosides (12)..(14)
ccgcagtatggatc

SEQ ID NO: 430 - DNA, 15 bp, Artificial Sequence
  LNA antisense gapmer oligonucleotide
  phosphorothiate Internucleoside linkages (1)..(15)
  LNA nucleosides (1)..(3)
  LNA nucleosides (13)..(15)
tccgcagtatggatc

SEQ ID NO: 431 - DNA, 12 bp, Artificial Sequence
  LNA antisense gapmer oligonucleotide
  phosphorothiate Internucleoside linkages (1)..(12)
  LNA nucleosides (1)..(2)
  LNA nucleosides (11)..(12)
cgcagtatggat

SEQ ID NO: 432 - DNA, 13 bp, Artificial Sequence
  LNA antisense gapmer oligonucleotide
  phosphorothiate Internucleoside linkages (1)..(13)
  LNA nucleosides (1)..(3)
  LNA nucleosides (12)..(13)
ccgcagtatggat

SEQ ID NO: 433 - DNA, 14 bp, Artificial Sequence
  LNA antisense gapmer oligonucleotide
  phosphorothiate Internucleoside linkages (1)..(14)
  LNA nucleosides (1)..(3)
  LNA nucleosides (12)..(14)
tccgcagtatggat

SEQ ID NO: 434 - DNA, 13 bp, Artificial Sequence
  LNA antisense gapmer oligonucleotide
  phosphorothiate Internucleoside linkages (1)..(13)
  LNA nucleosides (1)..(3)
  LNA nucleosides (12)..(13)
tccgcagtatgga

SEQ ID NO: 435 - DNA, 12 bp, Artificial Sequence
  LNA antisense gapmer oligonucleotide
  phosphorothiate Internucleoside linkages (1)..(12)
  LNA nucleosides (1)..(2)
  5-methyl c (4)..(4)
  LNA nucleosides (11)..(12)
ttccgcagtatg

SEQ ID NO: 436 - DNA, 13 bp, Artificial Sequence
  LNA antisense gapmer oligonucleotide
  phosphorothiate Internucleoside linkages (1)..(13)
  LNA nucleosides (1)..(3)
  LNA nucleosides (12)..(13)
cgtaaagagaggt

SEQ ID NO: 437 - DNA, 16 bp, Artificial Sequence
  LNA antisense gapmer oligonucleotide
  phosphorothiate Internucleoside linkages (1)..(16)
  LNA nucleosides (1)..(3)
  5-methyl c (4)..(4)
  LNA nucleosides (14)..(16)
ccgcgtaaagagaggt

SEQ ID NO: 438 - DNA, 12 bp, Artificial Sequence
  LNA antisense gapmer oligonucleotide
  phosphorothiate Internucleoside linkages (1)..(12)
  LNA nucleosides (1)..(2)
  LNA nucleosides (11)..(12)
cgtaaagagagg

SEQ ID NO: 439 - DNA, 14 bp, Artificial Sequence
  LNA antisense gapmer oligonucleotide
  phosphorothiate Internucleoside linkages (1)..(14)
  LNA nucleosides (1)..(3)
  LNA nucleosides (12)..(14)
cgcgtaaagagagg

SEQ ID NO: 440 - DNA, 15 bp, Artificial Sequence
  LNA antisense gapmer oligonucleotide
  phosphorothiate Internucleoside linkages (1)..(15)
  LNA nucleosides (1)..(3)
  5-methyl c (4)..(4)
  LNA nucleosides (13)..(15)
ccgcgtaaagagagg

SEQ ID NO: 441 - DNA, 13 bp, Artificial Sequence
  LNA antisense gapmer oligonucleotide
  phosphorothiate Internucleoside linkages (1)..(13)
  LNA nucleosides (1)..(3)
  LNA nucleosides (12)..(13)
cgcgtaaagagag

SEQ ID NO: 442 - DNA, 14 bp, Artificial Sequence
  LNA antisense gapmer oligonucleotide
  phosphorothiate Internucleoside linkages (1)..(14)
  LNA nucleosides (1)..(3)
  5-methyl c (4)..(4)
  LNA nucleosides (12)..(14)
ccgcgtaaagagag

SEQ ID NO: 443 - DNA, 12 bp, Artificial Sequence
  LNA antisense gapmer oligonucleotide
  phosphorothiate Internucleoside linkages (1)..(12)
  LNA nucleosides (1)..(2)
  5-methyl c (3)..(3)
  LNA nucleosides (11)..(12)
cgcgtaaagaga

SEQ ID NO: 444 - DNA, 13 bp, Artificial Sequence
  LNA antisense gapmer oligonucleotide
  phosphorothiate Internucleoside linkages (1)..(13)
  LNA nucleosides (1)..(3)
  5-methyl c (4)..(4)
  LNA nucleosides (12)..(13)
ccgcgtaaagaga

SEQ ID NO: 445 - DNA, 12 bp, Artificial Sequence
  LNA antisense gapmer oligonucleotide
  phosphorothiate Internucleoside linkages (1)..(12)
  LNA nucleosides (1)..(2)
  5-methyl c (4)..(4)
  LNA nucleosides (11)..(12)
ccgcgtaaagag

SEQ ID NO: 446 - DNA, 15 bp, Artificial Sequence
  LNA antisense gapmer oligonucleotide
  phosphorothiate Internucleoside linkages (1)..(15)
  LNA nucleosides (1)..(3)
  5-methyl c (9)..(9)
  LNA nucleosides (13)..(15)
ggcacagacggggag

SEQ ID NO: 447 - DNA, 16 bp, Artificial Sequence
  LNA antisense gapmer oligonucleotide
  phosphorothiate Internucleoside linkages (1)..(16)
  LNA nucleosides (1)..(3)
  5-methyl c (10)..(10)
  LNA nucleosides (14)..(16)
aggcacagacggggag

SEQ ID NO: 448 - DNA, 14 bp, Artificial Sequence
  LNA antisense gapmer oligonucleotide
  phosphorothiate Internucleoside linkages (1)..(14)
  LNA nucleosides (1)..(3)
  5-methyl c (9)..(9)
  LNA nucleosides (12)..(14)
ggcacagacgggga

SEQ ID NO: 449 - DNA, 15 bp, Artificial Sequence
  LNA antisense gapmer oligonucleotide
  phosphorothiate Internucleoside linkages (1)..(15)
  LNA nucleosides (1)..(3)
  5-methyl c (10)..(10)
  LNA nucleosides (13)..(15)
aggcacagacgggga

SEQ ID NO: 450 - DNA, 16 bp, Artificial Sequence
  LNA antisense gapmer oligonucleotide
  phosphorothiate Internucleoside linkages (1)..(16)
  LNA nucleosides (1)..(3)
  5-methyl c (11)..(11)
  LNA nucleosides (14)..(16)
aaggcacagacgggga

SEQ ID NO: 451 - DNA, 14 bp, Artificial Sequence
  LNA antisense gapmer oligonucleotide
  phosphorothiate Internucleoside linkages (1)..(14)
  LNA nucleosides (1)..(3)
  5-methyl c (10)..(10)
  LNA nucleosides (12)..(14)
aggcacagacgggg

SEQ ID NO: 452 - DNA, 15 bp, Artificial Sequence
  LNA antisense gapmer oligonucleotide
  phosphorothiate Internucleoside linkages (1)..(15)
  LNA nucleosides (1)..(3)
  5-methyl c (11)..(11)
  LNA nucleosides (13)..(15)
aaggcacagacgggg

SEQ ID NO: 453 - DNA, 16 bp, Artificial Sequence
  LNA antisense gapmer oligonucleotide
  phosphorothiate Internucleoside linkages (1)..(16)
  LNA nucleosides (1)..(3)
  5-methyl c (12)..(12)
  LNA nucleosides (14)..(16)
gaaggcacagacgggg

SEQ ID NO: 454 - DNA, 16 bp, Artificial Sequence
  LNA antisense gapmer oligonucleotide
  phosphorothiate Internucleoside linkages (1)..(16)
  LNA nucleosides (1)..(3)
  5-methyl c (13)..(13)
  LNA nucleosides (14)..(16)
agaaggcacagacggg

SEQ ID NO: 455 - DNA, 15 bp, Artificial Sequence
  LNA antisense gapmer oligonucleotide
  phosphorothiate Internucleoside linkages (1)..(15)
  LNA nucleosides (1)..(3)
  LNA nucleosides (13)..(15)
gagaaggcacagacg

SEQ ID NO: 456 - DNA, 14 bp, Artificial Sequence
  LNA antisense gapmer oligonucleotide
  phosphorothiate Internucleoside linkages (1)..(14)
  LNA nucleosides (1)..(3)
  LNA nucleosides (12)..(14)
cgaagtgcacacgg

SEQ ID NO: 457 - DNA, 14 bp, Artificial Sequence
  LNA antisense gapmer oligonucleotide
  phosphorothiate Internucleoside linkages (1)..(14)
  LNA nucleosides (1)..(3)
  LNA nucleosides (12)..(14)
gcgaagtgcacacg

SEQ ID NO: 458 - DNA, 13 bp, Artificial Sequence
  LNA antisense gapmer oligonucleotide
  phosphorothiate Internucleoside linkages (1)..(13)
  LNA nucleosides (1)..(3)
  LNA nucleosides (12)..(13)
gcgaagtgcacac

SEQ ID NO: 459 - DNA, 14 bp, Artificial Sequence
  LNA antisense gapmer oligonucleotide
  phosphorothiate Internucleoside linkages (1)..(14)
  LNA nucleosides (1)..(3)
  LNA nucleosides (12)..(14)
agcgaagtgcacac

SEQ ID NO: 460 - DNA, 15 bp, Artificial Sequence
  LNA antisense gapmer oligonucleotide
  phosphorothiate Internucleoside linkages (1)..(15)
  LNA nucleosides (1)..(3)
  5-methyl c (4)..(4)
  LNA nucleosides (13)..(15)
aagcgaagtgcacac

SEQ ID NO: 461 - DNA, 16 bp, Artificial Sequence
  LNA antisense gapmer oligonucleotide
  phosphorothiate Internucleoside linkages (1)..(16)
  LNA nucleosides (1)..(3)
  5-methyl c (5)..(5)
  LNA nucleosides (14)..(16)
gaagcgaagtgcacac

SEQ ID NO: 462 - DNA, 13 bp, Artificial Sequence
  LNA antisense gapmer oligonucleotide
  phosphorothiate Internucleoside linkages (1)..(13)
  LNA nucleosides (1)..(3)
  LNA nucleosides (12)..(13)
agcgaagtgcaca

SEQ ID NO: 463 - DNA, 14 bp, Artificial Sequence
  LNA antisense gapmer oligonucleotide
  phosphorothiate Internucleoside linkages (1)..(14)
  LNA nucleosides (1)..(3)
  5-methyl c (4)..(4)
  LNA nucleosides (12)..(14)
aagcgaagtgcaca

SEQ ID NO: 464 - DNA, 16 bp, Artificial Sequence
  LNA antisense gapmer oligonucleotide
  phosphorothiate Internucleoside linkages (1)..(16)
  LNA nucleosides (1)..(3)
  5-methyl c (6)..(6)
  LNA nucleosides (14)..(16)
tgaagcgaagtgcaca

SEQ ID NO: 465 - DNA, 13 bp, Artificial Sequence
  LNA antisense gapmer oligonucleotide
  phosphorothiate Internucleoside linkages (1)..(13)
  LNA nucleosides (1)..(3)
  5-methyl c (4)..(4)
  LNA nucleosides (12)..(13)
aagcgaagtgcac

SEQ ID NO: 466 - DNA, 14 bp, Artificial Sequence
  LNA antisense gapmer oligonucleotide
  phosphorothiate Internucleoside linkages (1)..(14)
  LNA nucleosides (1)..(3)
  5-methyl c (5)..(5)
  LNA nucleosides (12)..(14)
gaagcgaagtgcac

SEQ ID NO: 467 - DNA, 15 bp, Artificial Sequence
  LNA antisense gapmer oligonucleotide
  phosphorothiate Internucleoside linkages (1)..(15)
  LNA nucleosides (1)..(3)
  5-methyl c (6)..(6)
  LNA nucleosides (13)..(15)
tgaagcgaagtgcac

SEQ ID NO: 468 - DNA, 16 bp, Artificial Sequence
  LNA antisense gapmer oligonucleotide
  phosphorothiate Internucleoside linkages (1)..(16)
  LNA nucleosides (1)..(3)
  5-methyl c (7)..(7)
  LNA nucleosides (14)..(16)
gtgaagcgaagtgcac

SEQ ID NO: 469 - DNA, 12 bp, Artificial Sequence
  LNA antisense gapmer oligonucleotide
  phosphorothiate Internucleoside linkages (1)..(12)
  LNA nucleosides (1)..(2)
  5-methyl c (4)..(4)
  LNA nucleosides (11)..(12)
aagcgaagtgca

SEQ ID NO: 470 - DNA, 13 bp, Artificial Sequence
  LNA antisense gapmer oligonucleotide
  phosphorothiate Internucleoside linkages (1)..(13)
  LNA nucleosides (1)..(3)
  5-methyl c (5)..(5)
  LNA nucleosides (12)..(13)
gaagcgaagtgca

SEQ ID NO: 471 - DNA, 14 bp, Artificial Sequence
  LNA antisense gapmer oligonucleotide
  phosphorothiate Internucleoside linkages (1)..(14)
  LNA nucleosides (1)..(3)
  5-methyl c (6)..(6)
  LNA nucleosides (12)..(14)
tgaagcgaagtgca

SEQ ID NO: 472 - DNA, 15 bp, Artificial Sequence
  LNA antisense gapmer oligonucleotide
  phosphorothiate Internucleoside linkages (1)..(15)
  LNA nucleosides (1)..(3)
  5-methyl c (7)..(7)
  LNA nucleosides (13)..(15)
gtgaagcgaagtgca

SEQ ID NO: 473 - DNA, 13 bp, Artificial Sequence
  LNA antisense gapmer oligonucleotide
  phosphorothiate Internucleoside linkages (1)..(13)
  LNA nucleosides (1)..(3)
  5-methyl c (6)..(6)
  LNA nucleosides (12)..(13)
tgaagcgaagtgc

SEQ ID NO: 474 - DNA, 14 bp, Artificial Sequence
  LNA antisense gapmer oligonucleotide
  phosphorothiate Internucleoside linkages (1)..(14)
  LNA nucleosides (1)..(3)
  5-methyl c (7)..(7)
  LNA nucleosides (12)..(14)
gtgaagcgaagtgc

SEQ ID NO: 475 - DNA, 13 bp, Artificial Sequence
  LNA antisense gapmer oligonucleotide
  phosphorothiate Internucleoside linkages (1)..(13)
  LNA nucleosides (1)..(3)
  5-methyl c (7)..(7)
  LNA nucleosides (12)..(13)
gtgaagcgaagtg

SEQ ID NO: 476 - DNA, 14 bp, Artificial Sequence
  LNA antisense gapmer oligonucleotide
  phosphorothiate Internucleoside linkages (1)..(14)
  LNA nucleosides (1)..(3)
  5-methyl c (8)..(8)
  LNA nucleosides (12)..(14)
ggtgaagcgaagtg

SEQ ID NO: 477 - DNA, 16 bp, Artificial Sequence
  LNA antisense gapmer oligonucleotide
  phosphorothiate Internucleoside linkages (1)..(16)
  LNA nucleosides (1)..(3)
  5-methyl c (10)..(10)
  LNA nucleosides (14)..(16)
gaggtgaagcgaagtg

SEQ ID NO: 478 - DNA, 12 bp, Artificial Sequence
  LNA antisense gapmer oligonucleotide
  phosphorothiate Internucleoside linkages (1)..(12)
  LNA nucleosides (1)..(2)
  5-methyl c (7)..(7)
  LNA nucleosides (11)..(12)
gtgaagcgaagt

SEQ ID NO: 479 - DNA, 13 bp, Artificial Sequence
  LNA antisense gapmer oligonucleotide
  phosphorothiate Internucleoside linkages (1)..(13)
  LNA nucleosides (1)..(3)
  5-methyl c (8)..(8)
  LNA nucleosides (12)..(13)
ggtgaagcgaagt

SEQ ID NO: 480 - DNA, 15 bp, Artificial Sequence
  LNA antisense gapmer oligonucleotide
  phosphorothiate Internucleoside linkages (1)..(15)
  LNA nucleosides (1)..(3)
  5-methyl c (10)..(10)
  LNA nucleosides (13)..(15)
gaggtgaagcgaagt

SEQ ID NO: 481 - DNA, 16 bp, Artificial Sequence
  LNA antisense gapmer oligonucleotide
  phosphorothiate Internucleoside linkages (1)..(16)
  LNA nucleosides (1)..(3)
  5-methyl c (11)..(11)
  LNA nucleosides (14)..(16)
agaggtgaagcgaagt

SEQ ID NO: 482 - DNA, 15 bp, Artificial Sequence
  LNA antisense gapmer oligonucleotide
  phosphorothiate Internucleoside linkages (1)..(15)
  LNA nucleosides (1)..(3)
  5-methyl c (11)..(11)
  LNA nucleosides (13)..(15)
agaggtgaagcgaag

SEQ ID NO: 483 - DNA, 16 bp, Artificial Sequence
  LNA antisense gapmer oligonucleotide
  phosphorothiate Internucleoside linkages (1)..(16)
  LNA nucleosides (1)..(3)
  5-methyl c (12)..(12)
  LNA nucleosides (14)..(16)
cagaggtgaagcgaag

SEQ ID NO: 484 - DNA, 14 bp, Artificial Sequence
  LNA antisense gapmer oligonucleotide
  phosphorothiate Internucleoside linkages (1)..(14)
  LNA nucleosides (1)..(3)
  5-methyl c (11)..(11)
  LNA nucleosides (12)..(14)
agaggtgaagcgaa

SEQ ID NO: 485 - DNA, 15 bp, Artificial Sequence
  LNA antisense gapmer oligonucleotide
  phosphorothiate Internucleoside linkages (1)..(15)
  LNA nucleosides (1)..(3)
  5-methyl c (12)..(12)
  LNA nucleosides (13)..(15)
cagaggtgaagcgaa

SEQ ID NO: 486 - DNA, 16 bp, Artificial Sequence
  LNA antisense gapmer oligonucleotide
  phosphorothiate Internucleoside linkages (1)..(16)
  LNA nucleosides (1)..(3)
  5-methyl c (13)..(13)
  LNA nucleosides (14)..(16)
gcagaggtgaagcgaa

SEQ ID NO: 487 - DNA, 15 bp, Artificial Sequence
  LNA antisense gapmer oligonucleotide
  phosphorothiate Internucleoside linkages (1)..(15)
  LNA nucleosides (1)..(3)
  LNA nucleosides (13)..(15)
gcagaggtgaagcga

SEQ ID NO: 488 - DNA, 16 bp, Artificial Sequence
  LNA antisense gapmer oligonucleotide
  phosphorothiate Internucleoside linkages (1)..(16)
  LNA nucleosides (1)..(3)
  LNA nucleosides (14)..(16)
tgcagaggtgaagcga

SEQ ID NO: 489 - DNA, 15 bp, Artificial Sequence
  LNA antisense gapmer oligonucleotide
  phosphorothiate Internucleoside linkages (1)..(15)
  LNA nucleosides (1)..(3)
  LNA nucleosides (13)..(15)
tgcagaggtgaagcg

SEQ ID NO: 490 - DNA, 16 bp, Artificial Sequence
  LNA antisense gapmer oligonucleotide
  phosphorothiate Internucleoside linkages (1)..(16)
  LNA nucleosides (1)..(3)
  LNA nucleosides (14)..(16)
gtgcagaggtgaagcg

SEQ ID NO: 491 - DNA, 16 bp, Artificial Sequence
  LNA antisense gapmer oligonucleotide
  phosphorothiate Internucleoside linkages (1)..(16)
  LNA nucleosides (1)..(3)
  LNA nucleosides (14)..(16)
cgtgcagaggtgaagc

SEQ ID NO: 492 - DNA, 15 bp, Artificial Sequence
  LNA antisense gapmer oligonucleotide
  phosphorothiate Internucleoside linkages (1)..(15)
  LNA nucleosides (1)..(3)
  LNA nucleosides (13)..(15)
cgtgcagaggtgaag

SEQ ID NO: 493 - DNA, 16 bp, Artificial Sequence
  LNA antisense gapmer oligonucleotide
  phosphorothiate Internucleoside linkages (1)..(16)
  LNA nucleosides (1)..(3)
  LNA nucleosides (14)..(16)
acgtgcagaggtgaag

SEQ ID NO: 494 - DNA, 14 bp, Artificial Sequence
  LNA antisense gapmer oligonucleotide
  phosphorothiate Internucleoside linkages (1)..(14)
  LNA nucleosides (1)..(3)
  LNA nucleosides (12)..(14)
cgtgcagaggtgaa

SEQ ID NO: 495 - DNA, 15 bp, Artificial Sequence
  LNA antisense gapmer oligonucleotide
  phosphorothiate Internucleoside linkages (1)..(15)
  LNA nucleosides (1)..(3)
  LNA nucleosides (13)..(15)
acgtgcagaggtgaa

SEQ ID NO: 496 - DNA, 13 bp, Artificial Sequence
  LNA antisense gapmer oligonucleotide
  phosphorothiate Internucleoside linkages (1)..(13)
  LNA nucleosides (1)..(3)
  LNA nucleosides (12)..(13)
cgtgcagaggtga

SEQ ID NO: 497 - DNA, 14 bp, Artificial Sequence
  LNA antisense gapmer oligonucleotide
  phosphorothiate Internucleoside linkages (1)..(14)
  LNA nucleosides (1)..(3)
  LNA nucleosides (12)..(14)
acgtgcagaggtga

SEQ ID NO: 498 - DNA, 13 bp, Artificial Sequence
  LNA antisense gapmer oligonucleotide
  phosphorothiate Internucleoside linkages (1)..(13)
  LNA nucleosides (1)..(3)
  5-methyl c (7)..(7)
  LNA nucleosides (12)..(13)
cgttcacggtggt

SEQ ID NO: 499 - DNA, 13 bp, Artificial Sequence
  LNA antisense gapmer oligonucleotide
  phosphorothiate Internucleoside linkages (1)..(13)
  LNA nucleosides (1)..(3)
  5-methyl c (9)..(9)
  LNA nucleosides (12)..(13)
ctcaaggtcggtc

SEQ ID NO: 500 - DNA, 13 bp, Artificial Sequence
  LNA antisense gapmer oligonucleotide
  phosphorothiate Internucleoside linkages (1)..(13)
  LNA nucleosides (1)..(3)
  5-methyl c (10)..(10)
  LNA nucleosides (12)..(13)
cctcaaggtcggt

SEQ ID NO: 501 - DNA, 14 bp, Artificial Sequence
  LNA antisense gapmer oligonucleotide
  phosphorothiate Internucleoside linkages (1)..(14)
  LNA nucleosides (1)..(3)
  5-methyl c (11)..(11)
  LNA nucleosides (12)..(14)
gcctcaaggtcggt

SEQ ID NO: 502 - DNA, 15 bp, Artificial Sequence
  LNA antisense gapmer oligonucleotide
  phosphorothiate Internucleoside linkages (1)..(15)
  LNA nucleosides (1)..(3)
  LNA nucleosides (13)..(15)
acagtctttgaagta

SEQ ID NO: 503 - DNA, 13 bp, Artificial Sequence
  LNA antisense gapmer oligonucleotide
  phosphorothiate Internucleoside linkages (1)..(13)
  LNA nucleosides (1)..(3)
  LNA nucleosides (12)..(13)
tttatgcctacag

SEQ ID NO: 504 - DNA, 14 bp, Artificial Sequence
  LNA antisense gapmer oligonucleotide
  phosphorothiate Internucleoside linkages (1)..(14)
  LNA nucleosides (1)..(3)
  LNA nucleosides (12)..(14)
aatttatgcctaca

SEQ ID NO: 505 - DNA, 13 bp, Artificial Sequence
  LNA antisense gapmer oligonucleotide
  phosphorothiate Internucleoside linkages (1)..(13)
  LNA nucleosides (1)..(3)
  LNA nucleosides (12)..(13)
aatttatgcctac

SEQ ID NO: 506 - DNA, 13 bp, Artificial Sequence
  LNA antisense gapmer oligonucleotide
  phosphorothiate Internucleoside linkages (1)..(13)
  LNA nucleosides (1)..(3)
  LNA nucleosides (12)..(13)
ccaatttatgcct

SEQ ID NO: 507 - DNA, 15 bp, Artificial Sequence
  LNA antisense gapmer oligonucleotide
  phosphorothiate Internucleoside linkages (1)..(15)
  LNA nucleosides (1)..(3)
  LNA nucleosides (13)..(15)
gcttggaggcttgaa

SEQ ID NO: 508 - DNA, 16 bp, Artificial Sequence
  LNA antisense gapmer oligonucleotide
  phosphorothiate Internucleoside linkages (1)..(16)
  LNA nucleosides (1)..(3)
  LNA nucleosides (14)..(16)
agcttggaggcttgaa

SEQ ID NO: 509 - DNA, 14 bp, Artificial Sequence
  LNA antisense gapmer oligonucleotide
  phosphorothiate Internucleoside linkages (1)..(14)
  LNA nucleosides (1)..(3)
  LNA nucleosides (12)..(14)
gcttggaggcttga

SEQ ID NO: 510 - DNA, 15 bp, Artificial Sequence
  LNA antisense gapmer oligonucleotide
  phosphorothiate Internucleoside linkages (1)..(15)
  LNA nucleosides (1)..(3)
  LNA nucleosides (13)..(15)
agcttggaggcttga

SEQ ID NO: 511 - DNA, 16 bp, Artificial Sequence
  LNA antisense gapmer oligonucleotide
  phosphorothiate Internucleoside linkages (1)..(16)
  LNA nucleosides (1)..(3)
  LNA nucleosides (14)..(16)
cagcttggaggcttga

SEQ ID NO: 512 - DNA, 13 bp, Artificial Sequence
  LNA antisense gapmer oligonucleotide
  phosphorothiate Internucleoside linkages (1)..(13)
  LNA nucleosides (1)..(3)
  LNA nucleosides (12)..(13)
gcttggaggcttg

SEQ ID NO: 513 - DNA, 14 bp, Artificial Sequence
  LNA antisense gapmer oligonucleotide
  phosphorothiate Internucleoside linkages (1)..(14)
  LNA nucleosides (1)..(3)
  LNA nucleosides (12)..(14)
agcttggaggcttg

SEQ ID NO: 514 - DNA, 15 bp, Artificial Sequence
  LNA antisense gapmer oligonucleotide
  phosphorothiate Internucleoside linkages (1)..(15)
  LNA nucleosides (1)..(3)
  LNA nucleosides (13)..(15)
cagcttggaggcttg

SEQ ID NO: 515 - DNA, 16 bp, Artificial Sequence
  LNA antisense gapmer oligonucleotide
  phosphorothiate Internucleoside linkages (1)..(16)
  LNA nucleosides (1)..(3)
  LNA nucleosides (14)..(16)
acagcttggaggcttg

SEQ ID NO: 516 - DNA, 16 bp, Artificial Sequence
  LNA antisense gapmer oligonucleotide
  phosphorothiate Internucleoside linkages (1)..(16)
  LNA nucleosides (1)..(3)
  LNA nucleosides (14)..(16)
cacagcttggaggctt

SEQ ID NO: 517 - DNA, 15 bp, Artificial Sequence
  LNA antisense gapmer oligonucleotide
  phosphorothiate Internucleoside linkages (1)..(15)
  LNA nucleosides (1)..(3)
  LNA nucleosides (13)..(15)
cacagcttggaggct

SEQ ID NO: 518 - DNA, 16 bp, Artificial Sequence
  LNA antisense gapmer oligonucleotide
  phosphorothiate Internucleoside linkages (1)..(16)
  LNA nucleosides (1)..(3)
  LNA nucleosides (14)..(16)
gcacagcttggaggct

SEQ ID NO: 519 - DNA, 15 bp, Artificial Sequence
  LNA antisense gapmer oligonucleotide
  phosphorothiate Internucleoside linkages (1)..(15)
  LNA nucleosides (1)..(3)
  LNA nucleosides (13)..(15)
gcacagcttggaggc

SEQ ID NO: 520 - DNA, 16 bp, Artificial Sequence
  LNA antisense gapmer oligonucleotide
  phosphorothiate Internucleoside linkages (1)..(16)
  LNA nucleosides (1)..(3)
  LNA nucleosides (14)..(16)
ggcacagcttggaggc

SEQ ID NO: 521 - DNA, 16 bp, Artificial Sequence
  LNA antisense gapmer oligonucleotide
  phosphorothiate Internucleoside linkages (1)..(16)
  LNA nucleosides (1)..(3)
  LNA nucleosides (14)..(16)
aggcacagcttggagg

SEQ ID NO: 522 - DNA, 15 bp, Artificial Sequence
  LNA antisense gapmer oligonucleotide
  phosphorothiate Internucleoside linkages (1)..(15)
  LNA nucleosides (1)..(3)
  LNA nucleosides (13)..(15)
aggcacagcttggag

SEQ ID NO: 523 - DNA, 16 bp, Artificial Sequence
  LNA antisense gapmer oligonucleotide
  phosphorothiate Internucleoside linkages (1)..(16)
  LNA nucleosides (1)..(3)
  LNA nucleosides (14)..(16)
aaggcacagcttggag

SEQ ID NO: 524 - DNA, 15 bp, Artificial Sequence
  LNA antisense gapmer oligonucleotide
  phosphorothiate Internucleoside linkages (1)..(15)
  LNA nucleosides (1)..(3)
  LNA nucleosides (13)..(15)
aaggcacagcttgga

SEQ ID NO: 525 - DNA, 16 bp, Artificial Sequence
  LNA antisense gapmer oligonucleotide
  phosphorothiate Internucleoside linkages (1)..(16)
  LNA nucleosides (1)..(3)
  LNA nucleosides (14)..(16)
caaggcacagcttgga

SEQ ID NO: 526 - DNA, 14 bp, Artificial Sequence
  LNA antisense gapmer oligonucleotide
  phosphorothiate Internucleoside linkages (1)..(14)
  LNA nucleosides (1)..(3)
  LNA nucleosides (12)..(14)
aaggcacagcttgg

SEQ ID NO: 527 - DNA, 15 bp, Artificial Sequence
  LNA antisense gapmer oligonucleotide
  phosphorothiate Internucleoside linkages (1)..(15)
  LNA nucleosides (1)..(3)
  LNA nucleosides (13)..(15)
caaggcacagcttgg

SEQ ID NO: 528 - DNA, 16 bp, Artificial Sequence
  LNA antisense gapmer oligonucleotide
  phosphorothiate Internucleoside linkages (1)..(16)
  LNA nucleosides (1)..(3)
  LNA nucleosides (14)..(16)
ccaaggcacagcttgg

SEQ ID NO: 529 - DNA, 14 bp, Artificial Sequence
  LNA antisense gapmer oligonucleotide
  phosphorothiate Internucleoside linkages (1)..(14)
  LNA nucleosides (1)..(3)
  LNA nucleosides (12)..(14)
caaggcacagcttg

SEQ ID NO: 530 - DNA, 15 bp, Artificial Sequence
  LNA antisense gapmer oligonucleotide
  phosphorothiate Internucleoside linkages (1)..(15)
  LNA nucleosides (1)..(3)
  LNA nucleosides (13)..(15)
ccaaggcacagcttg

SEQ ID NO: 531 - DNA, 14 bp, Artificial Sequence
  LNA antisense gapmer oligonucleotide
  phosphorothiate Internucleoside linkages (1)..(14)
  LNA nucleosides (1)..(3)
  LNA nucleosides (12)..(14)
ccaaggcacagctt

SEQ ID NO: 532 - DNA, 13 bp, Artificial Sequence
  LNA antisense gapmer oligonucleotide
  phosphorothiate Internucleoside linkages (1)..(13)
  LNA nucleosides (1)..(3)
  LNA nucleosides (12)..(13)
tgcgaatccacac

SEQ ID NO: 533 - DNA, 14 bp, Artificial Sequence
  LNA antisense gapmer oligonucleotide
  phosphorothiate Internucleoside linkages (1)..(14)
  LNA nucleosides (1)..(3)
  5-methyl c (4)..(4)
  LNA nucleosides (12)..(14)
gtgcgaatccacac

SEQ ID NO: 534 - DNA, 15 bp, Artificial Sequence
  LNA antisense gapmer oligonucleotide
  phosphorothiate Internucleoside linkages (1)..(15)
  LNA nucleosides (1)..(3)
  LNA nucleosides (13)..(15)
ggagttcttcttcta

SEQ ID NO: 535 - DNA, 16 bp, Artificial Sequence
  LNA antisense gapmer oligonucleotide
  phosphorothiate Internucleoside linkages (1)..(16)
  LNA nucleosides (1)..(3)
  LNA nucleosides (14)..(16)
gggagttcttcttcta

SEQ ID NO: 536 - DNA, 15 bp, Artificial Sequence
  LNA antisense gapmer oligonucleotide
  phosphorothiate Internucleoside linkages (1)..(15)
  LNA nucleosides (1)..(3)
  LNA nucleosides (13)..(15)
gggagttcttcttct

SEQ ID NO: 537 - DNA, 16 bp, Artificial Sequence
  LNA antisense gapmer oligonucleotide
  phosphorothiate Internucleoside linkages (1)..(16)
  LNA nucleosides (1)..(3)
  LNA nucleosides (14)..(16)
agggagttcttcttct

SEQ ID NO: 538 - DNA, 15 bp, Artificial Sequence
  LNA antisense gapmer oligonucleotide
  phosphorothiate Internucleoside linkages (1)..(15)
  LNA nucleosides (1)..(3)
  LNA nucleosides (13)..(15)
agggagttcttcttc

SEQ ID NO: 539 - DNA, 16 bp, Artificial Sequence
  LNA antisense gapmer oligonucleotide
  phosphorothiate Internucleoside linkages (1)..(16)
  LNA nucleosides (1)..(3)
  LNA nucleosides (14)..(16)
gagggagttcttcttc

SEQ ID NO: 540 - DNA, 14 bp, Artificial Sequence
  LNA antisense gapmer oligonucleotide
  phosphorothiate Internucleoside linkages (1)..(14)
  LNA nucleosides (1)..(3)
  LNA nucleosides (12)..(14)
agggagttcttctt

SEQ ID NO: 541 - DNA, 15 bp, Artificial Sequence
  LNA antisense gapmer oligonucleotide
  phosphorothiate Internucleoside linkages (1)..(15)
  LNA nucleosides (1)..(3)
  LNA nucleosides (13)..(15)
gagggagttcttctt

SEQ ID NO: 542 - DNA, 16 bp, Artificial Sequence
  LNA antisense gapmer oligonucleotide
  phosphorothiate Internucleoside linkages (1)..(16)
  LNA nucleosides (1)..(3)
  LNA nucleosides (14)..(16)
cgagggagttcttctt

SEQ ID NO: 543 - DNA, 15 bp, Artificial Sequence
  LNA antisense gapmer oligonucleotide
  phosphorothiate Internucleoside linkages (1)..(15)
  LNA nucleosides (1)..(3)
  LNA nucleosides (13)..(15)
cgagggagttcttct

SEQ ID NO: 544 - DNA, 16 bp, Artificial Sequence
  LNA antisense gapmer oligonucleotide
  phosphorothiate Internucleoside linkages (1)..(16)
  LNA nucleosides (1)..(3)
  LNA nucleosides (14)..(16)
gcgagggagttcttct

SEQ ID NO: 545 - DNA, 15 bp, Artificial Sequence
  LNA antisense gapmer oligonucleotide
  phosphorothiate Internucleoside linkages (1)..(15)
  LNA nucleosides (1)..(3)
  LNA nucleosides (13)..(15)
gcgagggagttcttc

SEQ ID NO: 546 - DNA, 16 bp, Artificial Sequence
  LNA antisense gapmer oligonucleotide
  phosphorothiate Internucleoside linkages (1)..(16)
  LNA nucleosides (1)..(3)
  LNA nucleosides (14)..(16)
ggcgagggagttcttc

SEQ ID NO: 547 - DNA, 14 bp, Artificial Sequence
  LNA antisense gapmer oligonucleotide
  phosphorothiate Internucleoside linkages (1)..(14)
  LNA nucleosides (1)..(3)
  LNA nucleosides (12)..(14)
gcgagggagttctt

SEQ ID NO: 548 - DNA, 15 bp, Artificial Sequence
  LNA antisense gapmer oligonucleotide
  phosphorothiate Internucleoside linkages (1)..(15)
  LNA nucleosides (1)..(3)
  LNA nucleosides (13)..(15)
ggcgagggagttctt

SEQ ID NO: 549 - DNA, 16 bp, Artificial Sequence
  LNA antisense gapmer oligonucleotide
  phosphorothiate Internucleoside linkages (1)..(16)
  LNA nucleosides (1)..(3)
  5-methyl c (4)..(4)
  LNA nucleosides (14)..(16)
aggcgagggagttctt

SEQ ID NO: 550 - DNA, 13 bp, Artificial Sequence
  LNA antisense gapmer oligonucleotide
  phosphorothiate Internucleoside linkages (1)..(13)
  LNA nucleosides (1)..(3)
  LNA nucleosides (12)..(13)
gcgagggagttct

SEQ ID NO: 551 - DNA, 14 bp, Artificial Sequence
  LNA antisense gapmer oligonucleotide
  phosphorothiate Internucleoside linkages (1)..(14)
  LNA nucleosides (1)..(3)
  LNA nucleosides (12)..(14)
ggcgagggagttct

SEQ ID NO: 552 - DNA, 15 bp, Artificial Sequence
  LNA antisense gapmer oligonucleotide
  phosphorothiate Internucleoside linkages (1)..(15)
  LNA nucleosides (1)..(3)
  5-methyl c (4)..(4)
  LNA nucleosides (13)..(15)
aggcgagggagttct

SEQ ID NO: 553 - DNA, 16 bp, Artificial Sequence
  LNA antisense gapmer oligonucleotide
  phosphorothiate Internucleoside linkages (1)..(16)
  LNA nucleosides (1)..(3)
  5-methyl c (5)..(5)
  LNA nucleosides (14)..(16)
gaggcgagggagttct

SEQ ID NO: 554 - DNA, 13 bp, Artificial Sequence
  LNA antisense gapmer oligonucleotide
  phosphorothiate Internucleoside linkages (1)..(13)
  LNA nucleosides (1)..(3)
  LNA nucleosides (12)..(13)
ggcgagggagttc

SEQ ID NO: 555 - DNA, 14 bp, Artificial Sequence
  LNA antisense gapmer oligonucleotide
  phosphorothiate Internucleoside linkages (1)..(14)
  LNA nucleosides (1)..(3)
  5-methyl c (4)..(4)
  LNA nucleosides (12)..(14)
aggcgagggagttc

SEQ ID NO: 556 - DNA, 15 bp, Artificial Sequence
  LNA antisense gapmer oligonucleotide
  phosphorothiate Internucleoside linkages (1)..(15)
  LNA nucleosides (1)..(3)
  5-methyl c (5)..(5)
  LNA nucleosides (13)..(15)
gaggcgagggagttc

SEQ ID NO: 557 - DNA, 16 bp, Artificial Sequence
  LNA antisense gapmer oligonucleotide
  phosphorothiate Internucleoside linkages (1)..(16)
  LNA nucleosides (1)..(3)
  5-methyl c (6)..(6)
  LNA nucleosides (14)..(16)
cgaggcgagggagttc

SEQ ID NO: 558 - DNA, 13 bp, Artificial Sequence
  LNA antisense gapmer oligonucleotide
  phosphorothiate Internucleoside linkages (1)..(13)
  LNA nucleosides (1)..(3)
  5-methyl c (4)..(4)
  LNA nucleosides (12)..(13)
aggcgagggagtt

SEQ ID NO: 559 - DNA, 14 bp, Artificial Sequence
  LNA antisense gapmer oligonucleotide
  phosphorothiate Internucleoside linkages (1)..(14)
  LNA nucleosides (1)..(3)
  5-methyl c (5)..(5)
  LNA nucleosides (12)..(14)
gaggcgagggagtt

SEQ ID NO: 560 - DNA, 15 bp, Artificial Sequence
  LNA antisense gapmer oligonucleotide
  phosphorothiate Internucleoside linkages (1)..(15)
  LNA nucleosides (1)..(3)
  5-methyl c (6)..(6)
  LNA nucleosides (13)..(15)
cgaggcgagggagtt

SEQ ID NO: 561 - DNA, 16 bp, Artificial Sequence
  LNA antisense gapmer oligonucleotide
  phosphorothiate Internucleoside linkages (1)..(16)
  LNA nucleosides (1)..(3)
  5-methyl c (7)..(7)
  LNA nucleosides (14)..(16)
gcgaggcgagggagtt

SEQ ID NO: 562 - DNA, 13 bp, Artificial Sequence
  LNA antisense gapmer oligonucleotide
  phosphorothiate Internucleoside linkages (1)..(13)
  LNA nucleosides (1)..(3)
  5-methyl c (5)..(5)
  LNA nucleosides (12)..(13)
gaggcgagggagt

SEQ ID NO: 563 - DNA, 14 bp, Artificial Sequence
  LNA antisense gapmer oligonucleotide
  phosphorothiate Internucleoside linkages (1)..(14)
  LNA nucleosides (1)..(3)
  5-methyl c (6)..(6)
  LNA nucleosides (12)..(14)
cgaggcgagggagt

SEQ ID NO: 564 - DNA, 15 bp, Artificial Sequence
  LNA antisense gapmer oligonucleotide
  phosphorothiate Internucleoside linkages (1)..(15)
  LNA nucleosides (1)..(3)
  5-methyl c (7)..(7)
  LNA nucleosides (13)..(15)
gcgaggcgagggagt

SEQ ID NO: 565 - DNA, 16 bp, Artificial Sequence
  LNA antisense gapmer oligonucleotide
  phosphorothiate Internucleoside linkages (1)..(16)
  LNA nucleosides (1)..(3)
  5-methyl c (8)..(8)
  LNA nucleosides (14)..(16)
tgcgaggcgagggagt

SEQ ID NO: 566 - DNA, 13 bp, Artificial Sequence
  LNA antisense gapmer oligonucleotide
  phosphorothiate Internucleoside linkages (1)..(13)
  LNA nucleosides (1)..(3)
  5-methyl c (6)..(6)
  LNA nucleosides (12)..(13)
cgaggcgagggag

SEQ ID NO: 567 - DNA, 14 bp, Artificial Sequence
  LNA antisense gapmer oligonucleotide
  phosphorothiate Internucleoside linkages (1)..(14)
  LNA nucleosides (1)..(3)
  5-methyl c (7)..(7)
  LNA nucleosides (12)..(14)
gcgaggcgagggag

SEQ ID NO: 568 - DNA, 15 bp, Artificial Sequence
  LNA antisense gapmer oligonucleotide
  phosphorothiate Internucleoside linkages (1)..(15)
  LNA nucleosides (1)..(3)
  5-methyl c (8)..(8)
  LNA nucleosides (13)..(15)
tgcgaggcgagggag

SEQ ID NO: 569 - DNA, 16 bp, Artificial Sequence
  LNA antisense gapmer oligonucleotide
  phosphorothiate Internucleoside linkages (1)..(16)
  LNA nucleosides (1)..(3)
  5-methyl c (4)..(4)
  5-methyl c (9)..(9)
  LNA nucleosides (14)..(16)
ctgcgaggcgagggag

SEQ ID NO: 570 - DNA, 12 bp, Artificial Sequence
  LNA antisense gapmer oligonucleotide
  phosphorothiate Internucleoside linkages (1)..(12)
  LNA nucleosides (1)..(2)
  5-methyl c (6)..(6)
  LNA nucleosides (11)..(12)
cgaggcgaggga

SEQ ID NO: 571 - DNA, 13 bp, Artificial Sequence
  LNA antisense gapmer oligonucleotide
  phosphorothiate Internucleoside linkages (1)..(13)
  LNA nucleosides (1)..(3)
  5-methyl c (7)..(7)
  LNA nucleosides (12)..(13)
gcgaggcgaggga

SEQ ID NO: 572 - DNA, 14 bp, Artificial Sequence
  LNA antisense gapmer oligonucleotide
  phosphorothiate Internucleoside linkages (1)..(14)
  LNA nucleosides (1)..(3)
  5-methyl c (8)..(8)
  LNA nucleosides (12)..(14)
tgcgaggcgaggga

SEQ ID NO: 573 - DNA, 15 bp, Artificial Sequence
  LNA antisense gapmer oligonucleotide
  phosphorothiate Internucleoside linkages (1)..(15)
  LNA nucleosides (1)..(3)
  5-methyl c (4)..(4)
  5-methyl c (9)..(9)
  LNA nucleosides (13)..(15)
ctgcgaggcgaggga

SEQ ID NO: 574 - DNA, 16 bp, Artificial Sequence
  LNA antisense gapmer oligonucleotide
  phosphorothiate Internucleoside linkages (1)..(16)
  LNA nucleosides (1)..(3)
  5-methyl c (5)..(5)
  5-methyl c (10)..(10)
  LNA nucleosides (14)..(16)
tctgcgaggcgaggga

SEQ ID NO: 575 - DNA, 15 bp, Artificial Sequence
  LNA antisense gapmer oligonucleotide
  phosphorothiate Internucleoside linkages (1)..(15)
  LNA nucleosides (1)..(3)
  5-methyl c (5)..(5)
  5-methyl c (10)..(10)
  LNA nucleosides (13)..(15)
tctgcgaggcgaggg

SEQ ID NO: 576 - DNA, 16 bp, Artificial Sequence
  LNA antisense gapmer oligonucleotide
  phosphorothiate Internucleoside linkages (1)..(16)
  LNA nucleosides (1)..(3)
  5-methyl c (6)..(6)
  5-methyl c (11)..(11)
  LNA nucleosides (14)..(16)
gtctgcgaggcgaggg

SEQ ID NO: 577 - DNA, 14 bp, Artificial Sequence
  LNA antisense gapmer oligonucleotide
  phosphorothiate Internucleoside linkages (1)..(14)
  LNA nucleosides (1)..(3)
  LNA nucleosides (12)..(14)
gttcccaagaatat

SEQ ID NO: 578 - DNA, 15 bp, Artificial Sequence
  LNA antisense gapmer oligonucleotide
  phosphorothiate Internucleoside linkages (1)..(15)
  LNA nucleosides (1)..(3)
  LNA nucleosides (13)..(15)
tgttcccaagaatat

SEQ ID NO: 579 - DNA, 13 bp, Artificial Sequence
  LNA antisense gapmer oligonucleotide
  phosphorothiate Internucleoside linkages (1)..(13)
  LNA nucleosides (1)..(3)
  LNA nucleosides (12)..(13)
gttcccaagaata

SEQ ID NO: 580 - DNA, 14 bp, Artificial Sequence
  LNA antisense gapmer oligonucleotide
  phosphorothiate Internucleoside linkages (1)..(14)
  LNA nucleosides (1)..(3)
  LNA nucleosides (12)..(14)
tgttcccaagaata

SEQ ID NO: 581 - DNA, 15 bp, Artificial Sequence
  LNA antisense gapmer oligonucleotide
  phosphorothiate Internucleoside linkages (1)..(15)
  LNA nucleosides (1)..(3)
  LNA nucleosides (13)..(15)
ttgttcccaagaata

SEQ ID NO: 582 - DNA, 13 bp, Artificial Sequence
  LNA antisense gapmer oligonucleotide
  phosphorothiate Internucleoside linkages (1)..(13)
  LNA nucleosides (1)..(3)
  LNA nucleosides (12)..(13)
tgttcccaagaat

SEQ ID NO: 583 - DNA, 14 bp, Artificial Sequence
  LNA antisense gapmer oligonucleotide
  phosphorothiate Internucleoside linkages (1)..(14)
  LNA nucleosides (1)..(3)
  LNA nucleosides (12)..(14)
ttgttcccaagaat

SEQ ID NO: 584 - DNA, 16 bp, Artificial Sequence
  LNA antisense gapmer oligonucleotide
  phosphorothiate Internucleoside linkages (1)..(16)
  LNA nucleosides (1)..(4)
  LNA nucleosides (13)..(16)
gaggcatagcagcagg

SEQ ID NO: 585 - DNA, 15 bp, Artificial Sequence
  LNA antisense gapmer oligonucleotide
  phosphorothiate Internucleoside linkages (1)..(15)
  LNA nucleosides (1)..(3)
  LNA nucleosides (12)..(15)
gaaccactgaacaaa

SEQ ID NO: 586 - DNA, 15 bp, Artificial Sequence
  LNA antisense gapmer oligonucleotide
  phosphorothiate Internucleoside linkages (1)..(15)
  LNA nucleosides (1)..(4)
  LNA nucleosides (13)..(15)
gaaccactgaacaaa

SEQ ID NO: 587 - DNA, 16 bp, Artificial Sequence
  LNA antisense gapmer oligonucleotide
  phosphorothiate Internucleoside linkages (1)..(16)
  LNA nucleosides (1)..(2)
  LNA nucleosides (13)..(16)
cgaaccactgaacaaa

SEQ ID NO: 588 - DNA, 16 bp, Artificial Sequence
  LNA antisense gapmer oligonucleotide
  phosphorothiate Internucleoside linkages (1)..(16)
  LNA nucleosides (1)..(4)
  LNA nucleosides (14)..(16)
cgaaccactgaacaaa

SEQ ID NO: 589 - DNA, 16 bp, Artificial Sequence
  LNA antisense gapmer oligonucleotide
  phosphorothiate Internucleoside linkages (1)..(16)
  LNA nucleosides (1)..(3)
  LNA nucleosides (13)..(16)
cgaaccactgaacaaa

SEQ ID NO: 590 - DNA, 16 bp, Artificial Sequence
  LNA antisense gapmer oligonucleotide
  phosphorothiate Internucleoside linkages (1)..(16)
  LNA nucleosides (1)..(4)
  LNA nucleosides (15)..(16)
cgaaccactgaacaaa

SEQ ID NO: 591 - DNA, 16 bp, Artificial Sequence
  LNA antisense gapmer oligonucleotide
  phosphorothiate Internucleoside linkages (1)..(16)
  LNA nucleosides (1)..(4)
  LNA nucleosides (13)..(16)
cgaaccactgaacaaa

SEQ ID NO: 592 - DNA, 15 bp, Artificial Sequence
  LNA antisense gapmer oligonucleotide
  phosphorothiate Internucleoside linkages (1)..(15)
  LNA nucleosides (1)..(4)
  LNA nucleosides (14)..(15)
cgaaccactgaacaa

SEQ ID NO: 593 - DNA, 15 bp, Artificial Sequence
  LNA antisense gapmer oligonucleotide
  phosphorothiate Internucleoside linkages (1)..(15)
  LNA nucleosides (1)..(4)
  LNA nucleosides (13)..(15)
cgaaccactgaacaa

SEQ ID NO: 594 - DNA, 15 bp, Artificial Sequence
  LNA antisense gapmer oligonucleotide
  phosphorothiate Internucleoside linkages (1)..(15)
  LNA nucleosides (1)..(3)
  LNA nucleosides (12)..(15)
cgaaccactgaacaa

SEQ ID NO: 595 - DNA, 14 bp, Artificial Sequence
  LNA antisense gapmer oligonucleotide
  phosphorothiate Internucleoside linkages (1)..(14)
  LNA nucleosides (1)..(2)
  LNA nucleosides (11)..(14)
cgaaccactgaaca

SEQ ID NO: 596 - DNA, 14 bp, Artificial Sequence
  LNA antisense gapmer oligonucleotide
  phosphorothiate Internucleoside linkages (1)..(14)
  LNA nucleosides (1)..(4)
  LNA nucleosides (13)..(14)
cgaaccactgaaca

SEQ ID NO: 597 - DNA, 14 bp, Artificial Sequence
  LNA antisense gapmer oligonucleotide
  phosphorothiate Internucleoside linkages (1)..(14)
  LNA nucleosides (1)..(3)
  LNA nucleosides (11)..(14)
cgaaccactgaaca

SEQ ID NO: 598 - DNA, 14 bp, Artificial Sequence
  LNA antisense gapmer oligonucleotide
  phosphorothiate Internucleoside linkages (1)..(14)
  LNA nucleosides (1)..(4)
  LNA nucleosides (12)..(14)
cgaaccactgaaca

SEQ ID NO: 599 - DNA, 13 bp, Artificial Sequence
  LNA antisense gapmer oligonucleotide
  phosphorothiate Internucleoside linkages (1)..(13)
  LNA nucleosides (1)..(2)
  LNA nucleosides (11)..(13)
cgaaccactgaac

SEQ ID NO: 600 - DNA, 13 bp, Artificial Sequence
  LNA antisense gapmer oligonucleotide
  phosphorothiate Internucleoside linkages (1)..(13)
  LNA nucleosides (1)..(3)
  LNA nucleosides (11)..(13)
cgaaccactgaac

SEQ ID NO: 601 - DNA, 15 bp, Artificial Sequence
  LNA antisense gapmer oligonucleotide
  phosphorothiate Internucleoside linkages (1)..(15)
  LNA nucleosides (1)..(2)
  LNA nucleosides (12)..(15)
ccgcagtatggatcg

SEQ ID NO: 602 - DNA, 15 bp, Artificial Sequence
  LNA antisense gapmer oligonucleotide
  phosphorothiate Internucleoside linkages (1)..(15)
  LNA nucleosides (1)..(4)
  LNA nucleosides (14)..(15)
ccgcagtatggatcg

SEQ ID NO: 603 - DNA, 15 bp, Artificial Sequence
  LNA antisense gapmer oligonucleotide
  phosphorothiate Internucleoside linkages (1)..(15)
  LNA nucleosides (1)..(4)
  LNA nucleosides (13)..(15)
ccgcagtatggatcg

SEQ ID NO: 604 - DNA, 15 bp, Artificial Sequence
  LNA antisense gapmer oligonucleotide
  phosphorothiate Internucleoside linkages (1)..(15)
  LNA nucleosides (1)..(3)
  LNA nucleosides (12)..(15)
ccgcagtatggatcg

SEQ ID NO: 605 - DNA, 13 bp, Artificial Sequence
  LNA antisense gapmer oligonucleotide
  phosphorothiate Internucleoside linkages (1)..(13)
  LNA nucleosides (1)..(4)
  LNA nucleosides (12)..(13)
cgcagtatggatc

SEQ ID NO: 606 - DNA, 13 bp, Artificial Sequence
  LNA antisense gapmer oligonucleotide
  phosphorothiate Internucleoside linkages (1)..(13)
  LNA nucleosides (1)..(2)
  LNA nucleosides (11)..(13)
cgcagtatggatc

SEQ ID NO: 607 - DNA, 13 bp, Artificial Sequence
  LNA antisense gapmer oligonucleotide
  phosphorothiate Internucleoside linkages (1)..(13)
  LNA nucleosides (1)..(3)
  LNA nucleosides (11)..(13)
cgcagtatggatc

SEQ ID NO: 608 - DNA, 13 bp, Artificial Sequence
  LNA antisense gapmer oligonucleotide
  phosphorothiate Internucleoside linkages (1)..(13)
  LNA nucleosides (1)..(2)
  LNA nucleosides (10)..(13)
cgcagtatggatc

SEQ ID NO: 609 - DNA, 14 bp, Artificial Sequence
  LNA antisense gapmer oligonucleotide
  phosphorothiate Internucleoside linkages (1)..(14)
  LNA nucleosides (1)..(4)
  LNA nucleosides (13)..(14)
gcgtaaagagaggt

SEQ ID NO: 610 - DNA, 14 bp, Artificial Sequence
  LNA antisense gapmer oligonucleotide
  phosphorothiate Internucleoside linkages (1)..(14)
  LNA nucleosides (1)..(2)
  LNA nucleosides (11)..(14)
gcgtaaagagaggt

SEQ ID NO: 611 - DNA, 14 bp, Artificial Sequence
  LNA antisense gapmer oligonucleotide
  phosphorothiate Internucleoside linkages (1)..(14)
  LNA nucleosides (1)..(3)
  LNA nucleosides (11)..(14)
gcgtaaagagaggt

SEQ ID NO: 612 - DNA, 14 bp, Artificial Sequence
  LNA antisense gapmer oligonucleotide
  phosphorothiate Internucleoside linkages (1)..(14)
  LNA nucleosides (1)..(4)
  LNA nucleosides (12)..(14)
gcgtaaagagaggt

SEQ ID NO: 613 - DNA, 15 bp, Artificial Sequence
  LNA antisense gapmer oligonucleotide
  phosphorothiate Internucleoside linkages (1)..(15)
  LNA nucleosides (1)..(4)
  LNA nucleosides (14)..(15)
cgcgtaaagagaggt

SEQ ID NO: 614 - DNA, 15 bp, Artificial Sequence
  LNA antisense gapmer oligonucleotide
  phosphorothiate Internucleoside linkages (1)..(15)
  LNA nucleosides (1)..(2)
  LNA nucleosides (12)..(15)
cgcgtaaagagaggt

SEQ ID NO: 615 - DNA, 15 bp, Artificial Sequence
  LNA antisense gapmer oligonucleotide
  phosphorothiate Internucleoside linkages (1)..(15)
  LNA nucleosides (1)..(4)
  LNA nucleosides (13)..(15)
cgcgtaaagagaggt

SEQ ID NO: 616 - DNA, 15 bp, Artificial Sequence
  LNA antisense gapmer oligonucleotide
  phosphorothiate Internucleoside linkages (1)..(15)
  LNA nucleosides (1)..(3)
  LNA nucleosides (12)..(15)
cgcgtaaagagaggt

SEQ ID NO: 617 - DNA, 13 bp, Artificial Sequence
  LNA antisense gapmer oligonucleotide
  phosphorothiate Internucleoside linkages (1)..(13)
  LNA nucleosides (1)..(2)
  LNA nucleosides (11)..(13)
gcgtaaagagagg

SEQ ID NO: 618 - DNA, 13 bp, Artificial Sequence
  LNA antisense gapmer oligonucleotide
  phosphorothiate Internucleoside linkages (1)..(13)
  LNA nucleosides (1)..(3)
  LNA nucleosides (11)..(13)
gcgtaaagagagg

SEQ ID NO: 619 - DNA, 13 bp, Artificial Sequence
  LNA antisense gapmer oligonucleotide
  phosphorothiate Internucleoside linkages (1)..(13)
  LNA nucleosides (1)..(2)
  LNA nucleosides (10)..(13)
gcgtaaagagagg

SEQ ID NO: 620 - DNA, 13 bp, Artificial Sequence
  LNA antisense gapmer oligonucleotide
  phosphorothiate Internucleoside linkages (1)..(13)
  LNA nucleosides (1)..(4)
  LNA nucleosides (12)..(13)
gcgtaaagagagg

SEQ ID NO: 621 - DNA, 15 bp, Artificial Sequence
  LNA antisense gapmer oligonucleotide
  phosphorothiate Internucleoside linkages (1)..(15)
  LNA nucleosides (1)..(2)
  LNA nucleosides (12)..(15)
agaaggcacagacgg

SEQ ID NO: 622 - DNA, 15 bp, Artificial Sequence
  LNA antisense gapmer oligonucleotide
  phosphorothiate Internucleoside linkages (1)..(15)
  LNA nucleosides (1)..(3)
  LNA nucleosides (12)..(15)
agaaggcacagacgg

SEQ ID NO: 623 - DNA, 15 bp, Artificial Sequence
  LNA antisense gapmer oligonucleotide
  phosphorothiate Internucleoside linkages (1)..(15)
  LNA nucleosides (1)..(4)
  LNA nucleosides (13)..(15)
agaaggcacagacgg

SEQ ID NO: 624 - DNA, 16 bp, Artificial Sequence
  LNA antisense gapmer oligonucleotide
  phosphorothiate Internucleoside linkages (1)..(16)
  LNA nucleosides (1)..(4)
  LNA nucleosides (14)..(16)
gagaaggcacagacgg

SEQ ID NO: 625 - DNA, 16 bp, Artificial Sequence
  LNA antisense gapmer oligonucleotide
  phosphorothiate Internucleoside linkages (1)..(16)
  LNA nucleosides (1)..(3)
  LNA nucleosides (13)..(16)
gagaaggcacagacgg

SEQ ID NO: 626 - DNA, 16 bp, Artificial Sequence
  LNA antisense gapmer oligonucleotide
  phosphorothiate Internucleoside linkages (1)..(16)
  LNA nucleosides (1)..(4)
  LNA nucleosides (13)..(16)
gagaaggcacagacgg

SEQ ID NO: 627 - DNA, 13 bp, Artificial Sequence
  LNA antisense gapmer oligonucleotide
  phosphorothiate Internucleoside linkages (1)..(13)
  LNA nucleosides (1)..(2)
  LNA nucleosides (11)..(13)
gaagtgcacacgg

SEQ ID NO: 628 - DNA, 13 bp, Artificial Sequence
  LNA antisense gapmer oligonucleotide
  phosphorothiate Internucleoside linkages (1)..(13)
  LNA nucleosides (1)..(3)
  LNA nucleosides (11)..(13)
gaagtgcacacgg

SEQ ID NO: 629 - DNA, 13 bp, Artificial Sequence
  LNA antisense gapmer oligonucleotide
  phosphorothiate Internucleoside linkages (1)..(13)
  LNA nucleosides (1)..(4)
  LNA nucleosides (11)..(13)
gaagtgcacacgg

SEQ ID NO: 630 - DNA, 13 bp, Artificial Sequence
  LNA antisense gapmer oligonucleotide
  phosphorothiate Internucleoside linkages (1)..(13)
  LNA nucleosides (1)..(3)
  LNA nucleosides (10)..(13)
gaagtgcacacgg

SEQ ID NO: 631 - DNA, 15 bp, Artificial Sequence
  LNA antisense gapmer oligonucleotide
  phosphorothiate Internucleoside linkages (1)..(15)
  LNA nucleosides (1)..(2)
  LNA nucleosides (13)..(15)
gcgaagtgcacacgg

SEQ ID NO: 632 - DNA, 15 bp, Artificial Sequence
  LNA antisense gapmer oligonucleotide
  phosphorothiate Internucleoside linkages (1)..(15)
  LNA nucleosides (1)..(3)
  LNA nucleosides (14)..(15)
gcgaagtgcacacgg

SEQ ID NO: 633 - DNA, 15 bp, Artificial Sequence
  LNA antisense gapmer oligonucleotide
  phosphorothiate Internucleoside linkages (1)..(15)
  LNA nucleosides (1)..(4)
  LNA nucleosides (14)..(15)
gcgaagtgcacacgg

SEQ ID NO: 634 - DNA, 15 bp, Artificial Sequence
  LNA antisense gapmer oligonucleotide
  phosphorothiate Internucleoside linkages (1)..(15)
  LNA nucleosides (1)..(2)
  LNA nucleosides (12)..(15)
gcgaagtgcacacgg

SEQ ID NO: 635 - DNA, 16 bp, Artificial Sequence
  LNA antisense gapmer oligonucleotide
  phosphorothiate Internucleoside linkages (1)..(16)
  LNA nucleosides (1)..(4)
  LNA nucleosides (15)..(16)
agcgaagtgcacacgg

SEQ ID NO: 636 - DNA, 16 bp, Artificial Sequence
  LNA antisense gapmer oligonucleotide
  phosphorothiate Internucleoside linkages (1)..(16)
  LNA nucleosides (1)..(2)
  5-methyl c (3)..(3)
  LNA nucleosides (13)..(16)
agcgaagtgcacacgg

SEQ ID NO: 637 - DNA, 16 bp, Artificial Sequence
  LNA antisense gapmer oligonucleotide
  phosphorothiate Internucleoside linkages (1)..(16)
  LNA nucleosides (1)..(2)
  5-methyl c (3)..(3)
  LNA nucleosides (14)..(16)
agcgaagtgcacacgg

SEQ ID NO: 638 - DNA, 16 bp, Artificial Sequence
  LNA antisense gapmer oligonucleotide
  phosphorothiate Internucleoside linkages (1)..(16)
  LNA nucleosides (1)..(3)
  LNA nucleosides (15)..(16)
agcgaagtgcacacgg

SEQ ID NO: 639 - DNA, 13 bp, Artificial Sequence
  LNA antisense gapmer oligonucleotide
  phosphorothiate Internucleoside linkages (1)..(13)
  LNA nucleosides (1)..(2)
  LNA nucleosides (10)..(13)
cgaagtgcacacg

SEQ ID NO: 640 - DNA, 13 bp, Artificial Sequence
  LNA antisense gapmer oligonucleotide
  phosphorothiate Internucleoside linkages (1)..(13)
  LNA nucleosides (1)..(3)
  LNA nucleosides (11)..(13)
cgaagtgcacacg

SEQ ID NO: 641 - DNA, 13 bp, Artificial Sequence
  LNA antisense gapmer oligonucleotide
  phosphorothiate Internucleoside linkages (1)..(13)
  LNA nucleosides (1)..(2)
  LNA nucleosides (11)..(13)
cgaagtgcacacg

SEQ ID NO: 642 - DNA, 15 bp, Artificial Sequence
  LNA antisense gapmer oligonucleotide
  phosphorothiate Internucleoside linkages (1)..(15)
  LNA nucleosides (1)..(3)
  LNA nucleosides (12)..(15)
agcgaagtgcacacg

SEQ ID NO: 643 - DNA, 15 bp, Artificial Sequence
  LNA antisense gapmer oligonucleotide
  phosphorothiate Internucleoside linkages (1)..(15)
  LNA nucleosides (1)..(4)
  LNA nucleosides (13)..(15)
agcgaagtgcacacg

SEQ ID NO: 644 - DNA, 15 bp, Artificial Sequence
  LNA antisense gapmer oligonucleotide
  phosphorothiate Internucleoside linkages (1)..(15)
  LNA nucleosides (1)..(4)
  LNA nucleosides (14)..(15)
agcgaagtgcacacg

SEQ ID NO: 645 - DNA, 15 bp, Artificial Sequence
  LNA antisense gapmer oligonucleotide
  phosphorothiate Internucleoside linkages (1)..(15)
  LNA nucleosides (1)..(2)
  5-methyl c (3)..(3)
  LNA nucleosides (12)..(15)
agcgaagtgcacacg

SEQ ID NO: 646 - DNA, 16 bp, Artificial Sequence
  LNA antisense gapmer oligonucleotide
  phosphorothiate Internucleoside linkages (1)..(16)
  LNA nucleosides (1)..(2)
  5-methyl c (4)..(4)
  LNA nucleosides (13)..(16)
aagcgaagtgcacacg

SEQ ID NO: 647 - DNA, 16 bp, Artificial Sequence
  LNA antisense gapmer oligonucleotide
  phosphorothiate Internucleoside linkages (1)..(16)
  LNA nucleosides (1)..(4)
  LNA nucleosides (15)..(16)
aagcgaagtgcacacg

SEQ ID NO: 648 - DNA, 16 bp, Artificial Sequence
  LNA antisense gapmer oligonucleotide
  phosphorothiate Internucleoside linkages (1)..(16)
  LNA nucleosides (1)..(3)
  5-methyl c (4)..(4)
  LNA nucleosides (13)..(16)
aagcgaagtgcacacg

SEQ ID NO: 649 - DNA, 16 bp, Artificial Sequence
  LNA antisense gapmer oligonucleotide
  phosphorothiate Internucleoside linkages (1)..(16)
  LNA nucleosides (1)..(4)
  LNA nucleosides (14)..(16)
aagcgaagtgcacacg

SEQ ID NO: 650 - DNA, 16 bp, Artificial Sequence
  LNA antisense gapmer oligonucleotide
  phosphorothiate Internucleoside linkages (1)..(16)
  LNA nucleosides (1)..(4)
  LNA nucleosides (13)..(16)
aagcgaagtgcacacg

SEQ ID NO: 651 - DNA, 15 bp, Artificial Sequence
  LNA antisense gapmer oligonucleotide
  phosphorothiate Internucleoside linkages (1)..(15)
  LNA nucleosides (1)..(2)
  5-methyl c (5)..(5)
  LNA nucleosides (12)..(15)
gaagcgaagtgcaca

SEQ ID NO: 652 - DNA, 15 bp, Artificial Sequence
  LNA antisense gapmer oligonucleotide
  phosphorothiate Internucleoside linkages (1)..(15)
  LNA nucleosides (1)..(4)
  5-methyl c (5)..(5)
  LNA nucleosides (14)..(15)
gaagcgaagtgcaca

SEQ ID NO: 653 - DNA, 15 bp, Artificial Sequence
  LNA antisense gapmer oligonucleotide
  phosphorothiate Internucleoside linkages (1)..(15)
  LNA nucleosides (1)..(3)
  5-methyl c (5)..(5)
  LNA nucleosides (12)..(15)
gaagcgaagtgcaca

SEQ ID NO: 654 - DNA, 15 bp, Artificial Sequence
  LNA antisense gapmer oligonucleotide
  phosphorothiate Internucleoside linkages (1)..(15)
  LNA nucleosides (1)..(4)
  5-methyl c (5)..(5)
  LNA nucleosides (12)..(15)
gaagcgaagtgcaca

SEQ ID NO: 655 - DNA, 16 bp, Artificial Sequence
  LNA antisense gapmer oligonucleotide
  phosphorothiate Internucleoside linkages (1)..(16)
  LNA nucleosides (1)..(2)
  5-methyl c (8)..(8)
  LNA nucleosides (14)..(16)
ggtgaagcgaagtgca

SEQ ID NO: 656 - DNA, 16 bp, Artificial Sequence
  LNA antisense gapmer oligonucleotide
  phosphorothiate Internucleoside linkages (1)..(16)
  LNA nucleosides (1)..(3)
  5-methyl c (8)..(8)
  LNA nucleosides (15)..(16)
ggtgaagcgaagtgca

SEQ ID NO: 657 - DNA, 16 bp, Artificial Sequence
  LNA antisense gapmer oligonucleotide
  phosphorothiate Internucleoside linkages (1)..(16)
  LNA nucleosides (1)..(4)
  5-methyl c (8)..(8)
  LNA nucleosides (15)..(16)
ggtgaagcgaagtgca

SEQ ID NO: 658 - DNA, 16 bp, Artificial Sequence
  LNA antisense gapmer oligonucleotide
  phosphorothiate Internucleoside linkages (1)..(16)
  LNA nucleosides (1)..(2)
  5-methyl c (8)..(8)
  LNA nucleosides (13)..(16)
ggtgaagcgaagtgca

SEQ ID NO: 659 - DNA, 15 bp, Artificial Sequence
  LNA antisense gapmer oligonucleotide
  phosphorothiate Internucleoside linkages (1)..(15)
  LNA nucleosides (1)..(2)
  5-methyl c (8)..(8)
  LNA nucleosides (13)..(15)
ggtgaagcgaagtgc

SEQ ID NO: 660 - DNA, 15 bp, Artificial Sequence
  LNA antisense gapmer oligonucleotide
  phosphorothiate Internucleoside linkages (1)..(15)
  LNA nucleosides (1)..(3)
  5-methyl c (8)..(8)
  LNA nucleosides (14)..(15)
ggtgaagcgaagtgc

SEQ ID NO: 661 - DNA, 15 bp, Artificial Sequence
  LNA antisense gapmer oligonucleotide
  phosphorothiate Internucleoside linkages (1)..(15)
  LNA nucleosides (1)..(4)
  5-methyl c (8)..(8)
  LNA nucleosides (14)..(15)
ggtgaagcgaagtgc

SEQ ID NO: 662 - DNA, 15 bp, Artificial Sequence
  LNA antisense gapmer oligonucleotide
  phosphorothiate Internucleoside linkages (1)..(15)
  LNA nucleosides (1)..(2)
  5-methyl c (8)..(8)
  LNA nucleosides (12)..(15)
ggtgaagcgaagtgc

SEQ ID NO: 663 - DNA, 16 bp, Artificial Sequence
  LNA antisense gapmer oligonucleotide
  phosphorothiate Internucleoside linkages (1)..(16)
  LNA nucleosides (1)..(2)
  5-methyl c (9)..(9)
  LNA nucleosides (14)..(16)
aggtgaagcgaagtgc

SEQ ID NO: 664 - DNA, 16 bp, Artificial Sequence
  LNA antisense gapmer oligonucleotide
  phosphorothiate Internucleoside linkages (1)..(16)
  LNA nucleosides (1)..(3)
  5-methyl c (9)..(9)
  LNA nucleosides (15)..(16)
aggtgaagcgaagtgc

SEQ ID NO: 665 - DNA, 16 bp, Artificial Sequence
  LNA antisense gapmer oligonucleotide
  phosphorothiate Internucleoside linkages (1)..(16)
  LNA nucleosides (1)..(4)
  5-methyl c (9)..(9)
  LNA nucleosides (15)..(16)
aggtgaagcgaagtgc

SEQ ID NO: 666 - DNA, 16 bp, Artificial Sequence
  LNA antisense gapmer oligonucleotide
  phosphorothiate Internucleoside linkages (1)..(16)
  LNA nucleosides (1)..(2)
  5-methyl c (9)..(9)
  LNA nucleosides (13)..(16)
aggtgaagcgaagtgc

SEQ ID NO: 667 - DNA, 15 bp, Artificial Sequence
  LNA antisense gapmer oligonucleotide
  phosphorothiate Internucleoside linkages (1)..(15)
  LNA nucleosides (1)..(4)
  5-methyl c (9)..(9)
  LNA nucleosides (14)..(15)
aggtgaagcgaagtg

SEQ ID NO: 668 - DNA, 15 bp, Artificial Sequence
  LNA antisense gapmer oligonucleotide
  phosphorothiate Internucleoside linkages (1)..(15)
  LNA nucleosides (1)..(2)
  5-methyl c (9)..(9)
  LNA nucleosides (12)..(15)
aggtgaagcgaagtg

SEQ ID NO: 669 - DNA, 15 bp, Artificial Sequence
  LNA antisense gapmer oligonucleotide
  phosphorothiate Internucleoside linkages (1)..(15)
  LNA nucleosides (1)..(3)
  5-methyl c (9)..(9)
  LNA nucleosides (12)..(15)
aggtgaagcgaagtg

SEQ ID NO: 670 - DNA, 15 bp, Artificial Sequence
  LNA antisense gapmer oligonucleotide
  phosphorothiate Internucleoside linkages (1)..(15)
  LNA nucleosides (1)..(4)
  5-methyl c (9)..(9)
  LNA nucleosides (13)..(15)
aggtgaagcgaagtg

SEQ ID NO: 671 - DNA, 14 bp, Artificial Sequence
  LNA antisense gapmer oligonucleotide
  phosphorothiate Internucleoside linkages (1)..(14)
  LNA nucleosides (1)..(4)
  5-methyl c (9)..(9)
  LNA nucleosides (13)..(14)
aggtgaagcgaagt

SEQ ID NO: 672 - DNA, 14 bp, Artificial Sequence
  LNA antisense gapmer oligonucleotide
  phosphorothiate Internucleoside linkages (1)..(14)
  LNA nucleosides (1)..(2)
  5-methyl c (9)..(9)
  LNA nucleosides (11)..(14)
aggtgaagcgaagt

SEQ ID NO: 673 - DNA, 14 bp, Artificial Sequence
  LNA antisense gapmer oligonucleotide
  phosphorothiate Internucleoside linkages (1)..(14)
  LNA nucleosides (1)..(3)
  5-methyl c (9)..(9)
  LNA nucleosides (11)..(14)
aggtgaagcgaagt

SEQ ID NO: 674 - DNA, 14 bp, Artificial Sequence
  LNA antisense gapmer oligonucleotide
  phosphorothiate Internucleoside linkages (1)..(14)
  LNA nucleosides (1)..(4)
  5-methyl c (9)..(9)
  LNA nucleosides (12)..(14)
aggtgaagcgaagt

SEQ ID NO: 675 - DNA, 14 bp, Artificial Sequence
  LNA antisense gapmer oligonucleotide
  phosphorothiate Internucleoside linkages (1)..(14)
  LNA nucleosides (1)..(4)
  LNA nucleosides (13)..(14)
cagaggtgaagcga

SEQ ID NO: 676 - DNA, 14 bp, Artificial Sequence
  LNA antisense gapmer oligonucleotide
  phosphorothiate Internucleoside linkages (1)..(14)
  LNA nucleosides (1)..(2)
  LNA nucleosides (11)..(14)
cagaggtgaagcga

SEQ ID NO: 677 - DNA, 14 bp, Artificial Sequence
  LNA antisense gapmer oligonucleotide
  phosphorothiate Internucleoside linkages (1)..(14)
  LNA nucleosides (1)..(3)
  LNA nucleosides (11)..(14)
cagaggtgaagcga

SEQ ID NO: 678 - DNA, 15 bp, Artificial Sequence
  LNA antisense gapmer oligonucleotide
  phosphorothiate Internucleoside linkages (1)..(15)
  LNA nucleosides (1)..(3)
  LNA nucleosides (13)..(15)
tagtaaactgagcca

SEQ ID NO: 679 - DNA, 15 bp, Artificial Sequence
  LNA antisense gapmer oligonucleotide
  phosphorothiate Internucleoside linkages (1)..(15)
  LNA nucleosides (1)..(2)
  LNA nucleosides (12)..(15)
tagtaaactgagcca

SEQ ID NO: 680 - DNA, 15 bp, Artificial Sequence
  LNA antisense gapmer oligonucleotide
  phosphorothiate Internucleoside linkages (1)..(15)
  LNA nucleosides (1)..(4)
  LNA nucleosides (14)..(15)
tagtaaactgagcca

SEQ ID NO: 681 - DNA, 15 bp, Artificial Sequence
  LNA antisense gapmer oligonucleotide
  phosphorothiate Internucleoside linkages (1)..(15)
  LNA nucleosides (1)..(3)
  LNA nucleosides (12)..(15)
tagtaaactgagcca

SEQ ID NO: 682 - DNA, 15 bp, Artificial Sequence
  LNA antisense gapmer oligonucleotide
  phosphorothiate Internucleoside linkages (1)..(15)
  LNA nucleosides (1)..(4)
  LNA nucleosides (13)..(15)
tagtaaactgagcca

SEQ ID NO: 683 - DNA, 16 bp, Artificial Sequence
  LNA antisense gapmer oligonucleotide
  phosphorothiate Internucleoside linkages (1)..(16)
  LNA nucleosides (1)..(3)
  LNA nucleosides (14)..(16)
ctagtaaactgagcca

SEQ ID NO: 684 - DNA, 16 bp, Artificial Sequence
  LNA antisense gapmer oligonucleotide
  phosphorothiate Internucleoside linkages (1)..(16)
  LNA nucleosides (1)..(2)
  LNA nucleosides (13)..(16)
ctagtaaactgagcca

SEQ ID NO: 685 - DNA, 16 bp, Artificial Sequence
  LNA antisense gapmer oligonucleotide
  phosphorothiate Internucleoside linkages (1)..(16)
  LNA nucleosides (1)..(4)
  LNA nucleosides (15)..(16)
ctagtaaactgagcca

SEQ ID NO: 686 - DNA, 15 bp, Artificial Sequence
  LNA antisense gapmer oligonucleotide
  phosphorothiate Internucleoside linkages (1)..(15)
  LNA nucleosides (1)..(3)
  LNA nucleosides (13)..(15)
ctagtaaactgagcc

SEQ ID NO: 687 - DNA, 15 bp, Artificial Sequence
  LNA antisense gapmer oligonucleotide
  phosphorothiate Internucleoside linkages (1)..(15)
  LNA nucleosides (1)..(2)
  LNA nucleosides (12)..(15)
ctagtaaactgagcc

SEQ ID NO: 688 - DNA, 15 bp, Artificial Sequence
  LNA antisense gapmer oligonucleotide
  phosphorothiate Internucleoside linkages (1)..(15)
  LNA nucleosides (1)..(4)
  LNA nucleosides (14)..(15)
ctagtaaactgagcc

SEQ ID NO: 689 - DNA, 15 bp, Artificial Sequence
  LNA antisense gapmer oligonucleotide
  phosphorothiate Internucleoside linkages (1)..(15)
  LNA nucleosides (1)..(2)
  LNA nucleosides (13)..(15)
ctagtaaactgagcc

SEQ ID NO: 690 - DNA, 15 bp, Artificial Sequence
  LNA antisense gapmer oligonucleotide
  phosphorothiate Internucleoside linkages (1)..(15)
  LNA nucleosides (1)..(3)
  LNA nucleosides (14)..(15)
ctagtaaactgagcc

SEQ ID NO: 691 - DNA, 15 bp, Artificial Sequence
  LNA antisense gapmer oligonucleotide
  phosphorothiate Internucleoside linkages (1)..(15)
  LNA nucleosides (1)..(3)
  LNA nucleosides (13)..(15)
gcactagtaaactga

SEQ ID NO: 692 - DNA, 15 bp, Artificial Sequence
  LNA antisense gapmer oligonucleotide
  phosphorothiate Internucleoside linkages (1)..(15)
  LNA nucleosides (1)..(2)
  LNA nucleosides (12)..(15)
gcactagtaaactga

SEQ ID NO: 693 - DNA, 15 bp, Artificial Sequence
  LNA antisense gapmer oligonucleotide
  phosphorothiate Internucleoside linkages (1)..(15)
  LNA nucleosides (1)..(4)
  LNA nucleosides (14)..(15)
gcactagtaaactga

SEQ ID NO: 694 - DNA, 15 bp, Artificial Sequence
  LNA antisense gapmer oligonucleotide
  phosphorothiate Internucleoside linkages (1)..(15)
  LNA nucleosides (1)..(3)
  LNA nucleosides (12)..(15)
gcactagtaaactga

SEQ ID NO: 695 - DNA, 15 bp, Artificial Sequence
  LNA antisense gapmer oligonucleotide
  phosphorothiate Internucleoside linkages (1)..(15)
  LNA nucleosides (1)..(4)
  LNA nucleosides (13)..(15)
gcactagtaaactga

SEQ ID NO: 696 - DNA, 16 bp, Artificial Sequence
  LNA antisense gapmer oligonucleotide
  phosphorothiate Internucleoside linkages (1)..(16)
  LNA nucleosides (1)..(3)
  LNA nucleosides (14)..(16)
ggcactagtaaactga

SEQ ID NO: 697 - DNA, 16 bp, Artificial Sequence
  LNA antisense gapmer oligonucleotide
  phosphorothiate Internucleoside linkages (1)..(16)
  LNA nucleosides (1)..(2)
  LNA nucleosides (13)..(16)
ggcactagtaaactga

SEQ ID NO: 698 - DNA, 16 bp, Artificial Sequence
  LNA antisense gapmer oligonucleotide
  phosphorothiate Internucleoside linkages (1)..(16)
  LNA nucleosides (1)..(4)
  LNA nucleosides (15)..(16)
ggcactagtaaactga

SEQ ID NO: 699 - DNA, 15 bp, Artificial Sequence
  LNA antisense gapmer oligonucleotide
  phosphorothiate Internucleoside linkages (1)..(15)
  LNA nucleosides (1)..(3)
  5-methyl c (4)..(4)
  LNA nucleosides (13)..(15)
caacggggtaaaggt

SEQ ID NO: 700 - DNA, 15 bp, Artificial Sequence
  LNA antisense gapmer oligonucleotide
  phosphorothiate Internucleoside linkages (1)..(15)
  LNA nucleosides (1)..(2)
  5-methyl c (4)..(4)
  LNA nucleosides (12)..(15)
caacggggtaaaggt

SEQ ID NO: 701 - DNA, 15 bp, Artificial Sequence
  LNA antisense gapmer oligonucleotide
  phosphorothiate Internucleoside linkages (1)..(15)
  LNA nucleosides (1)..(4)
  LNA nucleosides (14)..(15)
caacggggtaaaggt

SEQ ID NO: 702 - DNA, 15 bp, Artificial Sequence
  LNA antisense gapmer oligonucleotide
  phosphorothiate Internucleoside linkages (1)..(15)
  LNA nucleosides (1)..(3)
  5-methyl c (4)..(4)
  LNA nucleosides (12)..(15)
caacggggtaaaggt

SEQ ID NO: 703 - DNA, 15 bp, Artificial Sequence
  LNA antisense gapmer oligonucleotide
  phosphorothiate Internucleoside linkages (1)..(15)
  LNA nucleosides (1)..(4)
  LNA nucleosides (13)..(15)
caacggggtaaaggt

SEQ ID NO: 704 - DNA, 15 bp, Artificial Sequence
  LNA antisense gapmer oligonucleotide
  phosphorothiate Internucleoside linkages (1)..(15)
  LNA nucleosides (1)..(3)
  5-methyl c (11)..(11)
  LNA nucleosides (13)..(15)
cagtatggatcggca

SEQ ID NO: 705 - DNA, 15 bp, Artificial Sequence
  LNA antisense gapmer oligonucleotide
  phosphorothiate Internucleoside linkages (1)..(15)
  LNA nucleosides (1)..(2)
  5-methyl c (11)..(11)
  LNA nucleosides (12)..(15)
cagtatggatcggca

SEQ ID NO: 706 - DNA, 15 bp, Artificial Sequence
  LNA antisense gapmer oligonucleotide
  phosphorothiate Internucleoside linkages (1)..(15)
  LNA nucleosides (1)..(2)
  5-methyl c (11)..(11)
  LNA nucleosides (13)..(15)
cagtatggatcggca

SEQ ID NO: 707 - DNA, 15 bp, Artificial Sequence
  LNA antisense gapmer oligonucleotide
  phosphorothiate Internucleoside linkages (1)..(15)
  LNA nucleosides (1)..(3)
  5-methyl c (11)..(11)
  LNA nucleosides (14)..(15)
cagtatggatcggca

SEQ ID NO: 708 - DNA, 16 bp, Artificial Sequence
  LNA antisense gapmer oligonucleotide
  phosphorothiate Internucleoside linkages (1)..(16)
  LNA nucleosides (1)..(3)
  5-methyl c (4)..(4)
  LNA nucleosides (14)..(16)
ttccgcagtatggatc

SEQ ID NO: 709 - DNA, 16 bp, Artificial Sequence
  LNA antisense gapmer oligonucleotide
  phosphorothiate Internucleoside linkages (1)..(16)
  LNA nucleosides (1)..(2)
  5-methyl c (4)..(4)
  LNA nucleosides (13)..(16)
ttccgcagtatggatc

SEQ ID NO: 710 - DNA, 16 bp, Artificial Sequence
  LNA antisense gapmer oligonucleotide
  phosphorothiate Internucleoside linkages (1)..(16)
  LNA nucleosides (1)..(4)
  LNA nucleosides (15)..(16)
ttccgcagtatggatc

SEQ ID NO: 711 - DNA, 16 bp, Artificial Sequence
  LNA antisense gapmer oligonucleotide
  phosphorothiate Internucleoside linkages (1)..(16)
  LNA nucleosides (1)..(3)
  5-methyl c (4)..(4)
  LNA nucleosides (13)..(16)
ttccgcagtatggatc

SEQ ID NO: 712 - DNA, 16 bp, Artificial Sequence
  LNA antisense gapmer oligonucleotide
  phosphorothiate Internucleoside linkages (1)..(16)
  LNA nucleosides (1)..(4)
  LNA nucleosides (14)..(16)
ttccgcagtatggatc

SEQ ID NO: 713 - DNA, 15 bp, Artificial Sequence
  LNA antisense gapmer oligonucleotide
  phosphorothiate Internucleoside linkages (1)..(15)
  LNA nucleosides (1)..(3)
  5-methyl c (4)..(4)
  LNA nucleosides (13)..(15)
ttccgcagtatggat

SEQ ID NO: 714 - DNA, 15 bp, Artificial Sequence
  LNA antisense gapmer oligonucleotide
  phosphorothiate Internucleoside linkages (1)..(15)
  LNA nucleosides (1)..(2)
  5-methyl c (4)..(4)
  LNA nucleosides (12)..(15)
ttccgcagtatggat

SEQ ID NO: 715 - DNA, 15 bp, Artificial Sequence
  LNA antisense gapmer oligonucleotide
  phosphorothiate Internucleoside linkages (1)..(15)
  LNA nucleosides (1)..(4)
  LNA nucleosides (14)..(15)
ttccgcagtatggat

SEQ ID NO: 716 - DNA, 15 bp, Artificial Sequence
  LNA antisense gapmer oligonucleotide
  phosphorothiate Internucleoside linkages (1)..(15)
  LNA nucleosides (1)..(3)
  5-methyl c (4)..(4)
  LNA nucleosides (12)..(15)
ttccgcagtatggat

SEQ ID NO: 717 - DNA, 15 bp, Artificial Sequence
  LNA antisense gapmer oligonucleotide
  phosphorothiate Internucleoside linkages (1)..(15)
  LNA nucleosides (1)..(4)
  LNA nucleosides (13)..(15)
ttccgcagtatggat

SEQ ID NO: 718 - DNA, 16 bp, Artificial Sequence
  LNA antisense gapmer oligonucleotide
  phosphorothiate Internucleoside linkages (1)..(16)
  LNA nucleosides (1)..(3)
  5-methyl c (5)..(5)
  LNA nucleosides (14)..(16)
gttccgcagtatggat

SEQ ID NO: 719 - DNA, 16 bp, Artificial Sequence
  LNA antisense gapmer oligonucleotide
  phosphorothiate Internucleoside linkages (1)..(16)
  LNA nucleosides (1)..(2)
  5-methyl c (5)..(5)
  LNA nucleosides (13)..(16)
gttccgcagtatggat

SEQ ID NO: 720 - DNA, 16 bp, Artificial Sequence
  LNA antisense gapmer oligonucleotide
  phosphorothiate Internucleoside linkages (1)..(16)
  LNA nucleosides (1)..(4)
  5-methyl c (5)..(5)
  LNA nucleosides (15)..(16)
gttccgcagtatggat

SEQ ID NO: 721 - DNA, 15 bp, Artificial Sequence
  LNA antisense gapmer oligonucleotide
  phosphorothiate Internucleoside linkages (1)..(15)
  LNA nucleosides (1)..(2)
  5-methyl c (5)..(5)
  LNA nucleosides (12)..(15)
gttccgcagtatgga

SEQ ID NO: 722 - DNA, 15 bp, Artificial Sequence
  LNA antisense gapmer oligonucleotide
  phosphorothiate Internucleoside linkages (1)..(15)
  LNA nucleosides (1)..(4)
  5-methyl c (5)..(5)
  LNA nucleosides (14)..(15)
gttccgcagtatgga

SEQ ID NO: 723 - DNA, 15 bp, Artificial Sequence
  LNA antisense gapmer oligonucleotide
  phosphorothiate Internucleoside linkages (1)..(15)
  LNA nucleosides (1)..(2)
  5-methyl c (5)..(5)
  LNA nucleosides (13)..(15)
gttccgcagtatgga

SEQ ID NO: 724 - DNA, 15 bp, Artificial Sequence
  LNA antisense gapmer oligonucleotide
  phosphorothiate Internucleoside linkages (1)..(15)
  LNA nucleosides (1)..(3)
  5-methyl c (5)..(5)
  LNA nucleosides (14)..(15)
gttccgcagtatgga

SEQ ID NO: 725 - DNA, 16 bp, Artificial Sequence
  LNA antisense gapmer oligonucleotide
  phosphorothiate Internucleoside linkages (1)..(16)
  LNA nucleosides (1)..(3)
  5-methyl c (6)..(6)
  LNA nucleosides (14)..(16)
agttccgcagtatgga

SEQ ID NO: 726 - DNA, 16 bp, Artificial Sequence
  LNA antisense gapmer oligonucleotide
  phosphorothiate Internucleoside linkages (1)..(16)
  LNA nucleosides (1)..(4)
  5-methyl c (6)..(6)
  LNA nucleosides (15)..(16)
agttccgcagtatgga

SEQ ID NO: 727 - DNA, 16 bp, Artificial Sequence
  LNA antisense gapmer oligonucleotide
  phosphorothiate Internucleoside linkages (1)..(16)
  LNA nucleosides (1)..(2)
  5-methyl c (6)..(6)
  LNA nucleosides (14)..(16)
agttccgcagtatgga

SEQ ID NO: 728 - DNA, 16 bp, Artificial Sequence
  LNA antisense gapmer oligonucleotide
  phosphorothiate Internucleoside linkages (1)..(16)
  LNA nucleosides (1)..(3)
  5-methyl c (6)..(6)
  LNA nucleosides (15)..(16)
agttccgcagtatgga

SEQ ID NO: 729 - DNA, 16 bp, Artificial Sequence
  LNA antisense gapmer oligonucleotide
  phosphorothiate Internucleoside linkages (1)..(16)
  LNA nucleosides (1)..(2)
  5-methyl c (6)..(6)
  LNA nucleosides (15)..(16)
agttccgcagtatgga

SEQ ID NO: 730 - DNA, 15 bp, Artificial Sequence
  LNA antisense gapmer oligonucleotide
  phosphorothiate Internucleoside linkages (1)..(15)
  LNA nucleosides (1)..(3)
  5-methyl c (6)..(6)
  LNA nucleosides (13)..(15)
agttccgcagtatgg

SEQ ID NO: 731 - DNA, 15 bp, Artificial Sequence
  LNA antisense gapmer oligonucleotide
  phosphorothiate Internucleoside linkages (1)..(15)
  LNA nucleosides (1)..(2)
  5-methyl c (6)..(6)
  LNA nucleosides (13)..(15)
agttccgcagtatgg

SEQ ID NO: 732 - DNA, 15 bp, Artificial Sequence
  LNA antisense gapmer oligonucleotide
  phosphorothiate Internucleoside linkages (1)..(15)
  LNA nucleosides (1)..(3)
  5-methyl c (6)..(6)
  LNA nucleosides (14)..(15)
agttccgcagtatgg

SEQ ID NO: 733 - DNA, 15 bp, Artificial Sequence
  LNA antisense gapmer oligonucleotide
  phosphorothiate Internucleoside linkages (1)..(15)
  LNA nucleosides (1)..(2)
  5-methyl c (6)..(6)
  LNA nucleosides (14)..(15)
agttccgcagtatgg

SEQ ID NO: 734 - DNA, 16 bp, Artificial Sequence
  LNA antisense gapmer oligonucleotide
  phosphorothiate Internucleoside linkages (1)..(16)
  LNA nucleosides (1)..(2)
  5-methyl c (7)..(7)
  LNA nucleosides (14)..(16)
gagttccgcagtatgg

SEQ ID NO: 735 - DNA, 16 bp, Artificial Sequence
  LNA antisense gapmer oligonucleotide
  phosphorothiate Internucleoside linkages (1)..(16)
  LNA nucleosides (1)..(3)
  5-methyl c (7)..(7)
  LNA nucleosides (15)..(16)
gagttccgcagtatgg

SEQ ID NO: 736 - DNA, 16 bp, Artificial Sequence
  LNA antisense gapmer oligonucleotide
  phosphorothiate Internucleoside linkages (1)..(16)
  LNA nucleosides (1)..(2)
  5-methyl c (7)..(7)
  LNA nucleosides (15)..(16)
gagttccgcagtatgg

SEQ ID NO: 737 - DNA, 15 bp, Artificial Sequence
  LNA antisense gapmer oligonucleotide
  phosphorothiate Internucleoside linkages (1)..(15)
  LNA nucleosides (1)..(4)
  5-methyl c (7)..(7)
  LNA nucleosides (14)..(15)
gagttccgcagtatg

SEQ ID NO: 738 - DNA, 15 bp, Artificial Sequence
  LNA antisense gapmer oligonucleotide
  phosphorothiate Internucleoside linkages (1)..(15)
  LNA nucleosides (1)..(2)
  5-methyl c (7)..(7)
  LNA nucleosides (13)..(15)
gagttccgcagtatg

SEQ ID NO: 739 - DNA, 15 bp, Artificial Sequence
  LNA antisense gapmer oligonucleotide
  phosphorothiate Internucleoside linkages (1)..(15)
  LNA nucleosides (1)..(3)
  5-methyl c (7)..(7)
  LNA nucleosides (14)..(15)
gagttccgcagtatg

SEQ ID NO: 740 - DNA, 15 bp, Artificial Sequence
  LNA antisense gapmer oligonucleotide
  phosphorothiate Internucleoside linkages (1)..(15)
  LNA nucleosides (1)..(2)
  5-methyl c (7)..(7)
  LNA nucleosides (14)..(15)
gagttccgcagtatg

SEQ ID NO: 741 - DNA, 16 bp, Artificial Sequence
  LNA antisense gapmer oligonucleotide
  phosphorothiate Internucleoside linkages (1)..(16)
  LNA nucleosides (1)..(4)
  5-methyl c (8)..(8)
  LNA nucleosides (15)..(16)
ggagttccgcagtatg

SEQ ID NO: 742 - DNA, 16 bp, Artificial Sequence
  LNA antisense gapmer oligonucleotide
  phosphorothiate Internucleoside linkages (1)..(16)
  LNA nucleosides (1)..(2)
  5-methyl c (8)..(8)
  LNA nucleosides (14)..(16)
ggagttccgcagtatg

SEQ ID NO: 743 - DNA, 16 bp, Artificial Sequence
  LNA antisense gapmer oligonucleotide
  phosphorothiate Internucleoside linkages (1)..(16)
  LNA nucleosides (1)..(3)
  5-methyl c (8)..(8)
  LNA nucleosides (15)..(16)
ggagttccgcagtatg

SEQ ID NO: 744 - DNA, 16 bp, Artificial Sequence
  LNA antisense gapmer oligonucleotide
  phosphorothiate Internucleoside linkages (1)..(16)
  LNA nucleosides (1)..(2)
  5-methyl c (8)..(8)
  LNA nucleosides (15)..(16)
ggagttccgcagtatg

SEQ ID NO: 745 - DNA, 16 bp, Artificial Sequence
  LNA antisense gapmer oligonucleotide
  phosphorothiate Internucleoside linkages (1)..(16)
  LNA nucleosides (1)..(3)
  5-methyl c (13)..(13)
  LNA nucleosides (14)..(16)
taaagagaggtgcgcc

SEQ ID NO: 746 - DNA, 16 bp, Artificial Sequence
  LNA antisense gapmer oligonucleotide
  phosphorothiate Internucleoside linkages (1)..(16)
  LNA nucleosides (1)..(2)
  LNA nucleosides (13)..(16)
taaagagaggtgcgcc

SEQ ID NO: 747 - DNA, 16 bp, Artificial Sequence
  LNA antisense gapmer oligonucleotide
  phosphorothiate Internucleoside linkages (1)..(16)
  LNA nucleosides (1)..(4)
  5-methyl c (13)..(13)
  LNA nucleosides (15)..(16)
taaagagaggtgcgcc

SEQ ID NO: 748 - DNA, 16 bp, Artificial Sequence
  LNA antisense gapmer oligonucleotide
  phosphorothiate Internucleoside linkages (1)..(16)
  LNA nucleosides (1)..(3)
  LNA nucleosides (13)..(16)
taaagagaggtgcgcc

SEQ ID NO: 749 - DNA, 16 bp, Artificial Sequence
  LNA antisense gapmer oligonucleotide
  phosphorothiate Internucleoside linkages (1)..(16)
  LNA nucleosides (1)..(4)
  5-methyl c (13)..(13)
  LNA nucleosides (14)..(16)
taaagagaggtgcgcc

SEQ ID NO: 750 - DNA, 15 bp, Artificial Sequence
  LNA antisense gapmer oligonucleotide
  phosphorothiate Internucleoside linkages (1)..(15)
  LNA nucleosides (1)..(3)
  LNA nucleosides (13)..(15)
taaagagaggtgcgc

SEQ ID NO: 751 - DNA, 15 bp, Artificial Sequence
  LNA antisense gapmer oligonucleotide
  phosphorothiate Internucleoside linkages (1)..(15)
  LNA nucleosides (1)..(2)
  LNA nucleosides (12)..(15)
taaagagaggtgcgc

SEQ ID NO: 752 - DNA, 15 bp, Artificial Sequence
  LNA antisense gapmer oligonucleotide
  phosphorothiate Internucleoside linkages (1)..(15)
  LNA nucleosides (1)..(3)
  LNA nucleosides (12)..(15)
taaagagaggtgcgc

SEQ ID NO: 753 - DNA, 15 bp, Artificial Sequence
  LNA antisense gapmer oligonucleotide
  phosphorothiate Internucleoside linkages (1)..(15)
  LNA nucleosides (1)..(4)
  LNA nucleosides (13)..(15)
taaagagaggtgcgc

SEQ ID NO: 754 - DNA, 16 bp, Artificial Sequence
  LNA antisense gapmer oligonucleotide
  phosphorothiate Internucleoside linkages (1)..(16)
  LNA nucleosides (1)..(3)
  LNA nucleosides (14)..(16)
gtaaagagaggtgcgc

SEQ ID NO: 755 - DNA, 16 bp, Artificial Sequence
  LNA antisense gapmer oligonucleotide
  phosphorothiate Internucleoside linkages (1)..(16)
  LNA nucleosides (1)..(2)
  LNA nucleosides (13)..(16)
gtaaagagaggtgcgc

SEQ ID NO: 756 - DNA, 15 bp, Artificial Sequence
  LNA antisense gapmer oligonucleotide
  phosphorothiate Internucleoside linkages (1)..(15)
  LNA nucleosides (1)..(3)
  LNA nucleosides (13)..(15)
gtaaagagaggtgcg

SEQ ID NO: 757 - DNA, 15 bp, Artificial Sequence
  LNA antisense gapmer oligonucleotide
  phosphorothiate Internucleoside linkages (1)..(15)
  LNA nucleosides (1)..(2)
  LNA nucleosides (12)..(15)
gtaaagagaggtgcg

SEQ ID NO: 758 - DNA, 15 bp, Artificial Sequence
  LNA antisense gapmer oligonucleotide
  phosphorothiate Internucleoside linkages (1)..(15)
  LNA nucleosides (1)..(3)
  LNA nucleosides (12)..(15)
gtaaagagaggtgcg

SEQ ID NO: 759 - DNA, 15 bp, Artificial Sequence
  LNA antisense gapmer oligonucleotide
  phosphorothiate Internucleoside linkages (1)..(15)
  LNA nucleosides (1)..(4)
  LNA nucleosides (13)..(15)
gtaaagagaggtgcg

SEQ ID NO: 760 - DNA, 16 bp, Artificial Sequence
  LNA antisense gapmer oligonucleotide
  phosphorothiate Internucleoside linkages (1)..(16)
  LNA nucleosides (1)..(2)
  LNA nucleosides (13)..(16)
cgtaaagagaggtgcg

SEQ ID NO: 761 - DNA, 16 bp, Artificial Sequence
  LNA antisense gapmer oligonucleotide
  phosphorothiate Internucleoside linkages (1)..(16)
  LNA nucleosides (1)..(4)
  LNA nucleosides (15)..(16)
cgtaaagagaggtgcg

SEQ ID NO: 762 - DNA, 16 bp, Artificial Sequence
  LNA antisense gapmer oligonucleotide
  phosphorothiate Internucleoside linkages (1)..(16)
  LNA nucleosides (1)..(3)
  LNA nucleosides (13)..(16)
cgtaaagagaggtgcg

SEQ ID NO: 763 - DNA, 16 bp, Artificial Sequence
  LNA antisense gapmer oligonucleotide
  phosphorothiate Internucleoside linkages (1)..(16)
  LNA nucleosides (1)..(4)
  LNA nucleosides (14)..(16)
cgtaaagagaggtgcg

SEQ ID NO: 764 - DNA, 15 bp, Artificial Sequence
  LNA antisense gapmer oligonucleotide
  phosphorothiate Internucleoside linkages (1)..(15)
  LNA nucleosides (1)..(3)
  LNA nucleosides (13)..(15)
cgtaaagagaggtgc

SEQ ID NO: 765 - DNA, 15 bp, Artificial Sequence
  LNA antisense gapmer oligonucleotide
  phosphorothiate Internucleoside linkages (1)..(15)
  LNA nucleosides (1)..(2)
  LNA nucleosides (12)..(15)
cgtaaagagaggtgc

SEQ ID NO: 766 - DNA, 15 bp, Artificial Sequence
  LNA antisense gapmer oligonucleotide
  phosphorothiate Internucleoside linkages (1)..(15)
  LNA nucleosides (1)..(4)
  LNA nucleosides (14)..(15)
cgtaaagagaggtgc

SEQ ID NO: 767 - DNA, 15 bp, Artificial Sequence
  LNA antisense gapmer oligonucleotide
  phosphorothiate Internucleoside linkages (1)..(15)
  LNA nucleosides (1)..(3)
  LNA nucleosides (12)..(15)
cgtaaagagaggtgc

SEQ ID NO: 768 - DNA, 15 bp, Artificial Sequence
  LNA antisense gapmer oligonucleotide
  phosphorothiate Internucleoside linkages (1)..(15)
  LNA nucleosides (1)..(4)
  LNA nucleosides (13)..(15)
cgtaaagagaggtgc

SEQ ID NO: 769 - DNA, 16 bp, Artificial Sequence
  LNA antisense gapmer oligonucleotide
  phosphorothiate Internucleoside linkages (1)..(16)
  LNA nucleosides (1)..(3)
  LNA nucleosides (14)..(16)
gcgtaaagagaggtgc

SEQ ID NO: 770 - DNA, 16 bp, Artificial Sequence
  LNA antisense gapmer oligonucleotide
  phosphorothiate Internucleoside linkages (1)..(16)
  LNA nucleosides (1)..(2)
  LNA nucleosides (13)..(16)
gcgtaaagagaggtgc

SEQ ID NO: 771 - DNA, 16 bp, Artificial Sequence
  LNA antisense gapmer oligonucleotide
  phosphorothiate Internucleoside linkages (1)..(16)
  LNA nucleosides (1)..(2)
  LNA nucleosides (14)..(16)
gcgtaaagagaggtgc

SEQ ID NO: 772 - DNA, 16 bp, Artificial Sequence
  LNA antisense gapmer oligonucleotide
  phosphorothiate Internucleoside linkages (1)..(16)
  LNA nucleosides (1)..(3)
  LNA nucleosides (15)..(16)
gcgtaaagagaggtgc

SEQ ID NO: 773 - DNA, 15 bp, Artificial Sequence
  LNA antisense gapmer oligonucleotide
  phosphorothiate Internucleoside linkages (1)..(15)
  LNA nucleosides (1)..(3)
  LNA nucleosides (13)..(15)
gcgtaaagagaggtg

SEQ ID NO: 774 - DNA, 15 bp, Artificial Sequence
  LNA antisense gapmer oligonucleotide
  phosphorothiate Internucleoside linkages (1)..(15)
  LNA nucleosides (1)..(2)
  LNA nucleosides (12)..(15)
gcgtaaagagaggtg

SEQ ID NO: 775 - DNA, 15 bp, Artificial Sequence
  LNA antisense gapmer oligonucleotide
  phosphorothiate Internucleoside linkages (1)..(15)
  LNA nucleosides (1)..(4)
  LNA nucleosides (14)..(15)
gcgtaaagagaggtg

SEQ ID NO: 776 - DNA, 15 bp, Artificial Sequence
  LNA antisense gapmer oligonucleotide
  phosphorothiate Internucleoside linkages (1)..(15)
  LNA nucleosides (1)..(3)
  LNA nucleosides (12)..(15)
gcgtaaagagaggtg

SEQ ID NO: 777 - DNA, 15 bp, Artificial Sequence
  LNA antisense gapmer oligonucleotide
  phosphorothiate Internucleoside linkages (1)..(15)
  LNA nucleosides (1)..(4)
  LNA nucleosides (13)..(15)
gcgtaaagagaggtg

SEQ ID NO: 778 - DNA, 16 bp, Artificial Sequence
  LNA antisense gapmer oligonucleotide
  phosphorothiate Internucleoside linkages (1)..(16)
  LNA nucleosides (1)..(3)
  LNA nucleosides (14)..(16)
cgcgtaaagagaggtg

SEQ ID NO: 779 - DNA, 16 bp, Artificial Sequence
  LNA antisense gapmer oligonucleotide
  phosphorothiate Internucleoside linkages (1)..(16)
  5-methyl c (1)..(1)
  5-methyl c (3)..(3)
  LNA nucleosides (13)..(16)
cgcgtaaagagaggtg

SEQ ID NO: 780 - DNA, 16 bp, Artificial Sequence
  LNA antisense gapmer oligonucleotide
  phosphorothiate Internucleoside linkages (1)..(16)
  LNA nucleosides (1)..(4)
  LNA nucleosides (15)..(16)
cgcgtaaagagaggtg

SEQ ID NO: 781 - DNA, 16 bp, Artificial Sequence
  LNA antisense gapmer oligonucleotide
  phosphorothiate Internucleoside linkages (1)..(16)
  LNA nucleosides (1)..(3)
  LNA nucleosides (13)..(16)
cgcgtaaagagaggtg

SEQ ID NO: 782 - DNA, 16 bp, Artificial Sequence
  LNA antisense gapmer oligonucleotide
  phosphorothiate Internucleoside linkages (1)..(16)
  LNA nucleosides (1)..(4)
  LNA nucleosides (14)..(16)
cgcgtaaagagaggtg

SEQ ID NO: 783 - DNA, 16 bp, Artificial Sequence
  LNA antisense gapmer oligonucleotide
  phosphorothiate Internucleoside linkages (1)..(16)
  LNA nucleosides (1)..(3)
  LNA nucleosides (14)..(16)
tgagaaggcacagacg

SEQ ID NO: 784 - DNA, 16 bp, Artificial Sequence
  LNA antisense gapmer oligonucleotide
  phosphorothiate Internucleoside linkages (1)..(16)
  LNA nucleosides (1)..(2)
  LNA nucleosides (13)..(16)
tgagaaggcacagacg

SEQ ID NO: 785 - DNA, 16 bp, Artificial Sequence
  LNA antisense gapmer oligonucleotide
  phosphorothiate Internucleoside linkages (1)..(16)
  LNA nucleosides (1)..(4)
  LNA nucleosides (15)..(16)
tgagaaggcacagacg

SEQ ID NO: 786 - DNA, 16 bp, Artificial Sequence
  LNA antisense gapmer oligonucleotide
  phosphorothiate Internucleoside linkages (1)..(16)
  LNA nucleosides (1)..(3)
  LNA nucleosides (13)..(16)
tgagaaggcacagacg

SEQ ID NO: 787 - DNA, 16 bp, Artificial Sequence
  LNA antisense gapmer oligonucleotide
  phosphorothiate Internucleoside linkages (1)..(16)
  LNA nucleosides (1)..(4)
  LNA nucleosides (14)..(16)
tgagaaggcacagacg

SEQ ID NO: 788 - DNA, 15 bp, Artificial Sequence
  LNA antisense gapmer oligonucleotide
  phosphorothiate Internucleoside linkages (1)..(15)
  LNA nucleosides (1)..(2)
  5-methyl c (11)..(11)
  LNA nucleosides (13)..(15)
gcctcaaggtcggtc

SEQ ID NO: 789 - DNA, 15 bp, Artificial Sequence
  LNA antisense gapmer oligonucleotide
  phosphorothiate Internucleoside linkages (1)..(15)
  LNA nucleosides (1)..(3)
  5-methyl c (11)..(11)
  LNA nucleosides (14)..(15)
gcctcaaggtcggtc

SEQ ID NO: 790 - DNA, 15 bp, Artificial Sequence
  LNA antisense gapmer oligonucleotide
  phosphorothiate Internucleoside linkages (1)..(15)
  LNA nucleosides (1)..(2)
  5-methyl c (11)..(11)
  LNA nucleosides (14)..(15)
gcctcaaggtcggtc

SEQ ID NO: 791 - DNA, 15 bp, Artificial Sequence
  LNA antisense gapmer oligonucleotide
  phosphorothiate Internucleoside linkages (1)..(15)
  LNA nucleosides (1)..(2)
  LNA nucleosides (13)..(15)
atgcctacagcctcc

SEQ ID NO: 792 - DNA, 15 bp, Artificial Sequence
  LNA antisense gapmer oligonucleotide
  phosphorothiate Internucleoside linkages (1)..(15)
  LNA nucleosides (1)..(3)
  LNA nucleosides (14)..(15)
atgcctacagcctcc

SEQ ID NO: 793 - DNA, 15 bp, Artificial Sequence
  LNA antisense gapmer oligonucleotide
  phosphorothiate Internucleoside linkages (1)..(15)
  LNA nucleosides (1)..(2)
  LNA nucleosides (14)..(15)
atgcctacagcctcc

SEQ ID NO: 794 - DNA, 16 bp, Artificial Sequence
  LNA antisense gapmer oligonucleotide
  phosphorothiate Internucleoside linkages (1)..(16)
  LNA nucleosides (1)..(4)
  LNA nucleosides (13)..(16)
accaatttatgcctac

SEQ ID NO: 795 - DNA, 16 bp, Artificial Sequence
  LNA antisense gapmer oligonucleotide
  phosphorothiate Internucleoside linkages (1)..(16)
  LNA nucleosides (1)..(3)
  LNA nucleosides (13)..(16)
accaatttatgcctac

SEQ ID NO: 796 - DNA, 16 bp, Artificial Sequence
  LNA antisense gapmer oligonucleotide
  phosphorothiate Internucleoside linkages (1)..(16)
  LNA nucleosides (1)..(4)
  LNA nucleosides (14)..(16)
accaatttatgcctac

SEQ ID NO: 797 - DNA, 16 bp, Artificial Sequence
  LNA antisense gapmer oligonucleotide
  phosphorothiate Internucleoside linkages (1)..(16)
  LNA nucleosides (1)..(3)
  LNA nucleosides (14)..(16)
accaatttatgcctac

SEQ ID NO: 798 - DNA, 16 bp, Artificial Sequence
  LNA antisense gapmer oligonucleotide
  phosphorothiate Internucleoside linkages (1)..(16)
  LNA nucleosides (1)..(2)
  LNA nucleosides (13)..(16)
accaatttatgcctac

SEQ ID NO: 799 - DNA, 17 bp, Artificial Sequence
  Antisense oligonucleotide GalNAc conjugate
  GalNAc2-C6 (1)..(1)
  phosphodiester lnternucleoside linkages (1)..(3)
  LNA nucleosides (3)..(5)
  phosphorothioate lnternucleoside linkages (4)..(17)
  LNA nucleosides (15)..(17)
cagaaccactgaacaaa

SEQ ID NO: 800 - DNA, 18 bp, Artificial Sequence
  Antisense oligonucleotide GalNAc conjugate
  GalNAc2-C6 (1)..(1)
  phosphodiester lnternucleoside linkages (1)..(3)
  LNA nucleosides, LNA C are 5-methyl C (3)..(5)
  phosphorothioate lnternucleoside linkages (4)..(18)
  LNA nucleosides (16)..(18)
cacgaaccactgaacaaa

SEQ ID NO: 801 - DNA, 17 bp, Artificial Sequence
  Antisense oligonucleotide GalNAc conjugate
  GalNAc2-C6 (1)..(1)
  phosphodiester lnternucleoside linkages (1)..(3)
  LNA nucleosides, LNA C are 5-methyl C (3)..(5)
  phosphorothioate lnternucleoside linkages (4)..(17)
  LNA nucleosides, LNA C are 5-methyl C (15)..(17)
cacgaaccactgaacaa

SEQ ID NO: 802 - DNA, 17 bp, Artificial Sequence
  Antisense oligonucleotide GalNAc conjugate
  GalNAc2-C6 (1)..(1)
  phosphodiester lnternucleoside linkages (1)..(3)
  LNA nucleosides, LNA C are 5-methyl C (3)..(5)
  phosphorothioate lnternucleoside linkages (4)..(17)
  LNA nucleosides, LNA C are 5-methyl C (15)..(17)
caccgcagtatggatcg

SEQ ID NO: 803 - DNA, 17 bp, Artificial Sequence
  Antisense oligonucleotide GalNAc conjugate
  phosphodiester lnternucleoside linkages (1)..(3)
  LNA nucleosides, LNA C are 5-methyl C (3)..(5)
  phosphorothioate lnternucleoside linkages (4)..(17)
  LNA nucleosides (15)..(17)
cacgcgtaaagagaggt

SEQ ID NO: 804 - DNA, 17 bp, Artificial Sequence
  Antisense oligonucleotide GalNAc conjugate
  GalNAc2-C6 (1)..(1)
  phosphodiester lnternucleoside linkages (1)..(3)
  LNA nucleosides (3)..(5)
  phosphorothioate lnternucleoside linkages (4)..(17)
  LNA nucleosides, LNA C are 5-methyl C (15)..(17)
caagaaggcacagacgg

SEQ ID NO: 805 - DNA, 18 bp, Artificial Sequence
  Antisense oligonucleotide GalNAc conjugate
  GalNAc2-C6 (1)..(1)
  phosphodiester lnternucleoside linkages (1)..(3)
  LNA nucleosides (3)..(5)
  phosphorothioate lnternucleoside linkages (4)..(18)
  LNA nucleosides, LNA C are 5-methyl C (16)..(18)
cagagaaggcacagacgg

SEQ ID NO: 806 - DNA, 17 bp, Artificial Sequence
  Antisense oligonucleotide GalNAc conjugate
  GalNAc2-C6 (1)..(1)
  phosphodiester lnternucleoside linkages (1)..(3)
  LNA nucleosides, LNA C are 5-methyl C (3)..(5)
  phosphorothioate lnternucleoside linkages (4)..(17)
  LNA nucleosides, LNA C are 5-methyl C (15)..(17)
cagcgaagtgcacacgg

SEQ ID NO: 807 - DNA, 18 bp, Artificial Sequence
  Antisense oligonucleotide GalNAc conjugate
  GalNAc2-C6 (1)..(1)
  phosphodiester lnternucleoside linkages (1)..(3)
  LNA nucleosides, LNA C are 5-methyl C (3)..(5)
  phosphorothioate lnternucleoside linkages (4)..(18)
  LNA nucleosides, LNA C are 5-methyl C (16)..(18)
caagcgaagtgcacacgg

SEQ ID NO: 808 - DNA, 17 bp, Artificial Sequence
  Antisense oligonucleotide GalNAc conjugate
  GalNAc2-C6 (1)..(1)
  phosphodiester lnternucleoside linkages (1)..(3)
  LNA nucleosides, LNA C are 5-methyl C (3)..(5)
  phosphorothioate lnternucleoside linkages (4)..(17)
  LNA nucleosides, LNA C are 5-methyl C (15)..(17)
caagcgaagtgcacacg

SEQ ID NO: 809 - DNA, 18 bp, Artificial Sequence
  Antisense oligonucleotide GalNAc conjugate
  GalNAc2-C6 (1)..(1)
  phosphodiester lnternucleoside linkages (1)..(3)
  LNA nucleosides (3)..(5)
  phosphorothioate lnternucleoside linkages (4)..(18)
  5-methyl C (11)..(11)
  LNA nucleosides, LNA C are 5-methyl C (16)..(18)
caaggtgaagcgaagtgc

SEQ ID NO: 810 - DNA, 17 bp, Artificial Sequence
  Antisense oligonucleotide GalNAc conjugate
  GalNAc2-C6 (1)..(1)
  phosphodiester lnternucleoside linkages (1)..(3)
  LNA nucleosides (3)..(5)
  phosphorothioate lnternucleoside linkages (4)..(17)
  5-methyl C (11)..(11)
  LNA nucleosides (15)..(17)
caaggtgaagcgaagtg

SEQ ID NO: 811 - DNA, 16 bp, Artificial Sequence
  Antisense oligonucleotide GalNAc conjugate
  GalNAc2-C6 (1)..(1)
  phosphodiester lnternucleoside linkages (1)..(3)
  LNA nucleosides, LNA C are 5-methyl C (3)..(5)
  phosphorothioate lnternucleoside linkages (4)..(16)
  LNA nucleosides, LNA C are 5-methyl C (14)..(16)
cacgaaccactgaaca

SEQ ID NO: 812 - DNA, 15 bp, Artificial Sequence
  Antisense oligonucleotide GalNAc conjugate
  GalNAc2-C6 (1)..(1)
  phosphodiester lnternucleoside linkages (1)..(3)
  LNA nucleosides, LNA C are 5-methyl C (3)..(5)
  phosphorothioate lnternucleoside linkages (4)..(15)
  LNA nucleosides, LNA C are 5-methyl C (14)..(15)
cacgaaccactgaac

SEQ ID NO: 813 - DNA, 15 bp, Artificial Sequence
  Antisense oligonucleotide GalNAc conjugate
  GalNAc2-C6 (1)..(1)
  phosphodiester lnternucleoside linkages (1)..(3)
  LNA nucleosides, LNA C are 5-methyl C (3)..(5)
  phosphorothioate lnternucleoside linkages (4)..(15)
  LNA nucleosides, LNA C are 5-methyl C (14)..(15)
cacgcagtatggatc

SEQ ID NO: 814 - DNA, 16 bp, Artificial Sequence
  Antisense oligonucleotide GalNAc conjugate
  GalNAc2-C6 (1)..(1)
  phosphodiester lnternucleoside linkages (1)..(3)
  LNA nucleosides, LNA C are 5-methyl C (3)..(5)
  phosphorothioate lnternucleoside linkages (4)..(16)
  LNA nucleosides (14)..(16)
cagcgtaaagagaggt

SEQ ID NO: 815 - DNA, 15 bp, Artificial Sequence
  Antisense oligonucleotide GalNAc conjugate
  GalNAc2-C6 (1)..(1)
  phosphodiester lnternucleoside linkages (1)..(3)
  LNA nucleosides, LNA C are 5-methyl C (3)..(5)
  phosphorothioate lnternucleoside linkages (4)..(15)
  LNA nucleosides (14)..(15)
cagcgtaaagagagg

SEQ ID NO: 816 - DNA, 15 bp, Artificial Sequence
  Antisense oligonucleotide GalNAc conjugate
  GalNAc2-C6 (1)..(1)
  phosphodiester lnternucleoside linkages (1)..(3)
  LNA nucleosides (3)..(5)
  phosphorothioate lnternucleoside linkages (4)..(15)
  5-methyl C (13)..(13)
  LNA nucleosides (14)..(15)
cagaagtgcacacgg

SEQ ID NO: 817 - DNA, 15 bp, Artificial Sequence
  Antisense oligonucleotide GalNAc conjugate
  GalNAc2-C6 (1)..(1)
  phosphodiester lnternucleoside linkages (1)..(3)
  LNA nucleosides, LNA C are 5-methyl C (3)..(5)
  phosphorothioate lnternucleoside linkages (4)..(15)
  LNA nucleosides, LNA C are 5-methyl C (14)..(15)
cacgaagtgcacacg

SEQ ID NO: 818 - DNA, 16 bp, Artificial Sequence
  Antisense oligonucleotide GalNAc conjugate
  GalNAc2-C6 (1)..(1)
  phosphodiester lnternucleoside linkages (1)..(3)
  LNA nucleosides (3)..(5)
  phosphorothioate lnternucleoside linkages (4)..(16)
  5-methyl C (11)..(11)
  LNA nucleosides (14)..(16)
caaggtgaagcgaagt

SEQ ID NO: 819 - DNA, 17 bp, Artificial Sequence
  Antisense oligonucleotide GalNAc conjugate
  GalNAc2-C6 (1)..(1)
  phosphodiester lnternucleoside linkages (1)..(3)
  LNA nucleosides (3)..(5)
  phosphorothioate lnternucleoside linkages (4)..(17)
  LNA nucleosides, LNA C are 5-methyl C (14)..(17)
cagaaccactgaacaaa

SEQ ID NO: 820 - DNA, 18 bp, Artificial Sequence
  Antisense oligonucleotide GalNAc conjugate
  GalNAc2-C6 (1)..(1)
  phosphodiester lnternucleoside linkages (1)..(3)
  LNA nucleosides (3)..(6)
  phosphorothioate lnternucleoside linkages (4)..(18)
  LNA nucleosides, LNA C are 5-methyl C (16)..(18)
cacgaaccactgaacaaa

SEQ ID NO: 821 - DNA, 15 bp, Artificial Sequence
  Antisense oligonucleotide GalNAc conjugate
  GalNAc2-C6 (1)..(1)
  phosphodiester lnternucleoside linkages (1)..(3)
  LNA nucleosides (3)..(5)
  phosphorothioate lnternucleoside linkages (4)..(15)
  LNA nucleosides, LNA C are 5-methyl C (13)..(15)
cagaagtgcacacgg

SEQ ID NO: 822 - DNA, 17 bp, Artificial Sequence
  Antisense oligonucleotide GalNAc conjugate
  GalNAc2-C6 (1)..(1)
  phosphodiester lnternucleoside linkages (1)..(3)
  LNA nucleosides (3)..(5)
  phosphorothioate lnternucleoside linkages (4)..(17)
  LNA nucleosides, LNA C are 5-methyl C (15)..(17)
catagtaaactgagcca

SEQ ID NO: 823 - DNA, 15 bp, Artificial Sequence
  Antisense oligonucleotide GalNAc conjugate
  GalNAc2-C6 (1)..(1)
  phosphodiester lnternucleoside linkages (1)..(3)
  LNA nucleosides, LNA C are 5-methyl C (3)..(5)
  phosphorothioate lnternucleoside linkages (4)..(15)
  LNA nucleosides, LNA C are 5-methyl C (13)..(15)
cacgaaccactgaac

SEQ ID NO: 824 - DNA, 16 bp, Artificial Sequence
  Antisense oligonucleotide GalNAc conjugate
  GalNAc2-C6 (1)..(1)
  phosphodiester lnternucleoside linkages (1)..(3)
  LNA nucleosides, LNA C are 5-methyl C (3)..(5)
  phosphorothioate lnternucleoside linkages (4)..(16)
  LNA nucleosides, LNA C are 5-methyl C (13)..(16)
cacgaaccactgaaca

SEQ ID NO: 825 - DNA, 15 bp, Artificial Sequence
  Antisense oligonucleotide GalNAc conjugate
  GalNAc2-C6 (1)..(1)
  phosphodiester lnternucleoside linkages (1)..(3)
  LNA nucleosides, LNA C are 5-methyl C (3)..(5)
  phosphorothioate lnternucleoside linkages (4)..(15)
  LNA nucleosides (13)..(15)
cagcgtaaagagagg

SEQ ID NO: 826 - DNA, 17 bp, Artificial Sequence
  Antisense oligonucleotide GalNAc conjugate
  GalNAc2-C6 (1)..(1)
  phosphodiester lnternucleoside linkages (1)..(3)
  LNA nucleosides (3)..(4)
  phosphorothioate lnternucleoside linkages (4)..(17)
  5-methyl C (11)..(11)
  LNA nucleosides (14)..(17)
caaggtgaagcgaagtg

SEQ ID NO: 827 - DNA, 24 bp, Artificial Sequence
  oligonucleotide target sequence
acggggcgcacctctctttacgcg

SEQ ID NO: 828 - DNA, 22 bp, Artificial Sequence
  oligonucleotide target sequence
cgtgtgcacttcgcttcacctc

SEQ ID NO: 829 - DNA, 16 bp, Artificial Sequence
  oligonucleotide target sequence
ccgtctgtgccttctc

SEQ ID NO: 830 - DNA, 15 bp, Artificial Sequence
  oligonucleotide target sequence
cgatccatactgcgg

SEQ ID NO: 831 - DNA, 15 bp, Artificial Sequence
  oligonucleotide target sequence
tggctcagtttacta

SEQ ID NO: 832 - DNA, 15 bp, Artificial Sequence
  oligonucleotide sequence motif
ccgcagtatggatcg

SEQ ID NO: 833 - DNA, 15 bp, Artificial Sequence
  oligonucleotide target sequence
ctagtgccatttgtt

SEQ ID NO: 834 - DNA, 15 bp, Artificial Sequence
  oligonucleotide sequence motif
tagtaaactgagcca

SEQ ID NO: 835 - DNA, 16 bp, Artificial Sequence
  oligonucleotide sequence motif
ctagtaaactgagcca

SEQ ID NO: 836 - DNA, 15 bp, Artificial Sequence
  oligonucleotide sequence motif
ctagtaaactgagcc

SEQ ID NO: 837 - DNA, 15 bp, Artificial Sequence
  oligonucleotide sequence motif
gcactagtaaactga

SEQ ID NO: 838 - DNA, 16 bp, Artificial Sequence
  oligonucleotide sequence motif
ggcactagtaaactga

SEQ ID NO: 839 - DNA, 15 bp, Artificial Sequence
  oligonucleotide sequence motif
caacggggtaaaggt

SEQ ID NO: 840 - DNA, 15 bp, Artificial Sequence
  oligonucleotide sequence motif
cagtatggatcggca

SEQ ID NO: 841 - DNA, 16 bp, Artificial Sequence
  oligonucleotide sequence motif
ttccgcagtatggatc

SEQ ID NO: 842 - DNA, 15 bp, Artificial Sequence
  oligonucleotide sequence motif
ttccgcagtatggat

SEQ ID NO: 843 - DNA, 16 bp, Artificial Sequence
  oligonucleotide sequence motif
gttccgcagtatggat

SEQ ID NO: 844 - DNA, 15 bp, Artificial Sequence
  oligonucleotide sequence motif
gttccgcagtatgga

SEQ ID NO: 845 - DNA, 16 bp, Artificial Sequence
  oligonucleotide sequence motif
agttccgcagtatgga

SEQ ID NO: 846 - DNA, 15 bp, Artificial Sequence
  oligonucleotide sequence motif
agttccgcagtatgg

SEQ ID NO: 847 - DNA, 16 bp, Artificial Sequence
  oligonucleotide sequence motif
gagttccgcagtatgg

SEQ ID NO: 848 - DNA, 15 bp, Artificial Sequence
  oligonucleotide sequence motif
gagttccgcagtatg

SEQ ID NO: 849 - DNA, 16 bp, Artificial Sequence
  oligonucleotide sequence motif
ggagttccgcagtatg

SEQ ID NO: 850 - DNA, 16 bp, Artificial Sequence
  oligonucleotide sequence motif
taaagagaggtgcgcc

SEQ ID NO: 851 - DNA, 15 bp, Artificial Sequence
  oligonucleotide sequence motif
taaagagaggtgcgc

SEQ ID NO: 852 - DNA, 16 bp, Artificial Sequence
  oligonucleotide sequence motif
gtaaagagaggtgcgc

SEQ ID NO: 853 - DNA, 15 bp, Artificial Sequence
  oligonucleotide sequence motif
gtaaagagaggtgcg

SEQ ID NO: 854 - DNA, 16 bp, Artificial Sequence
  oligonucleotide sequence motif
cgtaaagagaggtgcg

SEQ ID NO: 855 - DNA, 15 bp, Artificial Sequence
  oligonucleotide sequence motif
cgtaaagagaggtgc

SEQ ID NO: 856 - DNA, 16 bp, Artificial Sequence
  oligonucleotide sequence motif
gcgtaaagagaggtgc

SEQ ID NO: 857 - DNA, 15 bp, Artificial Sequence
  oligonucleotide sequence motif
gcgtaaagagaggtg

SEQ ID NO: 858 - DNA, 16 bp, Artificial Sequence
  oligonucleotide sequence motif
cgcgtaaagagaggtg

SEQ ID NO: 859 - DNA, 16 bp, Artificial Sequence
  oligonucleotide sequence motif
tgagaaggcacagacg

SEQ ID NO: 860 - DNA, 15 bp, Artificial Sequence
  oligonucleotide sequence motif
gcctcaaggtcggtc

SEQ ID NO: 861 - DNA, 15 bp, Artificial Sequence
  oligonucleotide sequence motif
atgcctacagcctcc

SEQ ID NO: 862 - DNA, 16 bp, Artificial Sequence
  oligonucleotide sequence motif
accaatttatgcctac